European Patent Specification EP 3 732 189 B1, published May 27, 2026. Title: GENETIC MODULATION OF PHOTOSYNTHETIC ORGANISMS FOR IMPROVED GROWTH. Applicant: SYNTHETIC GENOMICS, INC. AJJAWI, Imad KUZMINOV, Fedor RADAKOVITS, Randor R. VERRUTO, John H. TACKE, Sarah SPREAFICO, Roberto LAMBERT, William F. GREINER, Jessica Nichole. The sequence listing filed with the application follows.

SEQUENCE LISTING (105 sequences)

SEQ ID NO: 1 - DNA, 4531 bp, Parachlorella sp.
atgtctggttcagctggatcgggccaggctactctcagacatgacggtggctctgctggcggcagtgggcctgtctcagacggtttttcaccggccggcctgaaggtaaagtagaaagacactcatacacatcttggttcggcgttgaaagtaggtcattaacatactctataaccaatatttgtaggttctggtcgtggacgacgacctcatgtgccttaaggtggtgtcagccatgttgaagaggtgcagctatcaaggtgaggtctttactggtgtctgttattgctgtaacatcatttcgctgttgcacaatttaaacatttgtaatttactgttgttattgcagtggccacttgtagcagtggcagcgaggcactgacacttctacgtgaacgcaacgaggacggatcctccgaccagttcgacctcgtactgtcagatgtttacatgccgggtatgtcgtattcctttgtaaactttacaatatgcgtctagtttgacgcgtacactttgtacactttgcaaaaacgcaccctgcgaggtctgccatttggtcactacaacttggccaccttggttgcaagtttgcaagttcgctctacgtcaacgctgcaaaatgaaccaattgttttgcactgaccctgccaaccttcatttgtggctgcagacatggacggtttcaagctgcttgaacacatcggtctagagttggagcttcccgttatcagtaagttgatcgagccgagtccagagcgaagcctgcttctatactattagcagctgtcttttgatatttgacagcttgacttgatatggtcacagagcatacttgcaaccaggttacctgttgaactagcaactgtgcccaagcatctcttcaagcacctccgtcagtccatagggtactgttgatttgtactctgcaatactgcactgtaatgcgctgtgaatcactgcccttcacctctagatggtgcttccctggagccctcccccacctccgcctcaagcccctcacatgcctctcccccccctgcagtgatgtcatccaacggggacacgaatgtcgtgctgcggggggtcacccacggggctgtggactttctgatcaagcccgttcgaattgaggagctgcggaacgtgtggcagcacgtggtgcgtcgtcgttccatggcgctggccaggacgccagacgaggggggacactcggacgaggactctcaggtgcccttggcagcttctgggcggcttgctgtgtcggatgccacttggactggggatgcacgaggggtggggggacaatgggagatgggccatagtaggccagagttgatggcagtggtggtgggggggagtaggcgggagagaagcagccatcctggtgttggttttgatgattgagtgcatggggatgatgcacaggtgagctgactggatgccttgtcttgctgtgctgcgctgcagcggcacagtgtgaaacgcaaggagtcggagcagagcccgctgcagctcagcacagagcagggcgggaacaagaagccaagagtggtgtggtcggtggagatgcaccaacaggtgtgcttgcgggcgggtgtatacgggggaggggggccagctgctggctgacctggcgtgcgcggtgcattgcacttggcgatgaggggcgtgcttcagtatgtagctgggacgcaattggttgtgctgtgtgaccagtgcacaaaatacatccctgaattccagtgggttgaacagagttgtcctggaggtgggaagcaaacgcgcacgtggtagaggggagcagggtgcagaacagccgcagcaggggtgttgcgcagtgtgcaggtatcctgcctccatgccccgggccatgggcatactacgctggtaccgtcaggatgggcgttgagcctggcttggggggcagggggcgagcgaatgcggaatgggagcggcaggtgctgggagggtggctgactggcttgcaggagcgcaagtcctgtcgggggcgtcgtcctgttccctcctgcccgcttcacccacgttcactctcatgcctccacactcctgctgctgacacacctgtcgccacctccgctgcagtttgtgaacgcggtcaactccctgggcattgacaaggcggtgcccaagcggattctggacctgatgaacgtggaggggctgacgcgcgagaacgtggccagccatctgcaggtgcctgccatgacccctcccaccagggacctggtgttttgacaccctggaactcctctttgacggagcctccagttcaattccagcaatcgaattgaatcaaaaagcatgtgcacccacgtgctgtttgaatgtcccatgtggtaggaaacacaactgcccccttgccatttgctggagggtgcccgctgcgccatgcccgagtgcgctgtgctcagcgttgtgctgcgccccccgctgactgaagctgacagcgtgcggctgaggagggtactgggggagggggggtgggaggcggccgctggcggcggaagggagggtgtgcacgcatggacacagggcctttccgccctgcacggcctctactgcaccctgccacgtgatgtatcgacatggtgggccatgctgtgctgtgccgctgcagaagtaccgcctgtacctgaagcgggtggagggagtgcaatcgggtgcggcagcctccaagcagcaccagcacccgcagtatcaccagcagcagcagcagcagcaagcgcaacctcgtgcagctgtctcccctgcagcagcttcctttggtgccctttccttgggagccccgcagcaggcgcagcagggcatgccgcagctggggatgcctgtgcaggtgaagactgcccccccccccctccccctttccatcttccctccatcagcctgctgttccttacccttgtcaacccgtctctcctttttcgcaagcagcgcaccaccccccatgcacgccttgcctggcactgttgtcagctgcccccctagaaatacacaaggtgtgggtgcaactggtgggaccccctcccccccccccctggggctgcagggtctccctccaaacttggcagccatgggatcccagccgccgcacatccccttccagcaggccctggccatgcaggcggcggctgcggcggctgcagccagcggcgcgctccccgggagtctgcccccctacatgccacccccggggatgatgccccccggcatgccggggggggtccccggtatgggaggggtggtggggcatcctcaggtacgggcagcacatgagtgggcaggggtattggagaggggaagggcagggaggttgcatgtgaggggctgcatggcaaagaggctgcagcgcaggtgttgcttgcagcacttcccctcggtggcgcttgcatcaaattttgaatcctcccccgatgggcacgcccgtgtgtgggggggggtgggatgggggatgggggtggttttgtggcatgtcgggcgctttcatctacccgggcccctgcccctgcctgtacgcgtgcgcatgtgtgcagatgcccgccccagggatggactttgcgggtttcaacgggtatggcaacgctgcgggggggctgatgtttggcgggcagcagcaggcgcagcacgcgcagcagcacgcgtcagcgcaagcgggctcgctggcgcagcagcaggcgcagcaagtatccatgggcttgggccttatgccccccccgttggggttcccgcccacctcgctcgccgcgccagccccgcgctccgcagcaactgagcccgccgcagccccactccccctgacgtcctcgccgccagctgcttcagcaggcggcagcggcggcccagcagcagctgctccgcagcacagcagcggcgccgcagcagcccaagccccccatcaccacccacagtgctcggagcagggagcgggggggctcccgcccccgctgcccgcgtccagcgccccgcagtcctatcccctccctcccccctcctcgcaggccgctttgcatgacccggacgaacactaccccccaggctcggcagaggtgagcacgtccccccgccccctccccccccccccccccccttcccttcaccctggcttggcgtgcaatgaaaccctaaataaccctaaaacctcattatcagttgcaaattggacccgtgaagcgggcgggggcaactgcgctctgctggtgtcagcgctgtctctgccggttcctgcccagcgtgcgcctgcatgcaaggggggatggggggggggaggcatttaacaataggccagtcatctccaatccaccgtcaatttcagccccctccccccccctccctcatccccttgcagatgcaccaccagcacctcccagggctgtgtggctttaacccggacgacctgctgggggggcagctgggggacatggggttcctgggggagctggggggggcggtgggaggaaagcacgaacaggacgacttcctggacctgctgctgaagggggaggaggagctgtga

SEQ ID NO: 2 - DNA, 1860 bp, Parachlorella sp.
atgtctggttcagctggatcgggccaggctactctcagacatgacggtggctctgctggcggcagtgggcctgtctcagacggtttttcaccggccggcctgaaggttctggtcgtggacgacgacctcatgtgccttaaggtggtgtcagccatgttgaagaggtgcagctatcaagtggccacttgtagcagtggcagcgaggcactgacacttctacgtgaacgcaacgaggacggatcctccgaccagttcgacctcgtactgtcagatgtttacatgccggacatggacggtttcaagctgcttgaacacatcggtctagagttggagcttcccgttatcatgatgtcatccaacggggacacgaatgtcgtgctgcggggggtcacccacggggctgtggactttctgatcaagcccgttcgaattgaggagctgcggaacgtgtggcagcacgtggtgcgtcgtcgttccatggcgctggccaggacgccagacgaggggggacactcggacgaggactctcagcggcacagtgtgaaacgcaaggagtcggagcagagcccgctgcagctcagcacagagcagggcgggaacaagaagccaagagtggtgtggtcggtggagatgcaccaacagtttgtgaacgcggtcaactccctgggcattgacaaggcggtgcccaagcggattctggacctgatgaacgtggaggggctgacgcgcgagaacgtggccagccatctgcagaagtaccgcctgtacctgaagcgggtggagggagtgcaatcgggtgcggcagcctccaagcagcaccagcacccgcagtatcaccagcagcagcagcagcagcaagcgcaacctcgtgcagctgtctcccctgcagcagcttcctttggtgccctttccttgggagccccgcagcaggcgcagcagggcatgccgcagctggggatgcctgtgcagggtctccctccaaacttggcagccatgggatcccagccgccgcacatccccttccagcaggccctggccatgcaggcggcggctgcggcggctgcagccagcggcgcgctccccgggagtctgcccccctacatgccacccccggggatgatgccccccggcatgccggggggggtccccggtatgggaggggtggtggggcatcctcagatgcccgccccagggatggactttgcgggtttcaacgggtatggcaacgctgcgggggggctgatgtttggcgggcagcagcaggcgcagcacgcgcagcagcacgcgtcagcgcaagcgggctcgctggcgcagcagcaggcgcagcaagtatccatgggcttgggccttatgccccccccgttggggttcccgcccacctcgctcgccgcgccagccccgcgctccgcagcaactgagcccgccgcagccccactccccctgacgtcctcgccgccagctgcttcagcaggcggcagcggcggcccagcagcagctgctccgcagcacagcagcggcgccgcagcagcccaagccccccatcaccacccacagtgctcggagcagggagcgggggggctcccgcccccgctgcccgcgtccagcgccccgcagtcctatcccctccctcccccctcctcgcaggccgctttgcatgacccggacgaacactaccccccaggctcggcagagatgcaccaccagcacctcccagggctgtgtggctttaacccggacgacctgctgggggggcagctgggggacatggggttcctgggggagctggggggggcggtgggaggaaagcacgaacaggacgacttcctggacctgctgctgaagggggaggaggagctgtga

SEQ ID NO: 3 - protein, 619 aa, Parachlorella sp.
MSGSAGSGQATLRHDGGSAGGSGPVSDGFSPAGLKVLVVDDDLMCLKVVSAMLKRCSYQVATCSSGSEALTLLRERNEDGSSDQFDLVLSDVYMPDMDGFKLLEHIGLELELPVIMMSSNGDTNVVLRGVTHGAVDFLIKPVRIEELRNVWQHVVRRRSMALARTPDEGGHSDEDSQRHSVKRKESEQSPLQLSTEQGGNKKPRVVWSVEMHQQFVNAVNSLGIDKAVPKRILDLMNVEGLTRENVASHLQKYRLYLKRVEGVQSGAAASKQHQHPQYHQQQQQQQAQPRAAVSPAAASFGALSLGAPQQAQQGMPQLGMPVQGLPPNLAAMGSQPPHIPFQQALAMQAAAAAAAASGALPGSLPPYMPPPGMMPPGMPGGVPGMGGVVGHPQMPAPGMDFAGFNGYGNAAGGLMFGGQQQAQHAQQHASAQAGSLAQQQAQQVSMGLGLMPPPLGFPPTSLAAPAPRSAATEPAAAPLPLTSSPPAASAGGSGGPAAAAPQHSSGAAAAQAPHHHPQCSEQGAGGLPPPLPASSAPQSYPLPPPSSQAALHDPDEHYPPGSAEMHHQHLPGLCGFNPDDLLGGQLGDMGFLGELGGAVGGKHEQDDFLDLLLKGEEEL

SEQ ID NO: 4 - DNA, 2802 bp, Parachlorella sp.
atggctgcccccccagtatctatctcttccaattttccaaaggttagtatttacgtaacatttgccgacagttgggcaataacgctgagttggagtgttgccaacaagcttttgtgccgtttccagggtttgcgggttctcttggtcgatcaacagccaagtaggagccatattgaagcgcagctgatgcagccggatcttaattacacaggtttgctgcagttttgcacattccaagcttggcctttctccgtgccaaacccagcgcgctgagctcttgttgtttgttgcagttactggttgcgagagcgtttctgaagctctttcatattgccgctcgggagtaagcagctttgacgtggtgcttgcggaggtgggtggtagtgcttcgcgaggtgcacagtgcgcaccgggaaaaacttgaaaagtatttgtaaaattaattttgaaacttctgtattattttacacctcttaacaatgcacccaatgtttgttatgagcgccacgttaccggacgtttgttgcaggcaaggatcgttgccgtcgacgagacttcggggcgcgcatttatcgactctcttgaagatacaccggttattcttatgtcggagggaagcacgacgggcgacgttcttcgtgcggtgaagcttggagctgtggactggctggataagcctctctccgtcctgaagctcaagaacatctggcagcactcagtgcgtaaggtaggtccggaaacaatatgatatctacaattggaaagttaccagtgtcaactatggaaaacgttgtactgggtgctagtttcagttgagccagttgcctgtatatgcatataaggggcagtgacgcagtgtctgccctgtgagctgtgatgcatcagggtgcacctgaagctggcagtggatcactccacccaagatgttgttgcaatccaatgtgttgctgatgccttgcttttctgacttgcaaacatggtgtgggataaaagcgttgctagacagccaccgtgctccacgttgtcttctgcatgcaaaactgcagatgatgcagcgcaccacgttttacgacacttgctccgagcagccaacccagccggcgcgcagcaagctttcttcaggaatcgaatcgccgagcacacccacgctgggagactctgtggacttggacgccatctcggcggcttccttcggcagcatcaaggacttgaccgatttttcattttccagcggagctgaggtgggcatcgctggttgtccagcactgcagcatttcccaccagcttggttggttgcctgtgttttagtgcagagcagaggccgaggctactggttcaaccagcctagttactcaaaacaattttggcaacctgctgacttctctcttaacctgcagagcgtttcacagcatgtacacttttcagtgggtttcgtaatttcgtagcgcacccgctggcttttttctgcaggtcctgagagcctcctttgacagctgtgacggctccgaggtcaacctaggcagcgctttgggccagcctcgcccccctctggcagtcaagcccagctcctttggccccctggtgagtggcatagctcagcaggagacccacaagtggctggaacccaccatgttggcgcgcaccctgccctcgcacgcgcggctgccgtctgcgcagcgcgccgcggtgcgccgctgtggagttgtggtgttgcggagtcactcgcgggccagtgcttcacagcccattctcgccgcacacaccctgcccgcacaaatggctgccacccccctaaagcggtcctcaggccacccggatgtgctcaggatggatccgccgaatctcgcacccctcctccctcaatcccggttgttcagacggtttggaacccctccggctctctacccctctgcaggtacccgtccctcccacctcccagtggccccagctgcaggctggctgcgtgtggggcactcccgtgggcggcccgctggcgcccccctccatgaccaacgcccagcatggtgccccccacagcgtgcccctggcagacgcacacttggccggcagcgccagttacatgtccctctcctctgtgagtctcctcccctccacccctacatcttccaatcgaacatgcgacgcacgcacacccatagtccctaaacaagtgctttggtgttttttcacttgcaaaccccaaccctgacacctgaagcgtgacacaggcgactgcgctgctccccgcccccacacgcccttggttgtttgtgccctgcacttctgccacgacatgcatgtcatgtcttttcacgcctgcgatgtcgctgcttaaacttgaaactcattgtggccggggtgcagctcatggaggaggacaccccctgtcccttggacatggatgcaccagaggacgggatgcagcttcctgttgacttcctgtctgttgccaacgtcagcagcaatggtaggtccagcaccagacgcctctgtctgctatgagacgcacctccagccgccccctctggacagacagcgcgctgcacgctctgcgcgctggaccttgccgcacacgcgcgcgacaaggcctggtgtgatgcttggatgtggaaggttccagcatggttggacaagatggtatcctggcacacatattggtatgcagcatacacccaggctgcccccttaccctcgcacgccctaccccttactgcaggcagcggtcccattgggttgaagctgaagaaaagcaacagcctgctgaacatgatcaacgcagcgctgatgtctggtggtcagtga

SEQ ID NO: 5 - protein, 359 aa, Parachlorella sp.
MAAPPVSISSNFPKGLRVLLVDQQPSRSHIEAQLMQPDLNYTVTGCESVSEALSYCRSGVSSFDVVLAEARIVAVDETSGRAFIDSLEDTPVILMSEGSTTGDVLRAVKLGAVDWLDKPLSVLKLKNIWQHSVRKMMQRTTFYDTCSEQPTQPARSKLSSGIESPSTPTLGDSVDLDAISAASFGSIKDLTDFSFSSGAEVLRASFDSCDGSEVNLGSALGQPRPPLAVKPSSFGPLVPVPPTSQWPQLQAGCVWGTPVGGPLAPPSMTNAQHGAPHSVPLADAHLAGSASYMSLSSLMEEDTPCPLDMDAPEDGMQLPVDFLSVANVSSNGSGPIGLKLKKSNSLLNMINAALMSGGQ

SEQ ID NO: 6 - protein, 119 aa, Parachlorella sp.
GLRVLLVDQQPSRSHIEAQLMQDLNYTVTGCESVSEALSYCRSGVSSFDVVLAEARIVAVDETSGRAFIDSLEDTPVILMSEGSTTGDVLRAVKLGAVDWLDKPLSVLKLKNIWQHSVR

SEQ ID NO: 7 - DNA, 1080 bp, Parachlorella sp.
atggctgcccccccagtatctatctcttccaattttccaaagggtttgcgggttctcttggtcgatcaacagccaagtaggagccatattgaagcgcagctgatgcagccggatcttaattacacagttactggttgcgagagcgtttctgaagctctttcatattgccgctcgggagtaagcagctttgacgtggtgcttgcggaggcaaggatcgttgccgtcgacgagacttcggggcgcgcatttatcgactctcttgaagatacaccggttattcttatgtcggagggaagcacgacgggcgacgttcttcgtgcggtgaagcttggagctgtggactggctggataagcctctctccgtcctgaagctcaagaacatctggcagcactcagtgcgtaagatgatgcagcgcaccacgttttacgacacttgctccgagcagccaacccagccggcgcgcagcaagctttcttcaggaatcgaatcgccgagcacacccacgctgggagactctgtggacttggacgccatctcggcggcttccttcggcagcatcaaggacttgaccgatttttcattttccagcggagctgaggtcctgagagcctcctttgacagctgtgacggctccgaggtcaacctaggcagcgctttgggccagcctcgcccccctctggcagtcaagcccagctcctttggccccctggtacccgtccctcccacctcccagtggccccagctgcaggctggctgcgtgtggggcactcccgtgggcggcccgctggcgcccccctccatgaccaacgcccagcatggtgccccccacagcgtgcccctggcagacgcacacttggccggcagcgccagttacatgtccctctcctctctcatggaggaggacaccccctgtcccttggacatggatgcaccagaggacgggatgcagcttcctgttgacttcctgtctgttgccaacgtcagcagcaatggcagcggtcccattgggttgaagctgaagaaaagcaacagcctgctgaacatgatcaacgcagcgctgatgtctggtggtcagtga

SEQ ID NO: 8 - DNA, 1707 bp, Parachlorella sp.
atgcttcggcagcagctgttgcacagcggcaggcagccgggtgcgacatgcagcttactaacctgctcgacatggcgaccgtctgccttgttcggccgtcctaagccccaaaaactgcacagccagcgcttgcagcatcagggccgcccctcccgcctcgtcgtgcgcagcgcaatgttcgacaacctgagccgcagcctggagagggcgtgggacatggtgcgcaaggacgggcggctaacggcggacaacatcaaggagcccatgcgggagattcgcagggcgctgcttgaggcggatgtgaggctgggggcgccgctgatcagattcttggtatctaccccccccccctcccaggtctccctccccgtggtgcgcaagtttgtgaaggcggtggaggagaaggcgctgggttctgcagtgaccaagggtgtcacccccgaccagcagctggtgaaggtggtgtacgaccagctgcgggagctgatgggggggcagcaggaagggctggtgcccacttcgccagaggagccgcaggtgatcttgatggcggggctgcagggcacggggaagacgacagctgcggggaagctggccttgttcctgcagaagaaggggcagaaggtgctgctggtggccaccgacatctaccgccccgccgccatcgaccagctggtgaagctgggcgacaggataggggtgccggtgttccagctgggaacccaggtgcagccgccggagattgcaaggcaggggctggagaaggcgcgagcagaggggtttgacgccgtcatcgtcgacacggcggggcggctgcagatcgaccagagcatgatggaggagctggtgcagatcaagtccacggtgaagccctccgacacgctgctagtggtcgatgcgatgacggggcaggaggcagccgggctggtgaaggcgttcaatgatgccgtggacatcacaggcgccgtgctgaccaagcttgacggggacagccgcggcggcgccgcgctgagcgtgcgccaggtcagcgggcggcccatcaagtttgtgggcatgggggagggcatggaggcgctggagcccttctaccccgagcgcatggccagcaggattctgggcatgggtgacgtggtcaccctggtggagaaggctgaggagagcatcaaggaagaggaggcgcaggagatatcgcggaagatgctgtcggccaaatttgactttgacgacttcctgaagcagtacaagatggtggcggggatggggaacatggcccaaatcatgaagatgctgccaggcatgaacaagtttacggagaagcagctggcgggcgttgagaagcagtacaaggtgtacgagagcatgatccagagcatgacggtgaaggagcgcaagcagccggagctgttggtgaagtcgccctccaggaggcggcgcatagcgcgcgggtcggggcgctcggagcgggaggtcacagagctgctgggggtgttcaccaacctgcggacgcagatgcagagcttctccaaaatgatggccatgggggggatgggcatgggctccatgatgagcgacgaggagatgatgcaggccacgctggcaggcgccggcccccgccccgtgccagctggcaaggtgcggcggaagaagctggccgcggcgggcgggtcgcggggcatggctgagctggcatccctgaaggcagaatga

SEQ ID NO: 9 - protein, 302 aa, Coccomyxa subellipsoidea
MGLKARAASVSVHSSANNTASPLSSGRRGFPHSGEMSGEDLARSDSWEMFPAGLKVLVVDDDPLCLKVVEHMLRRCNYQVTTCPNGKAALEKLRDRSVHFDLVLSDVYMPDMDGFKLLEHIGLELDLPVIMMSSNGETNVVLRGVTHGAVDFLIKPVRVEELRNVWQHVVRRKRDQAVSQARDSRDISDEEGTDDGKPRDKKRKEVILVLWWDMQRRDSDDGVSAKKARVVWSVEMHQQFVQAVNQLGIDKAVPKRILDLMNVDGLTRENVASHLQVPHLSIFSPLFAELMSTLPRRCFYDF

SEQ ID NO: 10 - protein, 269 aa, Ostreococcus lucimarinus
FPAGLGVLVVDDDLLCLKVVEKMLKACKYKVTACSTAKTALEILRTRKEEFDIVLSDVHMPDMDGFKLLEIIQFELALPVLMMSANSDSSVVLRGIIHGAVDYLLKPVRIEELRNIWQHVVRRDYSSAKSSGSEDVEASSPSKRAKTSGSNSKSEEVDRTASEMSSGKARKKPTGKKGGKSVKEAEKKDVVDNSNSKKPRVVWSAELHAQFVTAVNQLGIDKAVPKRILDLMGVQGLTENVASHLQKYRLYLKRLQGNDARGGGNASST

SEQ ID NO: 11 - protein, 941 aa, Chlamydomonas reinhardtii
MDSQGVKLEEHPGHTGGHWQGFPAGLRLLVVDDDPLCLKVVEQMLRKCSYEVTVCSNATTALNILRDKNTEYDLVLSDVYMPDMDGFRLLELVGLEMDLPVIMMSSNGDTSNVLRGVTHGACDYLIKPVRLEELRNLWQHVVRRRRQHAQEIDSDEQSQERDEDQTRNKRKADAAGVTGDQCRLNGSGSGGAAGPGSGGGAGGMTDEMLMMSGGENGSNKKARVVWSVEMHQQFVNAVNQLGIDKAVPKKILEIMGVDGSAGRLADTSGRDVCGTVYRLYLKRVSGVTPSGHHHNAAHKSNKPSPHTTPPPPALPGQAGTHPANQATAIPPPPQPGSGTAAGAGAAAAGTGGGAAAANGHAATTGAGTPGAAPGAGGGVGGTGAGGLGSGPDGAAAAAGPGPGAAVPGGLGGLPLPPGAGPGPGPGGFGGPSPPPPPHPAALLANPMAAAVAGLNQSLLNAMGSLGVGVGGMSPLGPVGPLGPLGGLPGLPGMQPPPLGMGGLQPGMGPLGPLGLPGMGGLPGLPGMNPMANLMQGMAAGMAAANQMNGMGGHMGGHMGGMNGPMGALAGMNGLNGAMMGGLPGMGGPQNMFQAAAAAAAQQQQQQQEQQHAMMQQAAAGLLASQQQQQQQQQQQQQQQALQQQQQQGMAVSPPGPHNATPNGQLHTHPQAHHPHQHGLHAHAHPHQHLNTAPAGALGLSPPQPPAGLLSASGLSSGPDGSGLGSGVGGLLDGLQQHPHHPQLQLAGSLGTGGTGRSSGAAGRGSLDLPADLMGMALLDFPPVPVPGGADVGMAGAGGGAAGAHHHGHQGHQGIGGGAGVGIAGGVGCGVPAAAHGLEPAILMDDPADLGAVFSDVMYGTPGGGGVPGGVPGGGVGLGLGAGQVPSGPAGAGGLHSHHHQHHHHQHHLGHVVPVGGVDPLAGDAAKMAMNDDDFFNFLLKN

SEQ ID NO: 12 - protein, 523 aa, Chromochloris zofingiensis
MDGFKLLETVGLELDLPVIMMSSNGEHTTVMRGVTHGACDFLIKPVRIEELRNIWQHVIRRTRHPVFRDLEPDDHEGGDYEASKKRKDLYRGENSSGSGGAGGLERDDDGSASKKPRVVWSVEMHQQFVQAVNQLGIDKAVPKKILELMNVDGLTRENVASHLQKYRLYLKRVQGVQAPFGLPNIQLPRQTSSKGAGSSSQQQHHQQQQHQQQHQHQHQTALGTGQQQSHQLQPCPVSTATPVMPSPDAMVAASMMSSQAMAAMAPGVMNPMTAMNSMMAGLNPNMMGMAAGLGLAGLGIGGMAGHPVPNPMLAGMGPMGLGLPPPPGMPPPPPGMPPGMPPGMPPGMPAMMQGLSMAGMSHLAAAGMRPPPGALGGHLGGPGLSPFGPPPPPGADPANMMANMSSMMANMQAALAFQADAAAAAQHQAASTGSVAPGRQQQVHQHQQAVGMAVDDAAAFPSPGCRPNGSADAGAQSAAEPNDFSRVFDDPFAQPAASPSGAAAAGSNEAPGMDDFLDFFLKS

SEQ ID NO: 13 - protein, 834 aa, Volvox carteri
MDGRAEGTVAIKQEDHASGHWHNFPAGLRLLVVDDDPLCLKVVEQMLRKCSYDVTTCTNATMALNLLRDKSTEYDLVLSDVYMPDMDGFKLLEVVGLEMDLPVIMMSSNGDTSNVLRGVTHGACDYLIKPVRLEELRNLWQHVVRRRRQLNLDMDSDEHSQERDDDQGRKRKADTAGCIGDQLRMMGAGCSGGANGLGSTGNLGAVATGSAGLGLGLGTAADELGLGLDNGSSKKARVVWSVEMHQQFVNAVNQLGIDKAVPKKILEIMNVDGLTRENVASHLQKYRLYLKRVSGAQQPGQNRVSRPSPPQPQSPQVPSQQQQSLPGGGGAAAAGAGQLQGGGGAAAAAASLASILAGGGPAGGGAGAGPPPGGGQLGADGGGPGPGLSSAVANAMSAAAAAGGFPTPPPPPPPHPAALLAANPMMAAAAGLNPLLGAMGGLGVGPLGPLNPLNGMPMPGMQPPLGLLPGLPGPGGQLGLGPLGPIGLPGPGPLPSLPAGLPLNPMANGLQQMAAANLMQGMAGMGQLPALSMNGMNGIMGPLPGVGLPGPQQHLFPQQQQPHLQQQQQQQQQKDLQMAQKQHQAAAAAAAVAAAVAAAQHQQQQPQAQQQPQPQQQQQQPGKLPQATVGTPALASPAGALPRQPSGQHPHTLSSSSLHTQQPHQQQLLHSQPSSTHLATNNTLAMAPALNGTLDVGGKGHLHAAGGQGAGAGAGAVLDIPPDLIGGLIEDGFGAPPGPTIQLAHGTAAVLDPTMLLDEGDNSDFAAVFQEMSSYGGGGVIGGGGSGAGAMGVLGHGLLAAGGPVMVDVAAGLAGVTETATRVDDDFLNFLLKS

SEQ ID NO: 14 - protein, 446 aa, Tetraselmis sp.
MSCTVASFPPAAGGQGSPATPVPYQDLLVKRQDQWSNFPAGLRVLVADNDPASLQQVEKMLKKCSYQVTLCSSGKNSLEILRKRREEFDLVLADANLPDIDGFKLLHVCHTELSLPVVLMSGTSDTQLVMRGVMDGARDFLIKPLRVEELKVLWQHLVRFTSEITKTDAQLNVVKVELDGGRPAGEVSTSQNGSQCTEREGEGNSSKKQRMNWSDEMHQQFVNAVNQLGIDKAVPKRILDLMSVEGLTRENVASHLQKYRIYLKRMANHQENGKQAVMSTDTIARAEAAYQGGMPQGQQMMQQEHSGQAVQYSQPHAPGGLHQQAMPAQMHMGMMPAGPQPGSMQMAPHHVMQMPNGQVMVMQQMGPRPGMPPGMPQQMMASSQQMGMLQPGMPAGQMLHFQHPQQVHQHPPSSGPMHAVQHMEYAYSQPMQMAGWPVQGQPGNQA

SEQ ID NO: 15 - protein, 490 aa, Tetraselmis sp.
MTPTPPMSCTVASFPPAAGGQGSPATPVPYQDLLVKRQDQWSNFPAGLRVLVADNDPASLQQVEKMLKKCSYQVTLCSSGKNSLEILRKRREEFDLVLADANLPDIDGFKLLHVCHTELSLPVVLMSGTSDTQLVMRGVMDGARDFLIKPLRVEELKVLWQHLVRFTSEITKTDAQLNVVKVELDGGRPAGEVSTSQNGSQCTEREGEGNSSKKQRMNWSDEMHQQFVNAVNQLGIDKAVPKRILDLMSVEGLTRENVASHLQKYRIYLKRMANHQENGKQAVMSTDTIARAEAAYQGGMPQGQQMMQQEHSGQAVQYSQPHAPGGLHQQAMPAQMHMGMMPAGPQPGSMQMAPHHVMQMPNGQVMVMQQMGPRPGMPPGMPQQMMASSQQMGMLQPGMPAGQMLHFQHPQQVHQHPPSSGPMHAGGEMIDPGSMQRLHQQPHYIGPNGQHMPAPAMGMPSGTVQHMEYAYSQPMQMAGWPVQGQPGNQA

SEQ ID NO: 16 - protein, 574 aa, Tetraselmis sp.
MTMPLGGGLCMKDRIHGDERYRSKAKRQVNTIFAFTQRNTWRGRFRLCSYRTTELLGGSKTTEPGRGTFVLQIFMCVKNASIDDGSRHISTSRGLESVLKRRGGQGAPAAPVPYHDLLVKRQDQWSNFPAGLRVLVADNDPASLQQVEKMLKKCSYQVTLCSSGKNSLEILRKRREEFDLVLADANLPDIDGFKLLHVCHTELSLPVVLMSGTSDTQLVMRGVMDGARDFLIKPLRVEELKVLWQHLVRFTSEITKTDAQLNVVKVELDSGRPAGEVSTSQNGSQCAEREGEGNSSKKQRMNWSDEMHQQFVNAVNQLGIDKAVPKRILDLMSVEGLTRENVASHLQKYRIYLKRMANHQENGKQAVMSTDTIARAEAAYQGGMPQGQQMMQQEHSGQAVQYSQPHAPSGLHQQAMPAQMHMGMMPAGPQPGSMQMAPHHVMQMPNGQVMVMQQMGPRPGMPPGMPQQMMASSQQMGMLQPGMPAGQMLHFQHPQQVHQHPPSSGPMHAGGEMIDPGSMQRLHQQPHYIVPNAQHMPAPAMGMPPGAVQHMEYAYSQPMQMAGWPVQGQPGSQA

SEQ ID NO: 17 - protein, 674 aa, Oocystis sp.
MLAFTHQRMTTAPALAVATSHFFAHVRVTTGSSAIATVFAARSRGSGLLAGFNTMENVKVEVPEVVPENVNFPAGLKVLVVDDDPLCLKVIDQMLRRCNYAATTCQSSLEALELLRSSKENHFDLVLSDVYMPDMDGFKLLEIIGLEMGLPVIMMSSNGETGVVFRGVTHGAVDFLIKPVRIEELRNLWQHVVRKTMVVPSNDKATSEEDGEESKHRVDRKRKESFHSRAREQVEIACSVVPALLWPTVPPSSVHPTSSSFLRSHVLLLQRSSGGKDVLDEGGSNAKKPRVVWSVEMHQQFVNAVNQLGIDKAVPKRILDLMNVDGLTRENVASHLQKYRLYLKRVAGINTATGSRNGKGRSDVSGLSGMPNGSLPMPGMMPPHMAAGMLLAGMAADVGPRPHPFPIMPMPAMALQGMHGGMAQMMQLPPGMPPPMMMPMAPLLPSQLAALGQQQQQQQQQQVARSESMPSENGVAGPSGSFTAMLNGPAPMESSPFAALQVFGPPQGMEQLTQQQQQQQQAGAAAFVAAFAAANGGDMQGGGGGPGPMLGGAGGAGPLLGGVGGGDPLHGGGGSSALGGRPMMSAEQPMGGSGGLASNSLTVQQNDLAQMCSQLDVNGLQAVAAAAAAGAMGAPGGAGGAMPPSSVGGVGPDMKLTEQDDFFSFLLKDSNLID

SEQ ID NO: 18 - protein, 488 aa, Micromonas sp.
MSTPAVSKGFPIGLRVLVVDDDPLCLKIVEKMLKRCQYEVTTFSRGAEALKTLRERKDDFDIVLSDVHMPDMDGFKLLEHIALELDIPVMMMSANCATDVVLRGIIHGAVDYLLKPVRIEELRNIWQHVVRRKRESSQGNLRSGEGGSNGRTVSGGSTGEGGGKDSKGSSEQHGDAKDKTGSAGGSGGSSKRKKGSGKKGDEGTDEVKDGSGGDENEDSSALKKPRVVWSAELHQQFVTAVNQLGIDKAVPKRILDLMGVQGLTRENVASHLQKYRLYLKRLQGVNSGGAPGGGPGFMSPIALDGSMVQGGPGGRVGSPAIGGPNGPIMVGHGHIDPAMLAGGAPQTIQMGMVYGGPGMGPPQMMAPNGKGGGGMPGGYVMQPGQMMAPNGQMMPVGQMGPGGMMVQGPGGGMMQMHDGGMMNGNGSYGSLQNMKQGNGVVMMPNGGMGGVDGAIPNMATGLINGQGLPDDDVLDMFLKDGLPEGEGF

SEQ ID NO: 19 - protein, 544 aa, Micromonas pusilla
MTAEKKELKVFPAGLRVLVVDDDPLCLRIVEKMLKRCQYEVTTFSRGAEALETLRARRDDFDIVLSDVHMPDMDGFKLLEHIALELDVPVMMMSANCATDVVLRGIIHGAVDYLLKPVRLEELRNIWQHVVRRQREPSKDGAAGKGGGASGAPEVSGDTHANTDDKQDGNATDSKGSGSQKRKSGKSGDDGGKDGGGSGGKDGDASNKGNNNKRKKGKSNDATETAGGAGVEDNDDTSGLKKPRVVWSPELHQQFVTAVNQLGIDKAVPKRILDLMGVQGLTRENVASHLQKYRLYLKRLQGVNNNGTVPSGAAGFMTGLAIDGVGGVMGPPTTGSPAMNGPGGPGGGLVMGPGHMGGPHMDGSGMMHMGPGGPMAGMTVVYGGGMPGGMPGGADSKNGASGQPPPGGYVVMGGPHGGGPGGAPMMMQHGGMVPGPGPGLVPGPGGSLMMPAGMMPDGGGGMVGVHVGPGVVMGQHQLGGKHSSGGAGMAGGSAAGKGAQRGGVGGAFDVPPTNGSLDADEIGDDVLTMFLKDGLPEMNDGDAL

SEQ ID NO: 20 - protein, 776 aa, Sphagnum fallax
MSGGDLSRVREGTADLDPVMASHQHPPPRQQSHQQPKNHQQEAHQQHCSSAETTSPNNTARGAGATYGKMEPADDFPAGLRILVVDDDPTCLAILKKMLQQCSYQVTTCGRATRALELLREDKDKFDLVISDVYMPDMDGFKLLELVGLEMDLPVIMMSGNGETSVVMKGITHGACDYLLKPVRIEELSNIWQHVVRKLRSEPKEHSASLEDGDRQRRGGAEDADNTSSAADTADGIWRNKKKKEAKEDEEDFEQDNDDPSTLKKPRVVWSVELHQQFVSAVNQLGIDKAVPKRILELMSVQGLTRENVASHLQKYRLYLKRLSGVTSQSNSLNVSFGGPDAGYGGLFGLDEMSDYRNLVTNGHLPAQTIAALHHANMAGRLGASSGMVGPSSPLDPSVLAQIAALQSGSLPRPGMDGSLQGNQAGLLQSLSGALDYNSLHQSHLLPAIGQLGQLDELPSLKSMQHQLGMGSLGGSTRNLAGSPNEELTMQLLQQRAQQQSGGSPINLPQATGILRPLSSNINQGGSVPNLVGVIPGTAIGLSNMCSGGREFGSSSGLLSASGSLMQSSTVEAQNLNFGGSSGSSGCSFQASVLSSKTGGLEDLNPAKRVRTTYSALSHSSPDLGQSSRPAWLGSQEGLVHGDPVYSPHQLSLPRQDIVGGIGSSGRPAYMGSQSMGSLGMNFPLSLAVDAGAVRPSLTRGQSLTEQVAANRELKFPKEERGRDNLMCARLGGGMITNESSSEELLNYLKQSHEGLGFMEGDLVSDGYPVDNLYVK

SEQ ID NO: 21 - protein, 715 aa, Physcomitrella patens
MGGGYLSSTVNMGESRDGGSPAMATLQQQQKHQPLNPNHQNPRNRSNSSPTNCYSNTAWGAKPAKLDTPDEFPVGMRVLVVDDNPTCLMILEQMLVRCAYRVTTCGKATEALSMLREDIGKFDVVISDVDMPDMDGFKLLELVGLEMDLPVIMVSGNGETSAVMKGITHGACDYLLKPVRIEELRNIWQHVVRKKRREVKAVATKSVEEAGGCERPKRGGGADDADYTSSATDTTDSNWKLTKRRKGEFKDENEEDNEQENDDPSTLKRPRVVWSVELHQQFVSAVNQLGIDKAVPKRILELMGVQGLTRENVASHLQKYRLYLKRLSGVTSQQGNMSAHFGGSDPFCMMPPDMSLANGQLTPQALAKFHMLGRMNATNGIGFSGGGLDPGMNQMFLQDLPRPPQLNSMLRNNTGLLASVPNGLQHLEQLSEPHHVHVVNELEHYPSNTKVYPQLNGNLDVSVGPLGAANGNLASNPNSDTLLMHILHSRASQQGVGSPSTLPQPRCGLNPTHLLSNDINFAPVGSLPNLAGSLGPAVGLSAIPGSAGGRDLSPSVGGSGASLSSPLGSLVRRPLMAEEQSNPVNSTNGTYSMAHSGQSPKPSGDTLPTPLNEGLEQQQPLWALYQNPMNQLSHGPSQGFPHDSLQWSVLTENLSFGDMGQSLSAGLISQFSSQGQDNGIGFAPPSQRGSYTRQSVSFPASSALDGRMVRSSYEP

SEQ ID NO: 22 - protein, 664 aa, Arabidopsis thaliana
MVNPGHGRGPDSGTAAGGSNSDPFPANLRVLVVDDDPTCLMILERMLMTCLYRVTKCNRAESALSLLRKNKNGFDIVISDVHMPDMDGFKLLEHVGLEMDLPVIMMSADDSKSVVLKGVTHGAVDYLIKPVRIEALKNIWQHVVRKKRNEWNVSEHSGGSIEDTGGDRDRQQQHREDADNNSSSVNEGNGRSSRKRKEEEVDDQGDDKEDSSSLKKPRVVWSVELHQQFVAAVNQLGVDKAVPKKILEMMNVPGLTRENVASHLQKYRIYLRRLGGVSQHQGNMNHSFMTGQDQSFGPLSSLNGFDLQSLAVTGQLPPQSLAQLQAAGLGRPTLAKPGMSVSPLVDQRSIFNFENPKIRFGDGHGQTMNNGNLLHGVPTGSHMRLRPGQNVQSSGMMLPVADQLPRGGPSMLPSLGQQPILSSSVSRRSDLTGALAVRNSIPETNSRVLPTTHSVFNNFPADLPRSSFPLASAPGISVPVSVSYQEEVNSSDAKGGSSAATAGFGNPSYDIFNDFPQHQQHNKNISNKLNDWDLRNMGLVFSSNQDAATATATAAFSTSEAYSSSSTQRKRRETDATVVGEHGQNLQSPSRNLYHLNHVFMDGGSVRVKSERVAETVTCPPANTLFHEQYNQEDLMSAFLKQEGIPSVDNEFEFDGYSIDNIQV

SEQ ID NO: 23 - protein, 1036 aa, Arabidopsis halleri
LSKKQNEDASGRKEEDGKGNEHNGMESCTRMKRTVWTVELHQKFVNAFQQLGLDKASPEQIHALMNVEGLPVINVASHLQKYRLFLKKIYEGQQLDMATIQLLLSAGSHFPQTPWTNHCSSFIQQGHHQNSSNSSETYHTTLSPRVQKVNTFQPSSSPLKPLLFPKSNISAFKEDFKSIKEPAIVGDSSLDSSKPRNSFQTASKFPKTDPCTGSYIIEIMTEPYYGKSSRRHSNFSAYMGDFKSIKDPEIVQESRTRKNHGRVVWSHELHQKFLNAIDQLGGNEKAIPKKILAVMNVEGLTRLNVATHLQKYRQCCSAEAQQLNMATRKLPSSEHLPQSPSTNHHSSLSPRVQDVNIRLWSSSPKRQDQILVYVLFSFENDNGREETTCRRIASTMELGSTEDGRHDKFPVGMRVLAVDDNPTCLRKLEELLLRCKYHVTKTMESRKALELLRENSNMFDLVISDVEMPDTDGFKLLEIGLEMDLPVIMLSAHSDYDSVMKGIIHGACDYLVKPVGLKELQNIWHHVVKKNIKSYAKNIGPSRQLLPPSESNLVPSASKKRKEKASDSGDEDDSDREEDDGEGSEQDGEESGTRKKPRVVWSQELHQKFVSAVQQLGLDKAVPKKILDLMSIEGLTRENVASHLQKYRLYLKKIDEGQQQNMTPDAFGTRDSSYFQMAQLDGLRDFTATRQIPSSGLLSRSHLTKLQPPMYSSINLQGMNSSSFIQQGHHHNSSNSANPFGTYHTTLSPRIQNVNLLQRTSSPLETLQFPRSKSYIGDFKGIGDRAVGGSFLDSCMPFGSSSTSLPSASTNTLMLQANYTQPLHIASDGNQPCIEGTPSNSASPNISFQGLSRFPSHSWQGNLNTTRFPPSSLPLNQAFLPDQVTCAGNNLGDCTSLVSAGNPGGEMQCEPQLLGGFMQNMNPLDGQKWEQQNSMLNNPFGNIEYPLSADNMVFRDNNATRNKGLDESLMNPIDNSQEYVGKATTMLDPEMKSGKPENDNQHDVFDDIMNEMMKQEENNGMVSVATRFGFDSFPPP

SEQ ID NO: 24 - protein, 774 aa, Arabidopsis lyrata
MGDFKSIKEPEIVQESRTRKNHGRVVWSHELHQKFLHAIDQLGGNDKAIPKKILAVMNVEGLTRLNVATHLQKYRQCCSTEAQQLNMATRKLPSSEHLPQSPSTNHHSSLSPRVQDNDNGREETTCRRIASTMELGSTEDGRHDKFPVGMRVLAVDDNPTCLRKLEELLLRCKYHVTKTMESRKALELLRENSNMFDLVISDVEMPDTDGFKLLEIGLEMDLPVIMLSAHSDYDSVMKGIIHGACDYLVKPVGLKELQNIWHHVVKKNIKSYAKNIGPSRQLLPPSESNLVPSASKKRKEKANDSGDEDDSDREEDDGEGSEQDGDEAGTRKKPRVVWSQELHQKFVSAVQQLGLDKAVPKKILDLMSIEGLTRENVASHLQKYRLYLKKIDEGQQQNMTPDAFGTRDSSYFQMAQLDGLRDFTATRQIPSSGLLSRSHLTKLQPPMYSSINLQGMNSSSFIQQGHHHNSSNSANPFGTYHTTLSPRIQNVNLFQRTSSPLETLQFPRSKSYIGDFKGIGDRAVGGSFLDSCMPFGSSSTSLPSASTNTLMLQANYTQPLHISSDGNQPCIEGTPSNSASPNISFQGLSRFPSHSWQGNLNTTRFPPSSLPLNPAFLPDQVTCAGNNLGDCTSLVSAGNPGGEIQCEPQLLGGFMQNMNPLDGQKWEQQNCTMLNNPFGNIEYPLPADNMVFRDNNATRSKGLDESLMNPIDNSQEYVGKATTMLDPEMKSGKPENDNQHDVFDDLMNEMMKQEENNGMVSVATRFGFDSFPPP

SEQ ID NO: 25 - protein, 578 aa, Helianthus annuus
MTTGSSFGSGSLGCKQETGVPDQFPAGLRVLVVDDDVICLKILEQMLRRCSYHVTTCSQATAALNLLRERKGCFDVVLSDVHMPDMDGFKLLELVGLEMDLPVIMMSADGRTNLVLRGIRHGACDYLIKPIREEQLKNIWQHVIRKKWNENKEHEHSGSVDDKDRHKRGGDDNDYASSVNEGGDGILTSHKKKRHNNKEEDDGELETDEPGGSKKARVVWSVELHQQFVTAVNQLGIDKAVPKRILELMNVPGLTRENVASHLQKFRLYLKRLSGVAQQGGGPNSFCGSIDQNPKLASYARFEIQALAASGQIPPQTLVALHAELLGQPTANVGMPVLDHQPLMQPSKCGPVDHVMSYGQTLPSNVTKQVPQPAIEDVHSGLGAWHSNNMVGGYGQLGGQNWHNMLLGMLQSQSHQLQKQSITVQPSRLVVPSQSSNFQAVNNGVPVNQTTGFNNSTVINYAVGQRTERDVENQIGGQSSVSNISVKEMGEKQISFGESVHVLDQGSLRNLGFVGKKSSIPSRFAVYEAAESLTHNLNYGDNNGERRVKQEPNIEFLENSKAGAHRVSQNDLMSKQVR

SEQ ID NO: 26 - protein, 428 aa, Vitis vinifera
MAALLKVPPQSSGGTNGSCKADVVVSDQFPAGLRVLVVDDDVTCLKILEQMLRRCLYHVTTCSQATIALNILREKKGCFDIVLSDVHMPDMDGYKLLEHVGLEMDLPVIMMSADGRTSAVMRGIRHGACDYLIKPIREEELKNIWQHVVRKKWNENKEHEHSGSLEDNDRHKRGGEDAEYASSVNEGAEGILKGQKKRRDSKDEDDGELENEDPSTSKKPRVVWSVELHQQFVSAVNQLGIDKAVPKRILELMNVPGLTRENVASHLQKFRLYLKRLSGVAQQQGGIPNSFCGPVEPNVKLGSLGRFDIQALAASGQIPPQTLAALQAELLGRPTSNLVLPAMDQPALLQASLQGPKCIPVEHGVAFGQPLVKCQTNISKHFPPTVVSTEDVPSGFGAWPSNSLGTVGTSGSLGGLSAQNNNILMDMK

SEQ ID NO: 27 - protein, 659 aa, Amborella trichopoda
MANVQKLPHSSISTASSYGSCRGEGVPDQFPAGLRVLVVDDDTTCLRILEQMLRKCMYKVTTCCRATDALDTLRGSKGCFDVVISDVYMPDMDGFKLLEHVGLEMDLPVIMMSADARFSAVMKGIKHGACDYLIKPVRIEELKNIWQHVVRKKWNETKEHDQSGSIEDNERHKRGSDDAEYASSVNEGTDGNWKVQKKRKDSKEEEDDGEQENEDPSAAKKPRVVWSVELHQQFVNAVNQLGIDKAVPKRILELMNVQGLTRENVASHLQKFRLYLKRLSGHQAGVSSSFCGSVDPNSKLGPLSQLDIRALTASGQIPSQTLAALQAELLGRPSNNVAMPVYGQTLVKCQPNLPKQFPQPNLPVDDVQSSLSIWQHHLSSGMPLGGLNPQNNGLLMQQQQQLTIESNRPCNVQPSCHVAPSNGGFTMRNNPTSSNASSVEYNSLLSSQGDVGQISQASGSDLATTVQSNGGFKSLDYRNMGQVSLESTSDLVSTQNNGFKGMELRNVGSLGGYPLSSSVSAGSTKTENGQSFSQVRTGPRMSMGPTGQFVGPPTIRRLPMVDGGTHRNSLGFVGKGVSIPSRFMPDSGSPTGVGEECTLPKQEVDPDFFDSLKVGPVGVQHYASGDLMSVLSKQQQASTGNLDCEFGIDGYQLGNIHVK

SEQ ID NO: 28 - protein, 669 aa, Ricinus communis
MAALQRVASSVSATASNYSSCKGNGVVTATADVAVSDQFPAGLRVLVVDDDTTCLRILEQMLRRCLYHVTTCSQAKVALNLLRERKGCFDVVLSDVHMPDMDGFKLLEHVGLEMDLPVIMMSADGRTSAVMRGIRHGACDYLIKPIREEELKNIWQHVVRKKWHENKEIEHSGSLEDNDRHKRGNEDAEYTSSVNEGTEGVLKGQKRRSNSKDEDDGEPDSDDPSTSKKPRVVWSVELHQQFVSAVNQLGIDKAVPKRILELMNVPGLTRENVASHLQKFRLYLKRLSGVAQQGGISSTFCGPMDSNVKLNSLGRFDIQALAASGQIPPQTLAALHAELFGRPTGSLVTTMDQPTLLQASRQSPKCIPVEHGVTFGQPIVKCSSGISKHFPQNMVSVEEVSSGYGAWPSNSLGTVGPSTNLGGMTTQNGNMLMDIFHQQQKQQQPQQQQSLADPSRSINVQPSCLVVPSQSSACFQAGNSPASVNQSNFNRNVVIDYSLLSSQSNNSALNIGHIPEGDLKTTGAVNGYSAPGSLSPPASSCSVNADSGVPRQVQNPTLAFGAVRQLPALSPNIFNIQGSYGVRSDDILDQGPFFKNLGFVGKGTCIPSRFAVDEFETPSSNLSHGKLYVENNDNKVKQEPNIDFTDTSRVGIPVLQQYPPNDLMSVFTE

SEQ ID NO: 29 - protein, 654 aa, Solanum lycopersicum
MVSMSGEVATCKSEATVVTDHFPVGLRVLVVDDDVVCLRIIEQMLRRCKYSVTTCTQAMVALNLLREKRGTFDIVLSDVHMPDMDGFKLLELVGLEMDLPVIMMSGDGRTNLVMRGVQHGACDYLIKPIRDEELKNIWQHVVRKRYNSSKEPECSGSLDDNDRYRRRSDDAECASSVIEGADGVLKPQKKKREAKEDDTEMENDDPSTTKKPRVVWSVELHQQFVSAVNQLGIDKAVPKRILELMNVPGLTRENVASHLQKFRLYLKRLSGVVQQQGGLPSTFCGPIEQNSELGSLGRFDIQALAASGQIPPETLTALHAELLGRSTSNLVLPAVEQQNLVQVSLQQAKCIPVDQVMAYGQPLLKCPASISNSKHLSQAILSAEDVHSGFGSQRAKNICMVPSSNPIAPNSNMLTAMMQQQQWQKQQQIELQHRQSGPPEVNRSINVQPSCLVLPSQLPGHFQVGDSPASISRAGSLSKSSVIDYGVLSPQSNNSSGVVQVLDRELKPECGLNRLPSGGSLSRSCSINADNSVDLQLHNSSSAFGSSKQLPGLIPSHLGSPVPYCINSSLVLDQGRMKGASIPSRFAVDESDSPMCNFNTAKIYLEETKVKQEPNMNVMENAKVGPAIFQKFQPGDLMSVFRLSFARVKVSSSP

SEQ ID NO: 30 - protein, 653 aa, Solanum tuberosum
MSGDVATCKSEATVVTDHFPLGLRVLVVDDDVVCLRIIEQMLRRCKYSVTTCTQAMVALNLLREKRGTFDIVLSDVHMPDMDGFKLLELVGLEMDLPVIMMSGDGRTNLVMRGVQHGACDYLIKPIRDEELKNIWQHVVRKRYNSSKELECSGSLDDNDRYKRGSDDAECASSVIEGADGVLKPQKKKREAKEEDDTEMENDDPSTSKKPRVVWSVELHQQFVSAVNQLGIDKAVPKRILELMNVPGLTRENVASHLQENQKFRLYLKRLSGVVQQQGGLPSTFCGPIEQNSELGSLGRFDIQALAASGQIPPETLTALHAELLGRSTSNLVLPAVEIQNLLQASLQQAKCIPADQVMAYGQPLLKCHPSISNSKHLSQSILSAEDVHSGFGSQRAKNICLVPSSNPIGLAAPNSNMLMAMMQQQQWQKQQQMELQHRRSGPPEVNHSINVQPSCLVLPSQLPGNFQVGDSPASISRAGSLSKSSVIDYGVLSPQSNNSSGVVQVLDRELKPECGLNRLPSGGSLSRSCSINADNSVGLQLHNSSSAFGSSKQLPALIPNHLGSPVPYYINSSQVLDQGHTRNPGVGKCASIPSRFAVDESDSPMCNFNTAKNYLEETKVKQEPNMNVMENAKVGPAIFQKFQPGDLMSVFSD

SEQ ID NO: 31 - protein, 669 aa, Gossypium hirsutum
MATMHRVVQSSVSTSDATTTSYDGLTSCKAADIVISDQFPAGLRVLVVDDDITCLKILEKMLHRCRYHVTTCPQAKVALNLLRERKGCFDVILSDVYMPDMDGYKLLEHVGLEMDLPVIMMSADGSTRAVMKGIRHGACDYLIKPIREEELKNIWQHVVRKKWNENKELEHSGSLDDTDQHKQRHDDAEYASSVNDATETSLKPLKKRSNSKEEDDGEIDNDDPSTSKKPRVVWSVELHQQFVSAVNQLGIDKAVPKRILELMNVPGLTRENVASHLQKFRLYLKRISGVAQQGGIANPLCGPVEANVKIGSLGSFNIQALAASGQIPPQTLAAVHAELLGRSAGNLVVATDQPALLQATPQGAKCIQVDQGVAFVQHSVKSESSSSKHFSQSFAPVEDVASGFRSWPSNNIGTAGPSNSGGLSSQNGNMLIDLLQQQQQLQKPQQRSTVSELRRSINVQPSCHVVPSQSSASFRAGNSPVSVTQNGSYSRTAVIDYSLLSSQSNCPSLNIGQVSDVNLQTTGVLSGYIPPASVSPSVSSCSVNADNCASQQVQTSSMTFKASRHLPGFVHSTSNIPDPYGSTKSGDLLNQEPFNNLGYINKGTCLPAKFAVDEFQSHLSSSSHGKVFSENIGTRVKQEPSMEFGDNAKVGIPMLQQFRPNDLMSVFTE

SEQ ID NO: 32 - protein, 681 aa, Theobroma cacao
MNSSSGKGSMSAASSSAAWKAGDVVPDQFPAGLRVLVVDDDPTCLMILEKMLRTCLYEVTKCNRAETALSLLRENKNGFDIVISDVHMPDMDGFKLLEHIGLEMDLPVIMMSADDGKHVVMKGVTHGACDYLIKPVRIEALKNIWQHVVRKRKNEWKDFEQSGSVEEGDRQPKQSEEADYSSSANEGNWKSSKKRKDDDDEAEERDDTSTLKKPRVVWSVELHQQFVAAVNQLGIDKAVPKKILELMNVPGLTRENVASHLQKYRLYLRRLSGVSQHQSNLNNSFMSPQEATFGPLSPLNGLDLQTLAATGQLPAQSLATFQAAGLGRSTAKSGIAMPLVDQRNIFSFENPKLRFGEGQQQHMNNNKQLNLLHGIPTTMEPKQLASLHHSAQSIGNINMQVTSHGVQGSQNNSLLIQMAQPQPRGQILNDSTGSHAPRLPSTLGQPILSNGIAANVSTRNGIPENIRGPGYNPVSQTSSLLNFPMNHTSELPGNSFPLGTTPGISSLTSKGAFQEDINSDVKGSGGFMPSYDIFNDLNQHKPQNWELQNVGMTFDASQHSNSLQGNLDLAQSILVQQGFSSGQMNGQNRSAAVVSKAMFSAGDCTEQGNAQNVNHHLNNLLVDNTIRIKSERVADAGPANLFPDHFGQEDLMSALLKQQDGIAPAENEFDFDGYSMDNIPV

SEQ ID NO: 33 - protein, 579 aa, Phaseolus vulgaris
MNLSNGKGSMSTVTTTAVMKSGDAVSDQFPAGLRVLVVDDDPTCLMILEKMLRTCLYEVTKCNRAETALSLLRENKNGFDIVSANEGSWRNSKKRRDEEEEAEDRDDTSTLKKPRVVWSVELHQQFVAAVDQLGIDKAVPKKILELMNVPGLTRENVASHLQKYRLYLRRLSGVSQHQNNLNNSFLGSQEATFGTISSINGIDLQTLAVTGQLPAQSLATLQAAGLGRSTAKTGVPMPLMDQRNLFSFENPRVRFGEGQQQHLSSSKPMNLLLGIPTNMEPKQLANLHQSTQSIASLNMRVNASATQGNPLMMQMPQSQPRGQMLSENTGPRVPRLPSSLGQPTVSNGISNGFLGRNGIAGNNRGPAYNPVPPNSSLLSFPMNQSSEVSVNNSLPLGSSPGISSITTKGSFQEEVTSGIKATGGFPSYDIFNELHHQKSHDWEITNPSLTYSASHHANPLQGNIDVSPSVLVHQGFSSTQQNGQSRDATLIGKAMFSLGEGSEQDNLQNAVQHLHPLLVDNSIRVKAERIPDASSQTNLFPDHYVQEDLMSALLKQQEGMGPAESEFEFDAYSLDNIPV

SEQ ID NO: 34 - protein, 679 aa, Glycine max
MNLSNGKGSMSTLTASVVMKSGDAVSDQFPAGLRVLVVDDDPTCLMILEKMLRTCLYEVTKCNRAETALSLLRENKNGFDIVISDVHMPDMDGFKLLEHIGLEMDLPVIMMSADDGKSVVMKGVTHGACDYLIKPVRIEALKNIWQHVVRKRKNEWKDAEQSGSAEEGDRQPKASDEADYSSSANEGSWRNSKKRRDEEEEAEDRDDTSTLKKPRVVWSVELHQQFVAAVDQLGIDKAVPKKILELMNVPGLTRENVASHLQKYRLYLRRLSGVSQHQNNMNNSFLSPQEATFGTISSINGIDLQTLAVAGQLPAQSLATLQAAGLGRPTGKAGVPMPLMDQRNLFSFENPRLRFGEGQQQHLSTSKPMNLLHGIPTNMEPKQLANLHQSTQSIGSLNMRVNASATQGSPLLMQMAQSQPRGQMLSENIGPRVPRLPSSLGQPTVSNGISNGLLGRNGIAGNNRGPAYNPVPPSSSLLSFPMNQTSEMSVNNSFPLGSTPGISSITTKGSFQEEVTSGIKGSGGFPSYDIFNELHHQKPHDWEITNPNLTYNASQHANPLQGNIDVTPSVLVHQGFSSTQQTGQSRDAALIGKAMFSMGEGLEQNNFQNASQNLNSLLLDNSIRVKAERIPDASSQTNLFPEHYGQEDLMSALLKQQEGMGPSENEFDFDGYSLDNIPV

SEQ ID NO: 35 - protein, 668 aa, Chenopodium quinoa
MNLGGGLMGSMAMPSSTVSRKSSEVVTADQFPVGLRVLVVDDDPTCLTILEKMLRTCRYEVTKTNRAEHALNMLRENKNGFDVVISDVHMPDMDGFKLLEQVGLEMDLPVIMMSADDSKQVVMKGVTHGACDYLIKPVRIEALKNIWQHVVRKKKYEYNKDVEQSGSWDEGDRQLKHDDAVSSPANDGSWKNSKRKSGEDDEADDKDDTTTLKKPRVVWSVELHQQFVAAVNQLGIDKAVPKKILELMNVPGLTRENVASHLQKYRLYLRRLSGVSQHQGGLNSSFMPQDPSFSTMSSLGGIDLQTLAATGQLSAQTLAAYTRLPPTIKPGISMPFVDQRNLFSFENSKLRYGDGQQSQISNVSKQMNLLHGFPTTMEPKQLAVLNQSAQTLGSMNMQANASSSHQSSSLLMQQMVPQQRGHISNESISSQVPRIQPSVGQPLQSNGNANAVLSRNGIPYDPVNQSASVVDFSVNHIPELPGNSFPLGSTPGITSITSKGFNQEEIGSDIKVSRGFVGSYDMFSELQHKPQEWQMQNPNMGFAGSSQHVPSVQSGVNVAPSIMVNQSYVSGQKNEQNGHSMAGKPMYSAGLENQHMGMQNVNQNYNSIHVNNSSRVKAESVSDVVNLGANLFDYSPEDMLSTIMLKQQEGIGSGDFDFDGYTLDNIPV

SEQ ID NO: 36 - protein, 670 aa, Malus domestica
  MOD_RES (195)..(195): Any amino acid
  MOD_RES (215)..(215): Any amino acid
  MOD_RES (530)..(530): Any amino acid
  MOD_RES (540)..(540): Any amino acid
  MOD_RES (579)..(579): Any amino acid
MAALQRVAQSSVSTTASSYGSCKVGGGVLSPSAGIEMAVPNQFPAGLRVLVVDDDTTCLRILELMLLRCLYQVTTCSEATVALNLLRERKDCFDVVLSDVHMPDMDGFKLLEHVGLEMDLPVIMMSADGRTSVVMRGIRHGACDFLIKPISEAELKNIWQHVVRKKWNGSKELEHSGSLEDNDPHKRGNNDFEYXSSVNEGTEVSLKGHKKRINXKEDDDGDTENDDLSTSKKPRVVWSVELHQQFVTAVNQLGLDKAVPKRILELMNVPGLTRENVASHLQKFRLYLKRLSGVAQQQSGIANPLCGPVDSNGKLGSLSRFDFQALAASGQIPPQTLAALQAELLGQPAGNLVPAMDQPALLHASLQAPKRPPVEHGVPFMQPFVKSQSNVSKHFPQSVISAEDASLGFGQWRSNSRSTVAPSNDHGGLSTQNSNLLMGIVPQEQRQHKRTQQQSVLTEPSRSFNVQPSCLVVPSQSSTGFQAGNSPASVNQSSSFNRSTVVDYSLPSDQSNNSLNVGHIPTGNPKTSGXLGGYSGPGSXCATSCLVNADNSTSYQNSTATFSDSRELPGFLHNTANSXGFYVDKSGEMLDQGPLRNLGFVGKETCIPSRFAVDDFESQMSNLNPGRIHVESSGTLVKQEPSEDYVDNAKLGIPILHQYSSSDFMSPFAD

SEQ ID NO: 37 - protein, 802 aa, Zea mays
PYPTHTLLPQPHLSLSACVLLVLLSLSSPALTSPPFPAVSWISRIQTTALVSLPSCLLPAYVQEGPCLGDPGAWFLGSAASAAVGFAEPEPPEMTVDELKLQARASGGHGAKDQFPVGMRVLAVDDDPTCLKILENLLLRCQYHVTTTGQAATALKLLREKKDQFDLVISDVHMPDMDGFKLLELVGLEMDLPVIMLSANGETQTVMKGITHGACDYLLKPVRIEQLRTIWQHVVRRRSCDAKNSGNDNDDSGKKLQVVSAEGDNGGVNRNKRISRKGRDDNGDDGDDSDDNSNENGDSSSQKKPRVVWSVELHRKFVAAVNQLGIDKAVPKKILDLMNVENITRENVASHLQKYRLYLKRLSADASRQANLTAAFGGRNPAYVNMGLDAFRQYNAYGRYRPVPTTNHSQPNNLLARMNSPAFGMHGLLPSQPLQIGHNQNNLSTSLGNVGGMNNGNLIRGAHMPLQDTSKCFPTGPSGNSFANISNSTQLVTTNNLPLQSLEPSNQQHLGRLHSSADPFNSFVGEPPQFADLGRCNTTWPTAVSSSNVQEIGQKDRIVNRPKLEPLSSFTEASSQIPLLGNEMQSHQVASLASNGLPMPFTQEAVPFAYGSSTNSREMLNNNLALSNSGVNSTLPNLRIDGSVVPGQTLGGSNSGGCVVPPLQDGRIDHQAVSSHLNYNNELMGTGRLQRGLSGGLDDIVVDMFRPDRADDGVSFIDGDWELRPGSSVTSEYQLCGICYLNSYDYVFKSGVNCGYRDIQHVYEPRNDVLFPLGNRFAVPFVDCHCIVASLAETEVKGKDQA

SEQ ID NO: 38 - protein, 591 aa, Brassica rapa
MLNPGVVGGSSNSDPFPSGLRVLVVDDDPTCLMILERMLKTCLYRVTKCNRAEIALSLLRKNKNGFDIVISDVHMPDMNGFKLLEHVGLEMDLPVIMMSADDSKSVVLKGVTHGAVDYLIKPVRIEALKNIWQHVVRKKQNVSEHSGSVEETGGDRQQQQRGDDDDDGNNSSSGNNEGNLRKRKEEEQGDDKEDTSSLKKPRVVWSVELHQQFVAAVNHLGVDKAVPKKILEMMNVQGLTRENVASHLQKYRIYLKRLGGVSQGNMNHSFLTGQDPSYGPLNGFDLQGLATAGQLQAQSLAQLQAVGLGQSSSPLIKPGITSVDQRSFFTFQNSKSRFGDGHGPMMMNGGGGNKQTSLLHGVPTGHMRLQQQQMAGMRVAGPSMQQQQQQSMLSRRSVPETRSSRVLPAATHSALNNSFPLASAPGMMSVSDTKGVNEFCNPSYDILNNFPQQQHHNNNNNRVNEWDLRNVGMVFNSHQDNTTSAAFSTSEAYSSSSTHKRKREAELVVEHGQNQQQPQSRSVKPMNQTYMDGGGSVRMKTETVTCPPQATTMFHEQYSNQDDLLSDLLKQEGLLDTEFDFEGYSFDSILV

SEQ ID NO: 39 - protein, 691 aa, Oryza sativa
MAPVEDGGGVEFPVGMKVLVVDDDPTCLAVLKRMLLECRYDATTCSQATRALTMLRENRRGFDVIISDVHMPDMDGFRLLELVGLEMDLPVIMMSADSRTDIVMKGIKHGACDYLIKPVRMEELKNIWQHVIRKKFNENKEHEHSGSLDDTDRTRPTNNDNEYASSANDGAEGSWKSQKKKRDKDDDDGELESGDPSSTSKKPRVVWSVELHQQFVNAVNHLGIDKAVPKKILELMNVPGLTRENVASHLQKFRLYLKRIAQHHAGIANPFCPPASSGKVGSLGGLDFQALAASGQIPPQALAALQDELLGRPTNSLVLPGRDQSSLRLAAVKGNKPHGEREIAFGQPIYKCQNNAYGAFPQSSPAVGGMPSFSAWPNNKLGMADSTGTLGGMSNSQNSNIVLHELQQQPDAMLSGTLHSLDVKPSGIVMPSQSLNTFSASEGLSPNQNTLMIPAQSSGFLAAMPPSMKHEPVLATSQPSSSLLGGIDLVNQASTSQPLISAHGGGNLSGLVNRNPNVVPSQGISTFHTPNNPYLVSPNSMGMGSKQPPGVLKTENSDALNHSYGYLGGSNPPMDSGLLSSQSKNTQFGLLGQDDITGSWSPLPNVDSYGNTVGLSHPGSSSSSFQSSNVALGKLPDQGRGKNHGFVGKGTCIPSRFAVDEIESPTNNLSHSIGSSGDIMSPDIFGFSGQM

SEQ ID NO: 40 - protein, 428 aa, Oocystis sp.
MALKRVPSFSGRPNFPAGLQILVVDSDSSSREAVEMQLKSHSYLATCCCTCGEAVEQLGTSKYDIVLAESKLVAAECVDSTRLCEAARALPLVLMCEDSTADDVLKGIRLGACDFLEKPLSPLKLKNIWQHVVRKMMEQMHVRRTDDADTCTTKSSRDQSCAIKGKSVASTPSCPKTPSPAASGADIGCSIATSVSKAGDVVGESSSSETRKEHCSETTECSDLKSCAAKSAVSAQTPVSTATVAATWGASKKKSTASATTSSVSNRPPLAIKMPAPAVAYTSGLAPFPPPMFVPGGWGQSSNPCVVGTPMMPPPPGMGMPPHHHAPYGQVPPPGYPVACMPSAFVPTPMGPGGVAFAPPPGASCTSAAYYPHPAVDASASATATFTGHVQIDLTNVSAEEPAPIGLALRKTASLLDLVSDRLGQRAC

SEQ ID NO: 41 - protein, 341 aa, Tetraselmis sp.
MLCPAVQVATMATVLASTHFSERPSFPADLEVLLLDSATQGAETASKLLLSCSYRVTVCRSVSEALSHMACKAFDVVLVEQKLFSGRDAAAAQLKALAGVIPTVVLSDSGSAKDTWAAIVGQAADVLIRPLTKQKLQTLWQHTVRMQRAASSASAATSMVAKPVAVLSSALKPAASSASLDKGQKRKLKDHMMGPIMAHPQVSNPGFIWGAPVMGVPAGQQAPQKSEAPVTPQKPGSEMHPELDATSHIAMGSSDNFNVPVYESGTDSQESQPTCDPTSLDDINEDDYAFIDFALSDSFPTVEEDEILPPIGLSLKKSSSLLNMLNGVLLSAHSVPLQLPQ

SEQ ID NO: 42 - protein, 558 aa, Arabidopsis thaliana
MSSSEEVVEVTVVKAPEAGGGKLSRRKIRKKDAGVDGLVKWERFLPKIALRVLLVEADDSTRQIIAALLRKCSYRVAAVPDGLKAWEMLKGKPESVDLILTEVDLPSISGYALLTLIMEHDICKNIPVIMMSTQDSVNTVYKCMLKGAADYLVKPLRRNELRNLWQHVWRRQTSLAPDSFPWNESVGQQKAEGASANNSNGKRDDHVVIGNGGDAQSSCTRPEMEGESADVEVSARDAVQMECAKSQFNETQLLANELQSKQAEAIDFMGASFRRTGRRNREESVAQYESRIELDLSLRRPNASENQSSGDRPSLHPSSASAFTRYVHRPLQTQCSASPVVPDQRKNVAASQDDNIVLMNQYNTSEPPPNAPRRNDTSFYTGTDSPGPPFSNQMNSWPGQGSYPTPTPINNIQFRGPNTAYTSAMAPASLSPSPSSVSPHEYSSMFHPFNSKPEGLQDRDCSMDVDDRRYVSSATEHSAIGNHIDQLIEKKNEDGYSSSVGKIQQSLQREAALTKFRMKRKDRCFEKKVRYESRKKLAEQRPRIKGQFVRQVQSTQAP

SEQ ID NO: 43 - protein, 186 aa, Arabidopsis thaliana
MAEVMLPRKMEILNHSSKFGSPDPLHVLAVDDSHVDRKFIERLLRVSSCKVTVVDSATRALQYLGLDVEEKSVGFEDLKVNLIMTDYSMPGMTGYELLKKIKESSAFREVPVVIMSSENILPRIDRCLEEGAEDFLLKPVKLSDVKRLRDSLMKVEDLSFTKSIQKRELETENVYPVHSQLKRAKI

SEQ ID NO: 44 - protein, 727 aa, Arabidopsis thaliana
MNANEEGEGSRYPITDRKTGETKFDRVESRTEKHSEEEKTNGITMDVRNGSSGGLQIPLSQQTAATVCWERFLHVRTIRVLLVENDDCTRYIVTALLRNCSYEVVEASNGIQAWKVLEDLNNHIDIVLTEVIMPYLSGIGLLCKILNHKSRRNIPVIMMSSHDSMGLVFKCLSKGAVDFLVKPIRKNELKILWQHVWRRCQSSSGSGSESGTHQTQKSVKSKSIKKSDQDSGSSDENENGSIGLNASDGSSDGSGAQSSWTKKAVDVDDSPRAVSLWDRVDSTCAQVVHSNPEFPSNQLVAPPAEKETQEHDDKFEDVTMGRDLEISIRRNCDLALEPKDEPLSKTTGIMRQDNSFEKSSSKWKMKVGKGPLDLSSESPSSKQMHEDGGSSFKAMSSHLQDNREPEAPNTHLKTLDTNEASVKISEELMHVEHSSKRHRGTKDDGTLVRDDRNVLRRSEGSAFSRYNPASNANKISGGNLGSTSLQDNNSQDLIKKTEAAYDCHSNMNESLPHNHRSHVGSNNFDMSSTTENNAFTKPGAPKVSSAGSSSVKHSSFQPLPCDHHNNHASYNLVHVAERKKLPPQCGSSNVYNETIEGNNNTVNYSVNGSVSGSGHGSNGPYGSSNGMNAGGMNMGSDNGAGKNGNGDGSGSGSGSGSGNLADENKISQREAALTKFRQKRKERCFRKKVRYQSRKKLAEQRPRVRGQFVRKTAAATDDNDIKNIEDS

SEQ ID NO: 45 - protein, 444 aa, Arabidopsis thaliana
MGEIVVLSSDDGMETIKNRVKSSEVVQWEKYLPKTVLRVLLVESDYSTRQIITALLRKCCYKVVAVSDGLAAWEVLKEKSHNIDLILTELDLPSISGFALLALVMEHEACKNIPVIMMSSQDSIKMVLKCMLRGAADYLIKPMRKNELKNLWQHVWRRLTLRDDPTAHAQSLPASQHNLEDTDETCEDSRYHSDQGSGAQAINYNGHNKLMENGKSVDERDEFKETFDVTMDLIGGIDKRPDSIYKDKSRDECVGPELGLSLKRSCSVSFENQDESKHQKLSLSDASAFSRFEESKSAEKAVVALEESTSGEPKTPTESHEKLRKVTSDQGSATTSSNQENIGSSSVSFRNQVLQSTVTNQKQDSPIPVESNREKAASKEVEAGSQSTNEGIAGQSSSTEKPKEEESAKQRWSRSQREAALMKFRLKRKDRCFDKKVRDTQASS

SEQ ID NO: 46 - protein, 204 aa, Arabidopsis thaliana
MALRDLSSSSSSPELHVLAVDDSFVDRKVLERLLKISACKVTTVESGTRALQYLGLDGDNGSSGLKDLKVNLIVTDYSMPGLTGYELLKKIKESSALREIPVVIMSSENIQPRIEQCMIEGAEEFLLKPVKLADVKRLKELIMRGGEAEEGKTKKLSPKRILQNDIDSSPSSSSSTSSSSSSHDVSSLDDDTPSSKRIKLESRG

SEQ ID NO: 47 - protein, 691 aa, Glycine max
MGEVVIMSGEKKSVRVEGVEKEDSGGSGSKAGEFKGLMRWEKFLPKMVLRVLLVEADDSTRQIIAALLRKCSYKVVAVPDGLKAWELLKGRPHNVDLILTEVDLPSISGYALLTLIMEHEICKNIPVIMMSSQDSISTVYKCMLRGAADYLVKPIRKNELRNLWQHVWRRQSSTTGINGLQDESVAQQKVEATAENNAASNRSSGDAACIQRNIELIEKGSDAQSSCTKPDCEAESDPVGNMQEFSLLKCGEAYPSGTETQQVETSFRLGQTLMMHDCHAGGLNVSIRKNGEASTTNDKDTDTEHFGNASISGEAHDNPYVQINSSKEAMDLIGAFHTHPNCSLKNSTVNCTGNFDHSPQLDLSLRRSCPGSFENKLTEERHTLMHSNASAFKRYTTRQLQISMPAVLINFSDQQREQITNCEKNISHIATGSNSDSSTPMQRCIVSPTTVQSKESELATSHPPQGHSLPIPVKGVRFNDLCTAYGSVLPSVFHTQSGPPAMPSPNSVVLLEPNFQVNAFYQSNMKESSSEQLYESRGPNGNTTQNHIVYTQEHKSEHAEDRGHISPTTDQSVSSSFCNGNASHLNSIGYGSNCGSSSNVDQVNTVWAASEGKHEDLTNNANSHRSIQREAALNKFRLKRKERCYEKKVRYESRKKLAEQRPRVKGQFVRQVHPDPLVAEKDGKEYDHSDF

SEQ ID NO: 48 - protein, 747 aa, Vitis vinifera
MGEVVVSSEAGGGGMEGEVEKKEVGSGVVRWERFLPRMVLRVLLVEADDSTRQIIAALLRKCSYKVAAVPDGLKAWEVLKARPHNIDLILTEVELPSISGFALLTLVMEHEICKNIPVIMMSSHGSINTVYKCMLRGAADFLVKPVRRNELKNLWQHVWRRQSSTVSGNGPQDESVAQQKVEATSENNPTSNHSSDHVACIQKNKEALNKVSDAQSSCSKPDLEAESAYMETMQDFSNPTWSRSLVSDTKMQKNEECAKLGPKFLMHNKEAGGTLEAACRDVNTMTQPEAVEPENDGQGANAPSEACGNNAILGSSSREAIDLIGVFDNSKKCTYGNSSSNNGTKKSDSIPQLDLSLRRSHPSSPENQVADERHTLNHSNGSAFSRYINRSLQPPHLPSTGVFNQQKNFGADSDKRLSQLVTGYNSDITSPTLSTQRSVISLATSPSGRVEIALCGPQQRAFPAPVPQNANNSTSQTNHKPEHKLDSLEGQGHFSPATDQNSSSSFGNGGASNLNSFGCGSICGSNGNANTVAVVQAAAEGKNEEGIFSHEGHSQRSIQREAALTKFRLKRKDRCFEKKVRYESRKKLAEQRPRVKGQFVRQVHTIPPPAEPDTYYGSSFDVQPQRSRYLSAQPLRASSSQLLYPTHTPLQESKYEGHEESNLLTASLVGTALPVAPSFGYEVGRDQTAGKLVLSLKLDGRVRWKVGTWVSGRYRLNVNCVAVMAFGPSIPSGPLSSKEGTQCSTTV

SEQ ID NO: 49 - protein, 799 aa, Theobroma cacao
MGIVQMNNNGPVANGLVELNTHIHDEHKKIRGGVIGEGQGLSVEEESWINEDVEDRNDGKTELVQVQGHAHGEQERSQQQPQGPLVHWERFLPLRSLKVLLVENDDSTRHVVCALLRNCGFEVTAVSNGLQAWKILEDLTNHIDLVLTEVVMPCLSGIGLLCKIMSHKTRMNIPVIMMSSHDSMSTVFRCLSKGAVDFLVKPIRKNELKNLWQHVWRKCHSSSSSGGQSGTQTQKSSKSKGTDSDNNTGSNDEDDNGSVGLNVQDGSDNGSGTQSSWTKRAVEVDSSQPISPWDQLADPPHSTCAQVIHSRHEVLGDSWVPVTATREYDELDNELENVVMGKDLEIGVPKITASQLEDPSEKVMTNIAGVNKDKLSAINPKKDDEKLEKAQLELNSEKSGGDLRNQAADLIGVITNNTEPHIESAVFDIPNGLPKVSDAKEKVNYDTKEMPFLELSLKRLRDVGDTGTSAHERNVLRHSDLSAFSRYNSGSTANQAPTGNVGSCSPLDNSSEAVKTDSMKNFQSTSNSIPPKQQSNGSSNNNDMGSTTNNAFSKPAVLSDKPAPKTSAKSFHPSSAFQPVQSGHGSALQPVAQGKADAALGNMILVKARGTDQQGKVQHHHHHYHHHHHHHVHNMLPNQKLGNHDDLSLENMAAAAPQCGSSNLSSLPHVEGNAANHSLTRSASGSNHGSNGQNGSSTVLNTRGMNLESENGVPGKGGAGGGIGSGGRNVVDQNRFAQREAALNKFRQKRKERCFEKKVRYQSRKKLAEQRPRIRGQFVRQISTTGKEAFRFRGAGLCT

SEQ ID NO: 50 - protein, 742 aa, Oryza sativa
MMGTAHHNQTAGSALGVGVGDANDAVPGAGGGGYSDPDGGPISGVQRPPQVCWERFIQKKTIKVLLVDSDDSTRQVVSALLRHCMYEVIPAENGQQAWTYLEDMQNSIDLVLTEVVMPGVSGISLLSRIMNHNICKNIPVIMMSSNDAMGTVFKCLSKGAVDFLVKPIRKNELKNLWQHVWRRCHSSSGSGSESGIQTQKCAKSKSGDESNNNNGSNDDDDDDGVIMGLNARDGSDNGSGTQAQSSWTKRAVEIDSPQAMSPDQLADPPDSTCAQVIHLKSDICSNRWLPCTSNKNSKKQKETNDDFKGKDLEIGSPRNLNTAYQSSPNERSIKPTDRRNEYPLQNNSKEAAMENLEESSVRAADLIGSMAKNMDAQQAARAANAPNCSSKVPEGKDKNRDNIMPSLELSLKRSRSTGDGANAIQEEQRNVLRRSDLSAFTRYHTPVASNQGGTGFMGSCSLHDNSSEAMKTDSAYNMKSNSDAAPIKQGSNGSSNNNDMGSTTKNVVTKPSTNKERVMSPSAVKANGHTSAFHPAQHWTSPANTTGKEKTDEVANNAAKRAQPGEVQSNLVQHPRPILHYVHFDVSRENGGSGAPQCGSSNVFDPPVEGHAANYGVNGSNSGSNNGSNGQNGSTTAVNAERPNMEIANGTINKSGPGGGNGSGSGSGNDMYLKRFTQREHRVAAVIKFRQKRKERNFGKKVRYQSRKRLAEQRPRVRGQFVRQAVQDQQQQGGGREAAADR

SEQ ID NO: 51 - protein, 766 aa, Zea mays
MGSACQAGTDGPSRKDVLGIGNAALENGHHQAEADADEWREKEEDLANNGHSAPPPGMQQVDEHKEEQRQSIHWERFLPVKTLRVLLVENDDSTRQVVSALLRKCCYEVIPAENGLHAWRYLEDLQNNIDLVLTEVFMPCLSGIGLLSKITSHKICKDIPVIMMSTNDSMSMVFKCLSKGAVDFLVKPLRKNELKNLWQHVWRRCHSSSGSESGIQTQKCAKLNTGDEYENGSDSNHDDEENDDGDDDDFSVGLNARDGSDNGSGTQSSWTKRAVEIDSPQPISPDQLVDPPDSTCAQVIHPRSEICSNKWLPTANKRNVKKQKENKDESMGRYLGIGAPRNSSAEYQSSLNDVSVNPIEKGHENHMSKCKSKKETMAEDDCTNMPSATNAETADLISSIARNTEGQQAVQAVDAPDGPSKMANGNDKNHDSHIEVTPHELGLKRSRTNGATAEIHDERNILKRSDQSAFTRYHTSVASNQGGARYGESSSPQDNSSEAMKTDSTCKMKSNSDAAPIKQGSNGSSNNDVGSSTKNVAARPSGDRERVASPLAIKSTQHASAFHTIQNQTSPANLIGEDKADEGISNTVKMSHPTEVPQGCVQHHHHVHYYLHVMTQKQPSTDRGSSDVHCGSSNVFDPPVEGHAANYSVNGGVSVGHNGCNGQNGSSAVPNIARPNIESINGTMSQNIAGGGIVSGSGSGNDMYQNRFLQREAALNKFRLKRKDRNFGKKVRYQSRKRLAEQRPRVRGQFVRQSEQEDQTAQGSER

SEQ ID NO: 52 - protein, 917 aa, Physcomitrella patens
MTADLCEFESESDPLQPLSAVGRAWVEPIVGTPVGAEWRIKGGFKAHKEVDRSREQVGSKRVDDREKNSGRLENGCRFADRTGGAVLKAREDPKDIAEQIRRELDHQFPVNDVLRTSESDEDGRREDSAEDHYEEGDAVAAVVFEKQRPREIAQTREQQQGGNAAAAAAGTQGGGGWESFLLKRNLKVLLVEDDDATRHVVGALLRNCNYEVTPVANGSLAWGLLEEANSNFDLVLTDVVMPYLSGVGLLSKMMKREACKRVPIVIMSSYDSLGIVFRCLSKGACDYLVKPVRKNELKNLWQHVWRKCHSSSGSRSGSGSQTGEVAKPRSRGVAAADNPSGSNDGNGSSDGSDNGSSRVNAQGGSDNGSGNQACMQPVQVLRNSAIPEAVDGDEEGQATSQDKGADLDGEMGHDLEMATRRSACVTTGKDQQPEDAQKQDEDAVCILQDAGPSPDGANAESPSSSGRNDAAEESSPKIIDLINVIACQPQTQDAEPQESENDDEELDPRGRSSPKNNSASDSGTSLELSLKRPRSAVGNGGELEERQPLRHSGGSAFSRYGSGGTIIQQYHQTGGSLPLSGYPVSGGYGVYGMSGGSPGGSLRLGMGMDRSGSSKGSVEGTTPPPSHPQSMEKVGGQDGYGNARQTTEDAMIVPGMPMAIPLPPPGMLAYDGVIGTYGPAMHPMYYAHPSAWMAAPSRHMGERGDVYNQSPAFQEQDSGSGNHSQAGQTHQHMHHHQGNQHHHHHHHHHHGSGAQPSGNAGVQDEQQQSVVPPGSSAPRCGSTGVDGRSGSSNGYGSTGNGNGSMNGSASGSNTGVNNGQSGFGATPMLTDNSGSNGVGGTDAAMDGVSGGNGLCTEQMRFARREAALNKFRQKRKERCFEKKVRYQSRKRLAEQRPRVRGQFVRQAVHDPSAGDAE

SEQ ID NO: 53 - protein, 1359 aa, Volvox carteri
MEFHVLLVEDDRVTLKTVEQLLRKCNYKVTCAANGREAIKVLTACRHSGVKVDLILTDILMPEVTGFDLINEVVHGDTFCDVPVVVMSSQDSQENVLQAFQAGAADYLIKPIRKNELATLWQHVWRANKAKGSGSGTTTNVTGQPLSGREDLEAGEAVAVAAAAAAASGKACAATHGHLKDSSGGSSGAAASVLQSTGGTLLPDRAATVRYPAAAAAPPPPGASELSGNVTAGEAQGSRTQHLRHLSGLAGMESTAATSAAAQGSSAAGPLRGCGGAGTAIAGGPRAPLGPLSFAPFGTSVAVHFDLNPASGAARRLVNSSGAIDASTGSGTAGVAASSRCAAGTSATVISWSHVDPTETDPAEAEPMYDTNADATAAKAAADGVAEADDDDVGDDGGAGPNHNDDDDEGGGDDDVSGDGDEDGNRPRKRPRLLQGSSHHHSHQHRLHSLGGTTTNTTTTTTAAKPKSTAGERGGAAALLACRTAAAAPLRGSGCATAGATGACRLAAAAAAAEGSQGSRAASASAGPDGGARESTATPSGDTFAESPSAYTATATTTSTATTSTTTGSGIEMQDDEQQQRQQPKQRPPASQPELEGHHHQQQYHHYYRRTSLEGGCANAPPLPVPSSARGASPAGTGPTESGSGRDSGCARITNGTAAGATAAMPPSHVSSASPPRCTATSAAATRGSSGAATAAAGAMTTALATAGSYPRGVDASPPPNRSMGSSGGDGGGTAAAAAGTARGSSPAAATPPLPPSTQQHGLPHPAAAPPPGAASPGGAVTLPPALQELAALGAARHAGLWTQRALLHQQQLLLQQQKQQKQQQHQQDQVVGAEKIHGGSTSAVANAAEQQQQQPLGAAAARRPSKAGVDGTEAGSGAVGGCASATAAVMAMEASEPHGAVGSSFTAADRQETPLQPLHAESAAAGGDMDGNRSTPATMPSGPTAAASGPSQTSNSLTVLRHSDRSAFTAFTVFLPSRVAGAAAAAAAAAAARPPPPPAPVQPPAPIFTHPAAAAAAAAAAAAGSGGAASVWYPHLHHHHHYLQQQQTHMGPLPPLPGAVHVLPSIMQLHMGVLAPGPPPQQQQQQHLQAKAPQKPHDSAAAAGGANGSLGPATSAAAATHMSYTGMQQRPGASSATTTSAGAVAFGQSPPHGLAAAAAAASTPPPPPPPPVCIPESVLQLIAHLSGRAAAELPVPETVTTAPLVVQKAPSAARLAAVAKYLEKRKHRNFQKKVRYESRKRLAEARPRVRGQFVKASTSAVAATTPAATGATVTSTSLRQPVYTAAGPAGLALPPAAAAAAASAAAARGVPPPSSRIGAVELAELVPDHDADIEDEGCDEPAAAEDSDGSVAVELAEV

SEQ ID NO: 54 - protein, 1102 aa, Chlamydomonas reinhardtii
MEANGFHVVLVEDDNICLKVVEQLLRKLSYRVSTASDGAAALKVLADCKQRGDKVDLILTDILMPEVTGFDLINEVVHGETFADIPVVVMSSQDSQESVLQAFQAGAADYLIKPIRKNELATLWQHVWRANRAKGGQTSSGAAHVGAGGRGGTSSRDGGGVAGTRCGPGDRGGSGGDAEGSGLGGGAGAVKDSSGGSTGAATSVLHSTGGTTLPSRAATGRHASTSAGHGVTSADPSNNQTSHAHAHAHAHAHGNAHAHAHLHMHGATDRAAQGSSANGPANHGAAGTGLQSAGMAGSTAAGAAAPAGESLAKPPFASLAVHFDLHSVLAGAGAAAANGGANAAAHTAGATGRESGQAAGAATGGIAAAGTVIGWSHADMDVDGGEAGAQDEDDEDEDDGVEAPAGTQNRKRAADDSGCDGAAANNNGNTAAKAGAAAIAAGGPGSSGRAKATDGARAEIRHNGGPMAARMAAAEGSQGSRAASGSAATGPGGAREGTATPSGDTFAESPSTFTSIINTTGSGSEADEQPVPLKHQEQQQQQQQQRVGEGDRAKPEPHPQNPAQAAHLPHPSAAPCSGGGGIAQAALPLGLQELAALGAARHKELWTQRHLMHQRQAAAAATAAAASAAAAAAMPTAGASAAAPAGPPSARPSASLADTGGDGPAAATAPETRADGPSGPATTQGPKRDAVAGAAAVGSSARSDSPLPAAAAATAGANGASGAASDVLAGAGSLALLRHSDRSAFTAFTVFLPGRVAAAAAAAAAAAAAATSAGASTGTANGAPPAPGTALAAAAAAAAAAASAVPLPHPHTAPPALFGVPPPSSVPPSSLSVLPPVMPLHPAAAAAAATAGGGKPSDAATYAAAAAAGLVPYPGFAPARPGPFPPPPGSGGPGAPPVYIPESVLQLIAHLSGRAAAEIPAVPAESVTAAPVVVQKSGGPASAARLAAVAKYLEKRKHRNFQKKVRYESRKRLAEARPRVRGQFVKAGTAGAAAAAAAAAAAAAAGTAATAAGTGTARGAATASGAAGKPELQGPDTAEEAAAATLLSAAAAMAAAAAGTSGPSGSGSGAMDVDGADPEADADVMDEDDGEDDGSDESAGEP

SEQ ID NO: 55 - protein, 936 aa, Chromochloris zofingiensis
MSADAGGQKPGVAEPGARTGPGFSVNSSFHVLLVDDDAVTLKYVEQLLRKCSYEVTTATNGREAIEVLEGRRGQVHIDLILTDISMPEVNGVQLIEEVVNGGKWKNLPVIVMSSHEAQANVLEAFQAGASDYLIKPLRRNELSTLWQHVWKASKLHQPHLHGEDDEDEDDTALDNGKFDSSAGNNKGSSGASTSAAGDATALSMADASRALYEHHPSHHHNHIGEPSIDTQASGQVGSNDPSLVIHPLDISPLPAAAPPLAVAGDPALAAAPLGTGGQDTPGSGDEQATAGTSVQQHQHSQAHHHSRHIPASGSGTTEHAPQSLSQHPHHHNHQHHHNSHHHHHQHDLAQQRQQHHHHHSNGVNQDHSQPNPDLTQMPSADQQSLLTLPHSPNGAMPLFKPSTSSAAMDCSTQQPLQQQQQHEHGSSSPALSRPHAEKSPFGVRYGGGNGGYSSSMSGASLPPGLQELAVLGQQRQAAREKDLQQRQQQQQKQQQQQQQTSALRHSDSSAFTAFTVFLPKGSNGLNRSSGVGVHGSNSQTSGGGAADLGRSASSMEILSTAETLVGQTAGGAGVNGVGSAKPGGDCLKEESPNDSTPSAEEGDEQDVKPPQSTSGAAAAEPAVATASGRAATAAIAVVADATVAKPDAPVATSDQKQVLPFPGVNGAAHLTGMNNGVSHSGTAGSYSELTQMLYAQLPHQGQPLPDHVMHFLHNFYRTMMEHQHQQQSQQMDQLHHHVQQQQQQQVQQQQRHLQQFATAPNGQAPPNHSNTNQHLQQQQQACGNQPLQHTSQPHCNGAAHLQHLQQSHSAPSLHTPGFTCTTTATQSNTEPSCMLTQSEGAPCASSYRAAAVAKYREKRKNRNYDKKVRYESRKRLAESRPRVKGQFVKQEVLAAAGLTALAELATANKRARLDVDYVTATGMTDADHMDTAEESS

SEQ ID NO: 56 - protein, 444 aa, Coccomyxa subellipsoidea
MAAGLKRIPSFSGRPGFPNGLQVLVVDGDTSSSQCLRQKLEELAYEVSCCSSGSDASALLRKEDSSYDILLVEAKALAKDATDGGSLRDSAAHLPLVLMSEKSSSTDAVWRGIELGAADVLEKPLSSLKLRNIWQHVVRKMMSSSQDSSREAVPCKMEPKSKGKGVSAPSSPRTPSPAASLLTISSGTMTEKSCKGGGDEASFSGVGDVKMSCSAEAPEPCDSRATAESPASTQTKVTFPGCLNSGGTALAASKNCSRKRKAKAPDTPASVASRPPLAIRPPAWASPFGPPHQGNTHVVGMAPPQCYMQGVDPTNGCVWGTPAGGVSQAPAYMPGWGFSPQPMLSGSFLQHPSTSDLHKCPSVGASSLASSLDSSLTLCGFGADLPDDDLLLEDVLLPDEDLLDLAPDEPATMKAPEQPPIGLKLKKSASLIDLINAQLSAATA

SEQ ID NO: 57 - DNA, 1284 bp, Oocystis sp.
atggcgctgaagcgcgttcctagcttttccggtcggccgaactttcccgccggtctgcagatcctggtggtggacagcgattcttcctcaagggaggctgtagagatgcaactcaaatcgcactcctatctagcaacctgttgttgcacctgcggcgaggctgtggagcagctcggcacgtcaaagtatgacatcgtgctggcagagtccaagctggttgctgcggagtgcgttgactcgacacggttgtgcgaggccgcaagggctctgcctctggttttgatgtgcgaggactcgacggcggacgacgtgttgaagggaatcaggctcggcgcttgcgactttctggagaagccgctgtccccactgaagctcaagaacatatggcagcacgttgttcgcaagatgatggagcagatgcacgtccgccgcacggacgacgcggatacgtgcactactaagagcagccgcgaccaaagctgcgcgatcaagggcaagtcggtggcttccacgccctcgtgtcccaagacaccttctcccgcggcttctggcgcagacatcggctgcagcatagccacgtcggtcagcaaggccggggacgtggtcggcgagtccagcagttccgagacgcgcaaggagcattgcagcgagaccacggagtgctccgacctcaagagctgcgccgcaaagtcagctgtgtcggcgcaaacgccggtatccaccgcgaccgttgcagctacctggggtgcgtcgaagaagaagtcgacagcatcagccactaccagcagtgtcagcaaccggccgccgctggcgatcaagatgccggcgccagctgtggcatacacgtcagggcttgcgccctttccgccgccgatgtttgtacctggcggctggggccagtcaagcaacccatgcgtggtgggcacgccaatgatgccaccgccgcccggcatgggcatgccgccccaccaccacgcgccctatggccaggtgccgccgccgggctatccagtcgcatgcatgcccagcgcctttgtgccgacgccgatgggccctggcggcgtggcgtttgcgccgccacctggcgccagctgcacatctgctgcgtactacccccatcctgctgtggatgcaagcgcgtctgcaactgccaccttcacgggccatgtgcagatcgacctgactaacgtgtctgctgaagagccggcgcccattggtttggcgctgcgcaagaccgcgtcgctgctcgacctggtcagcgatcgcctgggccagcgtgcgtgc

SEQ ID NO: 58 - DNA, 1026 bp, Tetraselmis sp.
atgctgtgccctgctgtccaggttgccaccatggccactgtcctggcttccacgcatttttcggagcgccccagcttcccggctgatctggaggtgctgcttctggattcagcaacgcagggcgcagaaactgcctcgaagctgttgctgtcgtgttcctatcgtgtcaccgtgtgccgatccgtgtctgaggctctgagccacatggcatgcaaggctttcgacgtggtcctggtggagcagaaacttttcagcggcagggatgcggccgctgcgcagctcaaggccctggcaggcgtcatccccaccgtggtcctgagtgacagcggcagtgcgaaggatacctgggctgccatcgttgggcaggcagccgatgtcctcatccgcccgctgaccaagcagaagctgcagacgctgtggcagcacactgtccgtatgcagcgcgcagcatcttcggcttcggcggctactagcatggttgccaagcctgttgccgtgctctcctcggctctgaagcccgctgcttccagtgcttcactggacaaggggcagaagcgcaagttgaaggatcatatgatggggcccatcatggcacacccgcaagtgtccaaccctggctttatctggggcgcaccagtgatgggcgttccggctggacagcaggctccccagaagtcagaggccccggtcaccccccagaagccaggctcagagatgcaccccgagctggatgccacaagccacatcgccatgggctccagcgacaacttcaacgtacctgtgtatgaaagcggcactgacagccaggagtcgcagccaacctgcgaccccacctctcttgatgacatcaatgaggatgactacgcgtttatcgatttcgcgctcagcgattcttttcccactgtggaggaggatgagatccttccacccattggcctttcgctgaagaagtccagctccctcctgaacatgctgaacggtgtgcttctctcggctcactctgtaccgctgcagctgccccagtag

SEQ ID NO: 59 - DNA, 2076 bp, Glycine max
atgggagaggtggtcatcatgagtggagagaagaagtcagttagagtggagggggtggagaaggaagatagtggtggaagtgggagcaaggctggtgaatttaaggggttgatgaggtgggagaagttcttgcccaagatggttttgagggtgctgttggttgaagcagatgattccacaagacaaattattgccgcgcttctcagaaaatgcagctacaaagtggttgctgttcctgatggcttgaaggcatgggaattactcaagggaagaccgcacaatgttgatctaattctgacagaagtggatttgccatccatatctggctatgcacttctcacattaattatggagcacgagatttgcaaaaacatccctgttataatgatgtcttcccaagattcaattagcacagtatacaaatgcatgttgagaggtgctgctgattatcttgttaagcctattagaaaaaatgaactgaggaacttgtggcaacatgtttggagaagacaatcatcaaccactggtattaatggcctccaagatgagagtgttgcacaacagaaggttgaagccactgcagaaaataatgctgctagtaatcgttcaagtggtgatgctgcttgcattcagagaaatatagaactaattgagaagggaagtgatgcacagagctcttgtaccaagcctgactgtgaagctgagagtgaccctgtcggtaacatgcaggaattttctctgctgaaatgtggggaagcatatccaagtggaacagagacacaacaggttgaaacaagctttcgcttaggccagacattaatgatgcatgactgtcatgctggaggattaaatgtgagtatccgcaaaaatggtgaggcaagcacgactaatgacaaggatactgatacagagcattttgggaatgctagcatcagtggtgaggctcatgacaatccctatgttcaaattaactcttccaaggaagctatggacttgattggagcatttcatactcatccaaactgttccctgaaaaattccacagttaattgcacaggcaactttgaccattctcctcaattggatctttctttgagaagatcttgtcccggaagctttgagaataaactcactgaagaaaggcacaccctgatgcattctaatgcttcagctttcaagcggtatactaccaggcaattgcaaatatcaatgcctgcagtgttaattaacttctctgatcaacaaagagaacagataacaaattgtgagaaaaacatctcacacatcgctactggcagcaactcagatagttcaacacctatgcaaagatgtattgtgtctccaactacagtccaatcaaaagaatctgaacttgcaacctcacaccccccgcaaggacattctctcccaattccagtaaagggtgtaaggttcaatgatctatgcacagcctatggttctgtacttccttcagtgtttcatacacagtcaggtccaccagcaatgccaagtccaaattcagttgtgctccttgaaccaaactttcaagtaaatgcattttatcagtcaaatatgaaagagagtagttcagagcagctttatgaatctcgtggtccaaatggaaacaccacccaaaaccacattgtgtacacacaggagcacaaatcagaacatgcagaagatcgaggacatatctctcctacaactgatcaaagtgtgtcaagtagtttctgcaatggaaatgcaagccatcttaacagcattggttatggaagcaactgtggaagtagcagcaatgttgatcaagttaacactgtttgggcagcttcagagggaaagcatgaagacctcacaaataatgcaaactctcatcgatctatccaaagagaagcagctctaaacaaatttcgcttgaaaaggaaagagagatgctatgagaagaaggttcgatacgagagcagaaaaaaactagcagagcagcgtcccagagttaaaggacaatttgttcgtcaagtgcatcctgatcctcttgttgcagaaaaagatggcaaagaatatgatcattcagatttctga

SEQ ID NO: 60 - DNA, 2244 bp, Vitis vinifera
atgggtgaggttgtggtgagcagtgaggcaggaggaggaggcatggagggtgaggtggagaagaaggaggtgggcagtggggttgtgaggtgggagaggtttcttcccagaatggttctcagggttttgttggttgaagcggacgattccaccaggcaaattatcgctgcgcttctcaggaaatgcagttacaaagttgctgctgttcctgatggcttaaaggcatgggaggtactgaaggctagaccccacaacattgacctcatattgacagaagtggagttgccatcaatatctggctttgctctcctcaccttggttatggaacatgagatctgcaaaaacattcctgttataatgatgtcctcacatggttcgataaacacggtttataaatgcatgttgagaggtgcagctgactttcttgttaagcctgttagaagaaatgagctgaagaatttgtggcaacatgtctggagaagacaatcgtcaactgttagcggaaatggcccccaagatgagagtgttgcacaacagaaggtcgaagccacttctgaaaacaaccccacaagtaatcactcaagtgatcatgttgcttgtattcagaaaaataaggaagcactcaataaagtgagtgatgctcagagctcttgttcaaagccagacttggaagctgagagtgcctacatggaaactatgcaggatttctcaaatccgacatggagcagatctcttgtgagtgacacaaaaatgcagaagaatgaagaatgtgccaaattgggcccgaaatttcttatgcacaataaagaagctgggggaacactggaggctgcctgcagggatgtgaacacaatgactcagcctgaagcagtggaaccagaaaatgatgggcaaggtgctaacgctcctagtgaggcttgtggtaacaatgccatattgggcagctcatctagagaagccatcgacttgattggagtatttgataattctaaaaaatgcacttatggaaattcttcttcaaataatggcaccaaaaagagtgattctattccacagttggacctttccttgagaagatctcatcctagtagccctgagaatcaagttgctgatgaaaggcatacactgaaccattctaatggctcggccttttcacgctacataaacaggtcattgcagccaccacatctaccatcaacaggtgttttcaatcagcagaaaaactttggagctgattctgataaacgtttatctcagctggttactggttataactctgatattactagtcccacactgagtactcaaagaagtgtgatctctctagctactagtccatctggacgagttgaaattgcactttgtggccctcaacagagagcttttcctgctccagttccacaaaatgccaacaattccaccagccagactaatcacaagccagagcacaaattggactcactggagggtcaagggcacttctctcctgccactgatcagaattcaagtagtagttttggtaatggtggtgcaagtaatctgaatagctttgggtgtggaagcatttgtggaagtaatgggaatgccaatacagttgctgttgttcaggccgctgcagagggcaagaatgaagaaggtatcttcagtcatgaaggacactctcaacgatctatccaaagagaagctgctctaaccaagtttcgcttgaagcggaaagacagatgctttgagaagaaggttcgttatgaaagcagaaagaagcttgcagagcagcgaccccgagtaaaaggacagtttgttcgacaagtgcataccatccccccacctgcagagcctgatacatactatggcagttcgtttgatgttcagcctcaaagaagccgatatctatcagctcaacctctcagggcctcatcttctcaactcctctatccaactcacactcctctccaagaatccaaatacgaaggtcatgaagaaagcaatctcttgacggcgtccttggttggaactgccctaccggtggctccatcttttggttatgaagttggacgtgatcagacggcaggaaaacttgttctgagtttaaagctcgatggccgggttcgatggaaggtggggacttgggtttctggccgataccgacttaacgttaattgtgttgctgtgatggcatttggaccctccatcccatctggtccactgagttcaaaagaaggaactcagtgctctactactgtttga

SEQ ID NO: 61 - DNA, 2400 bp, Theobroma cacao
atggggatagttcaaatgaataataatggtcctgtggccaatgggttggttgaattgaatacacatattcatgatgagcacaagaaaataaggggtggggtcataggtgaggggcagggcctctcagtggaagaagagtcatggattaatgaggatgtggaagacaggaatgatgggaagacagagttggttcaggttcagggccatgcgcatggtgagcaagagaggtcacagcaacagcctcaaggtcctttggttcactgggagaggtttttacctctaaggtctttgaaggttctactggtggaaaatgatgactcaactcgccatgttgtctgtgcattgctgcgaaattgtggatttgaagttactgctgtgtcaaatggactgcaagcttggaagatcttggaagatctaaccaatcatattgatcttgttttaactgaggtagtgatgccttgtttgtcaggcattggccttttatgcaagataatgagccacaaaactcgcatgaatattccagtgattatgatgtcatctcatgattctatgagtacagtctttaggtgtttgtccaagggtgcagttgactttttagtgaagcctatacgaaagaatgagcttaaaaatctttggcagcatgtttggaggaaatgccacagctctagcagtagtggaggccaaagtggtacacagacccaaaaatcctcaaaatcaaaaggtactgattcagacaacaatactggaagtaatgatgaggatgacaacggcagtgttggtttgaatgttcaggatggaagtgacaatggaagtggcactcagagctcatggacaaagagagcagtagaagtcgacagctcccagccaatatcaccatgggaccagttagctgatcctcctcatagcacttgtgcccaggttatccattctagacatgaagtgttaggtgacagctgggttccagtaacagcgacgagggagtatgatgagctggataatgaactagaaaatgttgttatgggcaaagacttggagataggggtacctaaaattacagcttcgcagcttgaagacccaagtgaaaaagtaatgaccaacatagctggtgttaataaagacaaattatctgcaataaaccctaagaaagatgatgagaaactagagaaagcgcaattggaacttaacagtgagaaatcaggtggtgatttgagaaatcaagctgctgacctgataggtgtcatcaccaataatactgaacctcatatagaaagcgcagtctttgacatcccaaatggcctccctaaggtctctgatgcaaaagagaaggtgaactacgacacgaaggaaatgccttttcttgagctcagtttaaagagactgagagatgtaggagacactggaacaagtgcccatgaacgaaatgtattgagacattcagacctttcagccttctcaagatacaattctggttcaactgccaatcaggctccaacaggaaatgttggtagttgttctccacttgataatagctcggaggcagttaaaacagattctatgaagaattttcagtctacctcaaatagcatacctccaaagcaacagtccaatggaagtagtaacaataatgacatgggttccaccactaataatgccttcagcaaaccagcggtactcagtgacaagccagcacctaaaacttcagctaaatctttccatccctcttctgccttccaaccagtgcagagtggccatggttctgccctgcaacctgtagcacaaggtaaggctgatgctgcactaggtaacatgattttagttaaagcaaggggcacagaccaacaggggaaagtgcagcatcaccatcatcattatcaccaccaccaccaccaccatgtccataacatgctcccaaatcaaaagttaggtaaccatgatgatttatctttggaaaatatggcagcagcagctccccagtgtgggtcatccaatctgtcaagtttaccacatgttgaaggcaatgctgctaaccacagtttgactagaagtgcatcaggaagtaaccatggaagcaatggacagaacgggagcagcactgtgttaaataccagaggaatgaatcttgaaagtgaaaatggggtgcctgggaaaggtggagctggcggtggaattggatctggaggcaggaatgtagttgatcaaaaccgttttgctcaaagagaagctgctttgaacaaattccgccagaaaaggaaagaaagatgctttgagaagaaggttcgatatcagagcagaaagaaactggctgagcagagaccacgcattcgaggacagtttgtgcgacagattagcactactgggaaggaagcattcagatttcgtggtgcaggattgtgcacttag

SEQ ID NO: 62 - DNA, 2229 bp, Oryza sativa
atgatgggaaccgctcatcacaaccaaaccgccggctctgccctcggagtcggagtcggagatgccaacgacgccgtgcctggggctgggggtgggggctacagcgacccggatggcggaccaatctccggtgtgcagcggccaccgcaggtctgctgggagcgcttcatccagaagaagactatcaaagtcttgctagttgatagcgatgactccaccaggcaggtggtcagtgccctgcttcgtcactgcatgtatgaagtcatccctgctgaaaatggccagcaagcatggacatatctagaagatatgcaaaacagcattgatcttgttttgacagaggttgttatgcctggtgtatctggaatttctctattgagtaggatcatgaaccacaatatttgcaagaatattccagtgattatgatgtcttcaaatgatgctatgggtacagtttttaagtgtttgtcaaagggcgctgttgacttcttagtcaagcccatacgtaagaatgaacttaagaacctatggcagcatgtgtggagacggtgccacagctccagtggcagtggaagtgaaagtggcattcagacacaaaagtgtgccaaatcaaaaagtggggatgaatccaataataacaatggcagcaatgacgatgatgacgacgatggtgtaatcatgggacttaatgcaagagatggcagtgataacggcagtggcactcaagcgcagagctcatggacaaagcgcgctgttgagattgacagtccacaggctatgtctccagatcaattagctgatccacctgatagcacttgtgcacaagtgatccacctgaagtcagatatatgcagcaatagatggttaccatgtacaagcaacaaaaattccaagaaacaaaaagaaactaatgatgacttcaaggggaaggacttggaaataggttctcctagaaatttaaacacagcttatcaatcctctccgaatgagagatccatcaaaccaacagatagacggaatgaatatccactgcaaaacaattcaaaggaggcagcgatggaaaatctggaggagtcaagtgttcgagctgctgacttaattggttcgatggccaaaaacatggatgcacaacaggcagcaagagccgcaaatgcccctaattgctcctccaaagtgccagaagggaaagataagaaccgtgataatattatgccatcacttgaattaagtttgaaaaggtcaagatcgactggggatggtgcaaacgcaatccaagaggaacaacggaatgttttgagacgatcagatctctcggcatttacgaggtaccatacacctgtggcttccaatcaaggtgggacaggattcatgggaagctgttcgctgcatgataatagctcagaggctatgaaaacggattctgcttacaacatgaagtcaaactcagatgctgcaccaataaaacaaggttctaatggtagtagcaataacaatgacatgggttccactacaaagaacgttgtgacaaagcctagtacaaataaggagagagtaatgtcaccctcagctgttaaggctaatggacacacatcagcatttcatcctgcacagcactggacgtctccagctaatacaacaggaaaagaaaagactgatgaagtggctaacaatgcagcaaagagggctcagcctggtgaagtacagagcaacctcgtacaacaccctcgcccaatacttcattatgttcatttcgatgtgtcacgtgagaatggtggatccggggcccctcaatgtggttcatccaatgtatttgatcctcctgtcgaaggtcatgctgccaactatggtgtcaatggaagcaactcaggcagtaacaatggaagcaatgggcagaatgggagtacgactgctgtaaatgctgaacggccaaatatggagatcgctaatggcaccatcaacaaaagtggacctggaggtggcaatggaagtggaagcggcagtggcaatgacatgtatctgaaacgcttcactcaacgagagcatagagtggctgcagtgatcaagtttagacagaaaaggaaagagcgcaacttcggaaaaaaggtgcggtaccagagcagaaagaggctggccgagcagcggccaagggtccgcggacagttcgtgcggcaagctgtgcaagaccaacaacagcagggtggtgggcgcgaagcggcagcggacagatga

SEQ ID NO: 63 - DNA, 2301 bp, Zea mays
atgggcagtgcttgccaagctggcacagacgggccttcccgcaaggatgtgttagggatagggaatgccgccttagagaatggccaccatcaggctgaagctgacgcagatgaatggagggaaaaggaagaggacttggccaacaacgggcacagtgcgccaccgccaggcatgcagcaggtggatgagcataaggaggaacaaagacaaagcattcactgggagaggttcctacctgtgaagacactgagagtcttgctggtggagaatgatgactctactcgtcaggtggtcagtgccctgctccgtaagtgctgctatgaagttattcctgctgaaaatggtttgcatgcatggcgatatcttgaagatctgcagaacaacatcgaccttgtattgactgaggttttcatgccttgtctatctggtatcggtctgcttagcaaaatcacaagtcacaaaatttgcaaagacattcctgtgattatgatgtctacgaatgattctatgagtatggtgtttaagtgtttgtcgaagggagcagttgatttcttggtaaaaccactacgtaagaatgagcttaagaacctttggcagcatgtttggaggcgatgccacagttccagtggaagtgaaagtggcatccagacacagaagtgtgccaaactaaatactggcgacgagtatgagaacggcagtgacagcaatcatgatgatgaagaaaatgatgacggcgacgatgacgacttcagtgttggactcaatgctagggatggaagtgacaatggcagtggtactcaaagctcatggacaaagcgtgctgtggagattgacagcccacaacctatatctcccgatcaactagttgatccacctgatagtacatgtgcacaagtaattcaccctagatcagagatatgcagtaacaagtggttaccgacagcaaacaaaaggaatgtcaagaaacagaaggagaataaagatgaatctatgggaagatacttaggaataggtgctcctaggaactcaagtgcagaatatcaatcatctctcaatgatgtatctgttaatccaatagaaaaaggacatgagaatcacatgtccaaatgcaaatctaaaaaggaaacaatggcagaagatgattgtacaaacatgcctagtgcaacaaatgctgaaactgctgatttgattagctcaatagccagaaacacagaaggccaacaagcagtacaagccgttgacgcaccagatggcccttccaaaatggctaatggaaatgataagaatcatgattctcatatcgaagtgacaccccatgagttgggtttgaagagatcgagaacaaatggagctacagcggaaatccatgatgagcgaaatattctgaaaagatcagatcagtcagccttcaccaggtaccatacatctgtggcttccaatcaaggtggagcaagatatggggaaagctcttcaccacaagataacagttctgaggccatgaaaacggactctacatgcaagatgaagtcaaattcagatgctgctccaataaagcagggctccaatggcagtagcaataacgatgtgggatccagtacaaagaatgttgctgcaaggccttcgggtgacagggagagagtagcgtcaccattagccatcaaatctacccagcatgcctcagcatttcatactatacagaatcaaacgtcaccagctaatctgattggggaagacaaagctgatgaaggaatttccaatacagtgaaaatgagccacccaacagaggttccacaaggctgcgtccagcatcatcatcatgtgcattattacctccatgttatgacacagaaacagccatcaacagaccgtggatcatcagatgttcactgtggttcgtcaaatgtgtttgatcctcctgttgaaggacatgctgcaaactacagtgtgaatgggggtgtctcagttggtcataatgggtgcaatgggcagaatggaagtagcgctgtccccaatattgcaagaccaaacatagagagtattaatggtaccatgagccaaaatattgccggaggtggcattgtaagtgggagtgggagtggcaatgacatgtatcagaatcggttcctgcaacgagaagctgcattgaacaaattcagactgaagcggaaagatcggaactttggtaaaaaggttcgctaccaaagcaggaagaggcttgctgagcagcggccacgggtccgaggacagtttgtgcgacaatctgagcaagaagatcaaacagcgcaaggttcagaaagatga

SEQ ID NO: 64 - DNA, 2034 bp, Physcomitrella patens
atgccatatctgtccggagttgggcttctgtcgaagatgatgaagcgggaagcatgcaagagagtgcctattgtcatcatgtcatcgtacgacagtcttggcatcgtgttccgctgcctctcgaaaggagcttgcgactatctcgtgaaaccagttaggaaaaacgagttgaagaatctgtggcagcacgtatggaggaagtgccacagttcgagtgggagcagaagtggaagcggaagccagactggggaagtagctaagcctcggagtcgtggtgtagcagccgctgacaatcctagtggaagcaatgatgggaatggcagcagtgatgggagtgataatgggagcagccgggtaaatgcccagggtggaagcgacaatggtagtggcaatcaagcttgcatgcaacctgtacaggttctgaggaacagcgcaattccagaagcagtagacggggatgaggaggggcaggcgacatcgcaagataagggtgctgacttggatggagagatggggcatgatctggagatggcaactcgaaggtctgcttgtgttaccaccggaaaagatcagcaaccagaggatgcccagaagcaagatgaggatgctgtatgtatcttgcaagatgcggggccatcacctgatggggctaatgccgagagcccatcatctagcggtcggaatgatgccgcagaggagtcttctccaaagatcattgacctgataaacgtcatagcgtgtcagccacagacccaggatgcagaacctcaagaaagtgagaacgatgacgaagaattggatccgcggggaaggagcagccctaaaaacaactccgcttcagattccggtacttcgctggagttaagtttgaaacggccacgatcggcggttggtaacggcggagaattagaagagcgtcaaccactgcgacattcaggaggctcggccttttctaggtatggcagcggaggaaccattatacagcaataccatcagactggaggttcactccctctcagtggttatcctgtgtctggtggatatggtgtatatggcatgtccggcggtagccctggaggatctcttcgtctgggaatgggaatggatcgaagtgggtcatcgaaaggaagtgtagaggggactacacccccaccctcgcatcctcagagcatggagaaagtgggtgggcaagatgggtacggcaatgcaagacagactacggaggatgcaatgatcgtacctggaatgcccatggctattcctctcccaccacctgggatgcttgcatatgatggcgttattggaacgtatggtccggcgatgcacccgatgtattatgctcaccctagcgcgtggatggcagctccgtctcgtcacatgggagagcggggagatgtctacaatcaatctcctgcatttcaagagcaggattctgggtctgggaatcattctcaagcggggcagactcaccagcacatgcaccaccaccaaggcaaccagcaccaccatcatcatcaccatcaccaccatgggagtggcgcccagccttctggaaatgcaggggtgcaagatgaacaacagcaatcagtggtaccgcctgggtcgagtgctcctcgctgcggctcgaccggtgtggatggtcgaagtggtagcagcaacggctacgggagcaccgggaatgggaatgggtccatgaacggaagtgcttcgggaagtaatactggcgtgaacaacggtcagagtggatttggtgcgacgccgatgttaactgacaacagtgggagtaacggcgtcggtggaacggatgcagccatggatggggtgagtgggggcaatgggctgtgcacagagcaaatgcgtttcgccagacgagaggctgccttgaataagtttaggcagaagagaaaggagcgatgctttgagaagaaggtgcgataccaaagcaggaaacggcttgcagaacaaagaccacgagtccgcggtcagtttgtgcggcaagcggtacatgatccgtctgctggtgacgccgaatag

SEQ ID NO: 65 - DNA, 4080 bp, Volvox carteri
atggagttccacgtactgctggtcgaagacgacagggtgacgctgaagacagttgagcagctactccggaaatgcaattacaaagttacctgtgcagcaaatggacgggaggcaataaaggtccttactgcctgccggcacagcggcgtcaaagtggaccttattttgaccgatatactgatgccggaggttaccggctttgacttaatcaatgaagtggtacatggggacaccttttgcgatgtgccagtggtcgtcatgtcctctcaagactcgcaggagaacgtgttacaggcattccaagcaggcgctgccgactaccttataaagcccattcgcaaaaatgagctggctacgctctggcagcatgtctggcgcgccaacaaggccaaggggtccggcagcggcaccaccactaacgtcaccgggcagcccctttccggtcgggaggatctggaggcaggcgaagccgtcgctgtcgccgccgccgccgccgctgccagcggcaaggcctgtgcagcaacgcatgggcatttgaaggacagcagcggcggcagcagcggcgccgccgcttctgtattgcagtccacgggcggaacactactgccggaccgtgctgccactgtacggtatccagctgcggcggcagcgccaccgccacctggcgcatccgagctatcagggaacgtgacggcgggcgaagctcaagggagccgtacgcagcatctgcgccatctgtccggcttggcggggatggaaagcacagcggcgacgtcagcggcggcgcaaggcagtagcgcagcagggccgctgcggggctgcggcggtgctggtactgctatagctggtgggccgcgcgcgcccttgggcccactttcattcgcgcccttcggcacttccgttgccgtacactttgacctgaaccccgcatccggcgcagctcgacggctggtcaactccagcggcgccatcgatgcgtcgacgggcagcggcactgctggcgtcgccgcttcatcgcgttgcgccgccggcacctccgccaccgtcatcagttggtcgcacgtcgatccgacggagacggacccagcggaggcggagcccatgtacgacacgaacgcggacgccaccgcggcgaaggcagcggctgacggtgtggcggaagctgacgacgacgatgttggcgacgacggcggtgctgggcccaaccacaatgacgatgatgacgagggtggcggcgacgacgacgtcagcggcgacggtgacgaggacggaaaccggcctcgcaagcgtccgcggctgcttcagggatcctcgcatcaccacagccaccagcatcgccttcacagcctaggcggtacgactaccaacaccaccaccactacgacagccgcgaagcctaagtcgacagcgggagaacgcggcggcgcggcggcgctactcgcatgccgtactgcggcggccgcacccctacgcggcagtggctgcgccaccgctggcgccaccggagcatgtcgactggcggcggcggcagcggcggcggagggctcccagggttctcgcgccgcgtcggcgtcggcaggccctgacggcggcgcgcgtgagagtacggctacccccagtggtgacacctttgcagagagcccgtccgcgtacactgcaaccgccacaacgaccagtacggcaacaaccagtacgacaacgggatccgggattgagatgcaggacgacgagcaacagcagcgacagcagcctaagcagcgtccgccggcatctcagccggaactggagggtcatcatcaccaacaacaatatcaccattattatcgacgcaccagcctggagggcggttgcgccaacgcaccccctctccctgtcccttcatctgcacggggtgcttccccggcaggcacgggtccgacggaaagcggctccgggagggatagcggctgtgccaggattacaaatggtacggcggcgggggcgacggcggcaatgccgccatctcacgtcagctcggcaagccccccccgctgtaccgccacttccgcggcggcgactcgcgggtcctctggtgctgctactgcggcagcgggtgccatgacaacagccttggcgacggccggcagctatccgcgaggagtggacgccagcccgccgccgaatagaagtatggggtccagcggcggtgatggcggcggaaccgccgctgcagctgccggtacggcacgagggagctcgcctgcggctgctacgccgccgctgccaccttctacgcagcagcacgggttgccgcatcccgcggcggcgccgccgccgggcgctgcatcgcctggcggcgccgtgacgctgccgccagcgcttcaggagctggcggcactgggggcggcccgccatgcggggctatggacccagcgggccttattgcatcagcagcaattgttgctgcagcagcagaagcagcagaagcaacaacagcaccaacaagaccaggtagtgggggcagagaagattcatggtgggtcgacgtcggctgtagccaacgccgccgagcagcagcagcagcagccgctgggggcggcggcggcacgtcgtcccagcaaagcgggcgtggacggaactgaggcgggaagtggcgcggtcggcggatgcgcatcggcgacagcggcggtcatggcgatggaggcgtcggagccgcatggcgcggttggcagctcctttacggcggcagatcggcaggagacgccgttgcagcctctgcatgctgaatctgcggcggcaggcggcgacatggacggcaaccgcagtacacccgcaactatgccgtcggggcctacggcagccgcatcgggcccttcgcagacgtcgaacagcttgacggtgctgcgacatagcgacagatccgctttcaccgcattcaccgttttcttgccaagcagggttgccggcgccgcggcggcggcggcggcggcagcagctgctcggccgccaccaccgccggcgccggtgcagccgccggcgccaatcttcacgcaccctgctgctgctgctgcagccgcggcggcggctgccgctggcagcggcggtgcagcctcagtgtggtatcctcacctccatcatcaccaccactacttgcagcagcagcagacgcacatgggtcccttgccgccactgccaggtgccgtacatgttctgccgtcgatcatgcagcttcacatgggagtactggcgccagggccgccgccacagcagcagcagcagcagcaccttcaggccaaggcgcctcagaagcctcatgattccgccgccgccgccggcggagctaacggctcgctaggtcccgcgacatcggctgcagcggccacgcacatgtcgtacactggcatgcaacagcgcccgggcgcctcatccgccaccaccaccagcgccggcgctgtagcgttcggtcaatctccacctcacgggctggcggcggcggcggccgccgctagcacgcctccgccgcctccaccgccgcctgtttgtattcccgaatcggtactacagctcattgcgcatctgtctggtcgggcggcggcggagctgcccgtaccggaaaccgtcacgacggcaccgttggtcgtacagaaggcgccgtcggcagcgcgattggctgctgtagcgaagtaccttgaaaagcggaagcaccgaaacttccaaaagaaggttcggtacgagagccgtaaacggctggcggaggccaggcctcgcgtacgcggccaattcgtcaaggcaagtacttccgcggtggcggcaaccacccctgccgccacgggcgccaccgtcacctctacgtcgctccgtcagcccgtttatacggcggccggcccggctggcctggcgctgccgccggcggcggcagcagcggcggccagcgccgccgccgcgaggggggttccgccgccgtcatcccgcatcggagcggtggagctggcggagttggtgcccgaccacgacgccgacattgaggacgaggggtgtgacgagcccgccgccgccgaggactccgacgggtccgtcgcggtggagctggcggaggtgtag

SEQ ID NO: 66 - DNA, 3309 bp, Chlamydomonas reinhardtii
atggaggctaacggcttccacgtcgtattagtcgaggatgataacatttgcctgaaagtggtggagcagctgctgcggaagctttcgtacagagtcagcaccgcatccgatggtgccgcagcgctcaaagtcctggctgactgcaagcagaggggcgacaaagtagacctcattctcacggacatcctgatgccagaggttaccgggtttgacctcatcaacgaggtcgtgcatggagagacctttgccgatattccggtcgtggttatgtcgtctcaagactcgcaggaaagtgtcttgcaggcatttcaggcgggcgcagcggactacctcatcaagcccattcggaaaaatgagcttgcaacgctctggcagcacgtctggcgtgcaaaccgcgccaagggtggacagaccagcagcggcgccgcgcatgtgggcgcaggcggcagggggggcaccagcagccgcgatggcggtggcgttgccgggacgcggtgcggcccaggcgaccgcggcggcagcggcggcgacgctgagggtagtgggctaggcggcggcgcgggtgcagtcaaggacagcagcggcggcagtaccggcgccgccacttcagtgctgcactccactggtggcacgacgctgccctcacgtgcggccaccggtcggcacgctagcacctcagctggacacggcgtcaccagcgctgaccccagcaacaaccaaacctcgcacgcgcacgcgcatgcgcatgcgcacgctcacgggaacgcgcacgcgcacgcgcaccttcatatgcacggcgcaacagatcgtgcggcgcagggcagcagcgctaacggcccggccaaccacggggccgctgggacagggctgcagtccgctgggatggcaggttccacggctgcaggcgcggctgcgcccgccggtgagtcgctggccaagccgcccttcgcctccctagccgtccacttcgacctgcactcagtcctggcgggcgcgggagcggctgcagccaatggtggcgccaatgccgcagctcacactgctggcgccaccgggcgagagagcggccaggcggcgggcgcggccacaggcggcattgccgccgccggcaccgtcatcggctggtcgcatgcggacatggacgtggacggaggggaggccggcgcgcaggatgaagatgacgaggacgaggacgacggcgtggaggcgccggcgggcacacagaaccggaagcgcgccgcggatgactcgggttgcgacggcgccgccgccaacaacaacggcaacactgccgcaaaggctggcgcagcggcaatcgccgcgggcgggcctgggagctcgggcagggcgaaggccacggacggcgcccgcgctgagattcgccacaacggtgggccgatggcggcgcggatggcggctgcagagggctctcaaggctcgcgcgctgcatcgggctcggcggcaacgggaccgggaggagcgcgggagggcactgcgacgcctagcggcgacacctttgcggagagcccttccaccttcacttccatcatcaacaccaccggctcgggcagcgaggccgacgagcagccagtgccgctgaagcaccaggaacagcaacagcagcaacagcagcagcgggtcggcgagggtgacagggcgaagcccgaaccgcacccacagaaccctgcccaggcagcacacctgccgcacccgtccgcggccccatgctcgggcggtggcggtattgcgcaagcggccctacccctagggctacaggagctggcagcgctgggggcggctcggcacaaagagctgtggacgcagcggcaccttatgcatcagcggcaggcggcggcagcggcgacagcagcggcggcctcggcagctgctgcagcggcaatgcccacggccggcgcgagcgccgcggctcctgcaggcccaccttcggcgcggccctccgcttccttggcagacacgggcggcgacggccccgcggctgcgacggcgcctgagacgcgcgcagatgggccctctggccctgccacgacgcagggccccaaacgagatgccgtcgcaggtgccgcggctgtcggcagctctgcacggagcgacagtccgctgccggcagccgccgccgcgacggcaggcgccaacggcgcgagcggcgccgcttctgacgtgttggcgggcgcaggcagccttgcgcttctccggcacagcgatcggtctgccttcaccgcgttcacggtcttcctgcccgggcgtgttgccgccgccgcggccgctgcagcggccgccgccgcagctgctaccagcgcgggcgccagcaccggcactgccaacggggctccgccggcaccgggcaccgctctggctgccgctgccgcagcagctgccgccgctgcgtcagcagtgccgctgccgcatccacacacagcgcccccagcgctgttcggcgtccctccgccgtcctccgtgcctcccagctcgctttctgtgctacctcctgtgatgccgctccatccggccgctgccgctgcagcggcgacggcgggtgggggcaagcccagcgacgcagccacgtatgccgcggctgctgcagctggattggtgccgtatccagggtttgcgccggcgcggccggggccatttccgccgccgccaggttctggtggccccggcgcgccgcctgtgtacatacccgagtcagtcctgcagctgattgcgcacctgtccggccgcgcggctgcggaaattccggcggtgccggcggagtcagtgacggcagcaccggtggttgtgcagaagagcggcggccctgcctcggcggcgcgactggcggcagtggccaagtacctggagaagcggaagcaccgcaatttccagaagaaggtgcgctacgagagccgcaagcggctcgccgaggcccggccacgcgtcagggggcagttcgtcaaggcgggcaccgcgggtgcagcggcagcggcagcggcagcggcagccgcagccgcagccggcactgccgctactgctgccggcaccggcacggccagaggtgctgccaccgcttctggggctgctgggaagccggagctacagggccccgacacggcagaagaggctgcggctgcgacgctgcttagcgcagcagctgctatggcagcagcggctgcgggcaccagtggccccagcggctctgggtccggcgcgatggatgtggacggtgccgacccggaagcagatgcagacgtcatggatgaggacgatggcgaagacgacgggtcggacgagtccgctggggagccctag

SEQ ID NO: 67 - DNA, 1335 bp, Coccomyxa subellipsoidea
atggctgcaggcctcaagcggatacccagcttctcggggcgaccaggattccccaacggtctgcaggtgttggttgtggacggggacaccagcagcagccagtgcttgcggcagaagctggaggagctggcatatgaagtcagctgctgctcgtccggatctgacgcttcggcgctcctgcgcaaggaggactccagctacgacattctcctagttgaggccaaagctctggcaaaggatgctactgatggaggcagtctcagagattctgcagcgcacctgccgctggtcctcatgtcagaaaagagcagcagcacagacgctgtatggcgaggcatagagctcggggcagcggacgttctggagaagccgctgtcctccttgaagctgcgcaacatctggcaacatgtcgttcgcaagatgatgagctcgtcccaggacagcagcagggaggcggtgccctgcaagatggagccgaagagcaagggcaagggcgtgtcagcgccctccagccctcgcactccctcccctgcagcctccctcctcaccatcagcagcggcacgatgacagagaagagctgcaagggcggcggcgatgaggcctccttctcaggtgtgggagatgtgaagatgtcctgctcggcagaggcgccggagccctgcgattcgcgcgcgaccgctgagtcacccgccagcacgcagaccaaggtcacgttcccggggtgcttgaatagcggcggcacggcgctcgcggctagcaagaattgcagccgcaagagaaaggcaaaggcgccggacactcctgcatcggtggcgagccggccgcctctggccatcaggccccccgcatgggcctccccatttggtcccccccaccagggcaacacccacgtcgtcggcatggccccgccacagtgctatatgcagggggttgaccccacgaacgggtgcgtatggggcacgccagcagggggcgtcagccaagcgccagcctacatgcccggctggggcttctcgccgcagccaatgctttccggcagcttcttgcagcatccctccaccagcgacctgcacaagtgccccagcgtgggtgccagcagcctggcaagcagcctggacagcagcctgacgctgtgcggctttggcgcggacctgcctgacgacgatctcctgttggaggacgtgcttctgccggacgaggatcttctggacttggccccagatgagcccgccaccatgaaggcccccgagcagccgcccatcggcctcaagctcaagaagtccgcttcactcatcgacctcatcaatgcgcaactgtccgccgccaccgcctga

SEQ ID NO: 68 - protein, 568 aa, Parachlorella sp.
MLRQQLLHSGRQPGATCSLLTCSTWRPSALFGRPKPQKLHSQRLQHQGRPSRLVVRSAMFDNLSRSLERAWDMVRKDGRLTADNIKEPMREIRRALLEADVRLGAPLIRFLVSTPPPSQVSLPVVRKFVKAVEEKALGSAVTKGVTPDQQLVKVVYDQLRELMGGQQEGLVPTSPEEPQVILMAGLQGTGKTTAAGKLALFLQKKGQKVLLVATDIYRPAAIDQLVKLGDRIGVPVFQLGTQVQPPEIARQGLEKARAEGFDAVIVDTAGRLQIDQSMMEELVQIKSTVKPSDTLLVVDAMTGQEAAGLVKAFNDAVDITGAVLTKLDGDSRGGAALSVRQVSGRPIKFVGMGEGMEALEPFYPERMASRILGMGDVVTLVEKAEESIKEEEAQEISRKMLSAKFDFDDFLKQYKMVAGMGNMAQIMKMLPGMNKFTEKQLAGVEKQYKVYESMIQSMTVKERKQPELLVKSPSRRRRIARGSGRSEREVTELLGVFTNLRTQMQSFSKMMAMGGMGMGSMMSDEEMMQATLAGAGPRPVPAGKVRRKKLAAAGGSRGMAELASLKAE

SEQ ID NO: 69 - DNA, 23 bp, Parachlorella sp.
gggacatggtgcgcaaggacggg

SEQ ID NO: 70 - DNA, 2667 bp, Parachlorella sp.
atggccaaactgacatccgctgttcctgtgttgacagcaagagatgttgcaggtgcagtggagttttgtgagttctgagaagctgattgttgtttaacttctttgaaagctttatcgaagattctgcaagcgatgaacattgcttgtcaagaccgagagctgcatgcccacttgacatccagctttgaacggctcttcatgtttgatttgtttctgattgtagggacagatagactggggtttagcagggactttgtggaggacgattttgcaggagtggtgagggatgatgtgacactgtttatctcagcagtgcaggatcaagtgagtgcagcgtcagctgtggcagttgttggctttcgtctcagtcagtagtttgctgggattgattatggagggcacagttgcaattttgagttgcacgttgcgacaagcgtgttgacaaagcgtggtcaagccggccagtcttgccggtggcgggtggcttggtctaacttccgctctacagcaatcgttttgttcatggttacggggctggcgtgccagaaagtcctggtcagccaccctcgcttcaaagccgtagcccaacaactttgcgaatatgttcgatttgcaggtggtgcccgataatacactggcatgggtttgggtgagaggtacagctctgcgtgcaacaggttgcaagatgcagcgcaggtcttccctggtcaaacgatgtatgcagagttgagaggcacttgagctgggtgaatggcgtgggctcgtaggtagtgtgcagggcaggaagggcagccaattttggagttgtggtccggtgtcgttgcttcgagccttattaggactcttgctcatcaaagcgttagttgtgaataagttgatctgaaaggatgttatgtacagcaagcagcagcagttaagagtctggggagtagctgcacagggcgaggtgtcaagatgggaagggtcctgcctccttatgtgtttttccctgtaggggaggaagcctcttatgggcaatggttgggcatattttccagccagcccttctttctataggggccagggtgggcccagctcgtcttggcttccaccaccaggagagtgagggcattgaagggccataaatagtcctcccatctacgtgcaccagagggtgtcgtctaggctgtgcatgccacgaggggaaggagccaagaatgagtgtatgggttgttttcatgtttaggctgggataaaactgttttcaattgcgcctgccgggtgaaaaccacagcagcatcagcaagcttggagaaggccagcccgcccagcacaggctcacgttcccactcaggcggtcagtcgggcgggggtgtgagtcaggcaggcgagggtgtctgtgcctgacatcagcacctctgcttagccactgcagcccctggagcagggtagggcgtcatttgcagcaatcacctgctgcctcacacgtcgcagcttggaatttcaacgaccatcagcgctggggttgttgagggatcatagcagattttggtgcagcctggttgtcatgctctttgtggaatggcctctatgttcgagcaattcgttggatgttgaggtgcttggggacagagagtcgaatgatgggccagggtcaaacatgcgagcgtttggctgagtcagcggtttttgctggtcactttttcttttgtttcttatttaggtttgatggatgtgttttgtgctgctgccctgaagctgcagcagcgtgtctgccctgcgctactgcgggcaccaaggctatgtgctggtgcactcggctgcgctgcacctgtgcacctcgcactccgtccagcctccatgcagcacacgtactcacggtgtcctcctgacctgtcgtacgctattccaaacttgctcttttgctgccgctgctctcgtacacaattgctgttgattatcgatatctaatcgagcgcctgctgactgaactccgcaggtttggatgaactgtatgcagagtggtctgaagtggtgagcaccaactttaggtgggtgggctctgaaggaggaggagggagcgggtgattaaacagggcctgcatgaagaggagcaggggctgcatggacagcagggggaaggtgcagaagggagggtcaagcggggttcaggtggctgtgggtttctgcacgagcagtgaaagaagctgtatccttccacctgctttcactggcgaaaggttgaaaacaggatgtcgcagctggaaagatgttgcgctgtcaagtgcaagccatggttgagggtatgcctgtgtgcatgtgcttcttaaagttactcctgttctatggttctgggtgcttgttgtttgtggtgcagggatgcaagcggacctgcaatgacagagattggagaacaaccttggggaagggagtttgcattgagagatcctgcaggtgagggggcatgtaagcaatggcaggcaattcaagaacgaatcattgctgcaaatgctgggatggtatgcagctgaggtatctattgccttgtattttgtctcgcattgcatcggtggtgcgttctgtggcctgaggcacagttcttgctgtttgataagggttcgactgagttgtcgtgtgtgctgtgctgcaggcaattgcgtgcactttgttgcagaagaacaggactga

SEQ ID NO: 71 - DNA, 530 bp, Parachlorella sp.
ccaccatgggggaggtttgaagtgtgcgcctgatataatcatacacctaaaagcaccacttgctgattgtgaagggactatgtcgtttatgacgggacgttacgctggccgatggtttgaatttggacgctgtggtagaatgttatatggacgtaaaggttggcatattgaaaatcgtcttcgcaggcaaacttctagacgtgtgacccaccggtaaaacgacaagcgtggcgcgtcgattgcgctttgaacgtcgtttgttggactccagatgaacctcaaaatcaaagcggtgattgacgaaaatcaaatgacagcccgcaaaatttcatcagccttcggatcggattctcagaatctgattgtccctgctggctacatttatgaaatttcgtacattttggcagaaatgtcccaataccatagcactgccgcctgagctcacccgagcaatgcatactgggtacctcgcccatctcgccctctttccaagcccagtgctgttgtaatagccaaagggctcagtaaca

SEQ ID NO: 72 - DNA, 546 bp, Parachlorella sp.
gcatagcatcagcctgtggcagggttgtggtagggctgagtggcagggttaaaggggttgcctaccccacccctactctcatgacaccagcaacagcagcagctcatgcagtactcaaatcactgatgtcaatggtgtgacacatttggttaaggctgctttttaaagtgctgctttgggggcagtgactgtgcagagcttggagcgtatccccatgtaatcagaaccgacgagagttcggggcaacctttcatcttcacattttttgtgatcagctacagagtctgaaatcaaatagaggctgccatctaaacgcaggagtcacaacgaaggcgaaaactccaattgctgtactcaatgcactaagtgattgttcaatggataaatacactatgctcaattcatgccagcagagctgctccttccagccagctacaatggctttttccacgccttttgaagtatgaatgttcagcttgctgtgcttgatgcatcaccataaacacaattctacaacatttcatgccaacaacagtacgggctttc

SEQ ID NO: 73 - DNA, 23 bp, Parachlorella sp.
tgcggtgaagcttggagctgtgg

SEQ ID NO: 74 - DNA, 23 bp, Parachlorella sp.
acaccaccttaaggcacatgagg

SEQ ID NO: 75 - protein, 549 aa, Chlamydomonas reinhardtii
MQTALRARSAAPRGACNRTAVAPVASAHLRGQYAPFSGAQARPALGRQRQQQQQQRRGALVIRSAMFDSLSRSIEKAQRLIGKSGTLTAENMKEPLKEVRRALLEADVSLPVVRRFIKKVEERALGTKVREGRAMGTKWKSVVNCPLQDGLGNRGVGRARTEVGHRAACVHGARGVGKTTAAGKLALYLKKAKKSCLLVATDVYRPAAIDQLVKLGAAIDVPVFEMGTDVSPVEIAKKGVEEARRLGVDAVIIDTAGRLQVDEGMMAELRDVKSAVRPSDTLLVVDAMTGQEAANLVRSFNEAVDISGAILTKMDGDSRGGAALSVREVSGKPIKFVGVGEKMEALEPFYPERMASRILGMGDVLTLYEKAEAAIKEEDAQKTMERLMEEKFDFNDFLNQWKAMNNMGGLQMLKMMPGFNKISEKQLYEAEKQFGVYEAIIGAMDEEERSNPEVLIKNLARRRRVAQDSGKSEAEVTKLMAAYTSMKAQVGGMSKLLKLQKAGADPQKANSLLQELVASAGKKVAPGKVRRKKEKEPLSKARGFGSSSK

SEQ ID NO: 76 - protein, 559 aa, Micromonas pusilla
MRHLLSSASIRQYDKWSLVSSHAKKPALVCASKHTKSAVKLQCTSRGSSNRTIQLLLFQQFRPAKRGKLLITRADSFGTLSERLNSAWSALKDEDDLSVENISLPLKDIRRALLEADVSLPVVRRFIKSVEEKSIGVKVTKGVSASQQLTKVVADELCELMGGFGGDKLIFRKEGEGPTVILMAGLQGVGKTTACGKLALFLKAQGKQSLLVATDVYRPAAIDQLKKLGEQIDVPVFELGTDFSPPDIARSGVEKAKLENFDVVIVDTAGRLQVDEMLMAELLATKAATRADETLLVVDAMTGQEAASLTAAFNDAVGITGAVLTKMDGDTRGGAALSVREVSGKPIKFIGSGEKLDALEPFFPERMTTRILGMGDVVSLVERAQVAVKEEQANLMRDKILSATFDFNDFLSQLEMMGKMGGMGGLTKMMPGMNTMSDKELQDAEKSLSVAKSLIMSMTPRERQFPDLLVAGSSAASRRGRVVEGSGRSDKDLANLIVMFGSMRVKMQSLSAQMNGTAKEVGLVPQLSEVDLNKLAFEGVGKRVSPGMVRRRKLNASFG

SEQ ID NO: 77 - protein, 568 aa, Micromonas sp.
MEARTKQARAPKGSIWCAQRARKDLRARGCRGLGSRISKGQPFSPLTLSTPAVTEIGFGTLLYGSRLSAGGSRRGETMLRRASAFGSLTERLNSVWATLKDEDDLSLENIKGPLKDIRRALLEADVSLPVVRRFIKNIEQKAIGTRVTKGVNAGQQLTKVVADELCELMGGFGGDSLAFKDPSMGPTVILMAGLQGVGKTTACGKLALYLKKQGKDSLLVATDVYRPAAIEQLKRLGEQVKTPVFDMGVRVDPPEVARLGLEKARAEGIDVVIIDTAGRLQVDVHLMEELRATKIATAADEILLVVDAMTGQEAAALTAAFDEAVGITGAVLTKMDGDTRGGAALSVREVSGKPIKFTGVGEKMEALEPFYPERMASRILGMGDVVTLVERAQQVVKNEEAEQMRDKILSATFDFNDFIKQMEMMGQMGGMDGFMKLLPGMSGMSEREMQEADKSLKVAKSLILSMTSKERQFPDILVAGASAKSRRKRIIEGAGRSEKDLSQLIVLFGSMRVKMQKMTAEITGASAEVGLTPQLSEEDMNTLANEGLRKNVSPGMVRRLRIRRLTGS

SEQ ID NO: 78 - protein, 481 aa, Paulinella chromatophora
MFDELSARFEEAVKSLKGLSAITENNVENALKQVRRALIEADVSLVVVKEFMEEVRSKSIGIEVVRGIKPDQKFIQVVYEQLIEIMGANNTPLHKQSHTVTVVLMAGLQGAGKTTAAAKLALYLKNQGEKVLMVAADVYRPAAIDQLFVLGKQIDVEVFTLNPESIPEDIAAAGLQKAIREGFDYLIVDTAGRLQIDTAMMQEMVRIRSAVNPNEILLVVDSMIGQEAAELTRAFHEQIGITGAVLTKLDGDARGGAALSIRKVSGAPIKFIGTGEKVEALQPFHPERMASRILGMGDIVTLVEKAQEEVELADVEKMQRKLQEASFDFSDFLQQMRLVKRMGSLGGLMKMIPGMNKIDSTMLREGEAQLKRIESMIGSMTPTEREKPELLASQPSRRGRIAKGSGHKIADVDKMLVDFQKMRGFMQQMTKGNNFANPLSMGANMFSQPNMTVPQTKISNTNESRMRNSRATKKKKGFGQL

SEQ ID NO: 79 - protein, 498 aa, Ostreococcus lucimarinus
MTRADAFAGMSDKLDKAWARLQGEKDLNADNVKAPLKDVRRALLEADVSLPVVRRFIARCEEKAVGMKVTKGVEPGQMLVKCVADELCELMGGVGAEGIKFRDDGEPTVVLMAGLQGVGKTTACGKLSLALRKQGKSVLLVATDVYRPAAIDQLKTLGKQIGVPVFDMGVDGNPPEIAARGVRKAKDEDIDVVIVDTAGRLNIDEKLMGELKATKEATSADETLLVVDAMTGQEAATLTASFNEAVEITGAILTKMDGDTRGGAALSVREVSGKPIKFTGVGEKMDALEPFYPERMTSRILGMGDIVSLVEKVQAGVKEEEAEKIKQKIMSATFDFNDFVGQLEMMNNMGGMKQIMQMMPGTAKLSEADMEAAGKSMTIAKSLINSMTKEERQYPDMLVASTTADSRRQRIVKGSGRTEADLAQLIMMFGGMRTQMQKMSGQLGGQAGDVGLQPQLSEAELSKLAMNKIRKTVKPGMVRRQKAKKVPKFLAERESFSQ

SEQ ID NO: 80 - protein, 426 aa, Ostreococcus tauri
MKVTKGVEPGQMLVKAVADELCELMGGVGAEGIKFRDDGEPTVILMAGLQGVGKTTACGKLSLAMRKQGKTVLLVATDVYRPAAIDQLKTLGTQIGVPVFDMGVDASPPEVAARGVRKAKEEDIDVVIVDTAGRLNIDEKLMSELKDTKLATKADETLLVVDAMTGQEAANLTASFQRGDGRRTRRGGAALSVARSFRKAHQFTASVKMDALEPFYPERMTSRILGMGDIVSLVEKVQSEVKEAEAEKLKEKILKATFDFNDFVTQLEMMNNMGSMKQIMQMLPGTTKLSESEMEAAEKSFKIARSLINSMTKEERQFPDMLVASTTAESRRARIVKGSGRTEADLAQLIIMFGSMRGKMQQLSGELGGEAGNVGLQPQLSAAELEKLTTNKLRKNIKPGMVRRLKSKKIPIAKNGDRMGISASAD

SEQ ID NO: 81 - protein, 510 aa, Volvox carteri
MSRPAALRGAGNRKLTATVTAAHLRGIAFTSIRTCQGAKGGSLGLPHPSPPLALPRRGRGRGAAVVVRAAMFDNLSKSLEKAQRLIGGCEVPGVGVVGKSGTLTAENMKEPLKEVRRALLEADVSLPVVRRFVKKVEERALGTKVIEGVTPDVQFIKVVSNELIELMGGGVGAKDLEPGFPQIILMAGLQGVGKTTAAGKLALYLKKAKKSCLLVATDVYRPAAIDQLVKLGAAIDVPVFELGTQVSGKPIKFVGVGEKMEALEPFYPERMASRILGMGDVLTLYEKAEAAIKEEDAKAVMDRLMEEKFDFNDFLNQWKSMNNMGGMQILKMMPGFNKERSNPEVIIKSLARRRRVAQDSGHSEAEVAKLMTAYTAMRTQVGGMSKLLKLQKSGGDPSQAEKLLKELVASAGKKVAPGKPPGDPAGSFISTPRTPHPPPGPLGPRSQVRRKKEKEPISKARGFGSPSNFNHDLSPPGSSPAAYTYTLSRLSCQRLCDGGGLLDDWNLWRR

SEQ ID NO: 82 - protein, 448 aa, Phaeodactylum tricornutum
MSEASIQPALREVRRALLDADVNVDVADTLIEGVRARSLGQEVLEGVTAEQQFVKAMYDELLDMMGGDSSVPMSDGPSNVPVATLASGTAADPAVILLAGLQGAGKTTAAGKLALFLKEQRKVLLVAADIYRPAAIKQLQVLGESIGVEVFTKGTDVDPVEIVNAGIQKARDEGYDTVIVDTAGRQVIDTDLMDELQRMKRAASPQETLLIVDAMTGQEAASLTAAFDSAIGLTGAILTKMDGDSRGGAAVSVRGVSGKPIKFVGTGEKTADLEPFYPDRMASRILGMGDVVSLVEKAASEVSDADALKMQQKMLDASFDFDDFVKQSELVTKMGSVAGIAKLMPGMANQLNMNQIREVEARLKKSKSMISSMTKKERANPELLIKDSSARSRLIRITKGSGCGLDEGQQFMSEFQRMKTMMSTRRFWRFWLMIQSLALAVTRPENTV

SEQ ID NO: 83 - protein, 486 aa, Thalassiosira pseudonana
MFDQLSNALTEVAKNFGGKQRMTENSIQPALKSVRRALLDADVNLDVATALIDGVKRRSLGKEVTKGVTAEQQFIKAMYDELLDMMGGEANESNTMATLAHSSVANEPAVILLAGLQGAGKTTAAGKLAFRLPKRNRKVLLVAADVYRPAAIEQLQILGKQIGVEVFSMGVDADPADIAKEAVEKAKREGFDTVVVDTAGRQVVDEELMEELRRVKKTVEPDETLLVVDAMTGQAAASLTASFDAAVGISGAILTKLDGDSRGGAAVSIRGVSGKPIKFVGVGEKTNDLEPFYPDRMASRILGMGDVISLVEKASMEVSDADAAKMQEKMAKAEFDFDDFMTQSRMVSKMGSMAGVAKMLPGMGNMIDSSQMRQVEERIKRSEAMICSMNKKERANPGLLLTDKSARSRLMRITKGSGLAFEDGLAFMSEFQKMRTMISRMAKQTGMGQPDGEGEMEPAMAGNRNARRAAKKKGKKGGRGGGMGFA

SEQ ID NO: 84 - protein, 530 aa, Aureococcus anophagefferens
MTMARRAATAALVLAAAWAFAPPQTKRATTQLYFFDKLAESITAATDVLSGKSRMTEANTKSALRDVRRSLLDADVAKVVVDGFVENVQASALDGEVAEGVDPGQQFVKIVYDELKRVMGGDDDELLFSDDPEAAAKARAGLAYRDDGAPTVVLLCGLQGAGKTTAAAKLALRLKEEEGKTPMLVAADVYRPAAVEQLQILGEQVGVPVYAEAFEAGAGDAVAIATAGVRAAKERGADVVIVDTAGRQVIEESLMAELRSVRAATKPDETLLVLDAMTGQDAASLAKRFDDACPLTGSVLTKLDGDARGGAALSVRAVSGKPIKFVGVGEKVGDLEPFFPARMASRILGMGDVVSLVEKASKQQSAAEAKAVMERTKQAKFNFDDYLDQARMVSNMGSFGAVAKMMPGMGGIDNDQIAAAEAKIKIQASLINSMTPKERGEPDLIIRDKSALARQKRIAAGSGRSVDQAKQFLSEFQQMRTMMAKMAGQAPPDGADAAAAPDPDALLNRAARRAKKKKGGKRKLKTAGFG

SEQ ID NO: 85 - protein, 556 aa, Ectocarpus siliculosus
MIMASLKHRSPPRGGAAATLSFFCCVCALFAQSSVAFVPAGGLSRCGVNDRSSSSCRAAAIGAAGRSSLPVSRSSSRRGRRGGCAGGASSPLGMMFDTLAENMAGVANLFTGQKTITESSVEGALNEVKRALLDADLNLMVTNTLVDAVKSKAVGMKLVDGVTAKQQFVNVMNDELVEIMGAEQAPLARRTDGKPTVILLAGLQGTGKTTAAAKLAKYLQQEEEPKKVLLVAGDVYRPAIDQLISLGKRIDVEVFSMGQGVDPVEITKAGLERAVEGEFDTVIVDTAGRQVVDDTLMTELKDIQVASEADEVLLVVDAMTGQEAATLASVFNEKIGITGAVLTKMDGDTRGGAALSVQGVSQKPIKFVGIGEKMSEEEAAKLAKKMINAEFDFNDFLKQAKMMKGMGSLGGVANMIPGMAGKITPQQLNQAEEGVQRAEGLIKFMTPEERRTPKLLILDPTSQARCRRIARDAGVKLSAVSAFLKEFQAMQSNMSRMGKQMADGDPNAGPGGQPSPFQGLGGDTAPGAAPSMNRQQRRQSKKNKAGRSAAPSKGFG

SEQ ID NO: 86 - DNA, 28452 bp, Artificial Sequence
  Description of Artificial Sequence: Synthetic polynucleotide
cgtctgattaaaccacgctgggagattagataatgaagcgtgcgcctgttattccaaaacatacgctcaatactcaaccggttgaagatacttcgttatcgacaccagctgccccgatggtggattcgttaattgcgcgcgtaggagtaatggctcgcggtaatgccattactttgcctgtatgtggtcgggatgtgaagtttactcttgaagtgctccggggtgatagtgttgagaagacctctcgggtatggtcaggtaatgaacgtgaccaggagctgcttactgaggacgcactggatgatctcatcccttcttttctactgactggtcaacagacaccggcgttcggtcgaagagtatctggtgtcatagaaattgccgatgggagtcgccgtcgtaaagctgctgcacttaccgaaagtgattatcgtgttctggttggcgagctggatgatgagcagatggctgcattatccagattgggtaacgattatcgcccaacaagtgcttatgaacgtggtcagcgttatgcaagccgattgcagaatgaatttgctggaaatatttctgcgctggctgatgcggaaaatatttcacgtaagattattacccgctgtatcaacaccgccaaattgcctaaatcagttgttgctcttttttctcaccccggtgaactatctgcccggtcaggtgatgcacttcaaaaagcctttacagataaagaggaattacttaagcagcaggcatctaaccttcatgagcagaaaaaagctggggtgatatttgaagctgaagaagttatcactcttttaacttctgtgcttaaaacgtcatctgcatcaagaactagtttaagctcacgacatcagtttgctcctggagcgacagtattgtataagggcgataaaatggtgcttaacctggacaggtctcgtgttccaactgagtgtatagagaaaattgaggccattcttaaggaacttgaaaagccagcaccctgatgcgacctcgttttagtctacgtttatctgtctttacttaatgtcctttgttacaggccagaaagcataactggcctgaatattctctctgggcccactgttccacttgtatcgtcggtctgataatcagactgggaccacggtcccactcgtatcgtcggtctgattattagtctgggaccacggtcccactcgtatcgtcggtctgattattagtctgggaccacggtcccactcgtatcgtcggtctgataatcagactgggaccacggtcccactcgtatcgtcggtctgattattagtctgggaccatggtcccactcgtatcgtcggtctgattattagtctgggaccacggtcccactcgtatcgtcggtctgattattagtctggaaccacggtcccactcgtatcgtcggtctgattattagtctgggaccacggtcccactcgtatcgtcggtctgattattagtctgggaccacgatcccactcgtgttgtcggtctgattatcggtctgggaccacggtcccacttgtattgtcgatcagactatcagcgtgagactacgattccatcaatgcctgtcaagggcaagtattgacatgtcgtcgtaacctgtagaacggagtaacctcggtgtgcggttgtatgcctgctgtggattgctgctgtgtcctgcttatccacaacattttgcgcacggttatgtggacaaaatacctggttacccaggccgtgccggcacgtgatcgcgcaggctcagctgcacagcagacgcaagggacagctcagcatctggaaccgccgacaccaggtgctgaggatgctgcacctttggcaaccccaataggtgcttttgggcgtactgctgtgcctgcgcctagggacattgactggtggcgggtcccgaaggagctgatgggaagctacgcacaagctgaagctggagacagcagctccaccaatgttgacttctctggggagcctccggccagcagcgtgtacaacgagaggggggacgcgttagtggagcaggaggtgaaggcagcaacggcgggtgtggattttgctggcaggaggagggccagggggttgttggacaatgctgagcctcccgatcttgataatggccctggagagcagccagcaggggcaacagtgagttggagctggaggcgattcagggataggcagggataggcagtgtagtggccagaactggctgctggaacctggggttactcagggtgaacgcaggcaaaggggtgcaggtgtattgaagctcttaatataagagagatgcgtcgaacatatatggtgatagtcttgagtggtgtgttgggtggaaggctgctgtttacggtgcaggaagttttcctggtacggtcgttatgtaatgcagcagcacgtatgtaagaaccagtcgacatttaacctatgcagtagcatatagttatgtgtcaaaatcataaattggccctatttgtggcgagcctatctttcaaatactactgttcctcgcactgtcctctaaaatttctccaaacaacgttgtaaaggtgctgatgttagcatatcatctctggcataactggatgcacccagccggctaacagtgggaagatgaagaggggcttgtacactacacttttcttgccaagactgttagcttgcccaagccagcacagcgattttcttgcaacaaacgtgagccttgcatctgcttttgattgcaacggccgactggtgagttattgtgcaagcagtgttctgctaaactgttcagaccaggttcgcagctggctaagatcggtatctggaaagctccaacgaacaggttttcaatacgtgctgcgtcaatatgcccttcttgttcactacagcgacctttccaatgttggatgtgaacaaatgtcgaagcgcacaataacctgaaagacattgttgctcattcccttttctttggtagcgtaggtttgtatatttagagttccagttctgtactagttgctctgcggcaacgattgaagtgtgtaccttatactgcacgttaaatatgataggttcagcgcggttctttaaatgacaaaataaatagtattcaacaaaaaaaaatagttgtttgacatgtcactttttcttttacataggtagcatgtcgtcaaatcgtcaatgcaaaccagcttgcgactaacgtaagcagtacaggggatagtacaatgagtttttcaccagcaatttggtccagtgttttcgcaccgccgtgaagcgcattcacattaaagtagcatcgctacacctgttctcatcttgttaggttcaaattttgcaacgtgtagctacaaagtggcaacagcgcaggctgttggtcactcgctaaggcttgcattggcaccctcgttgctctgtgtaggagcgtgcatttgtgctcaagactgttatttttgacttcaaaaactttatcgatagcgcactgcctcgtttttacaagatagccttctgtgagcagccctgccccatgcgcctttaggctttctgtggcaatgtctggttcagctggatcgggccaggctactctcagacatgacggtggctctgctggcggcagtgggcctgtctcagacggtttttcaccggccggcctgaaggtaaagtagaaagacactcatacacatcttggttcggcgttgaaagtaggtcattaacatactctataaccaatatttgtaggttctggtcgtggacgacgagttaaccttggaaatccctaccaggctattctccacagcccgaaccccttaagctagacgaacacagttagcataacttcgtataggatactttatacgaagttatgcggccgcccaccatgggggaggtttgaagtgtgcgcctgatataatcatacacctaaaagcaccacttgctgattgtgaagggactatgtcgtttatgacgggacgttacgctggccgatggtttgaatttggacgctgtggtagaatgttatatggacgtaaaggttggcatattgaaaatcgtcttcacaggcaaacttctagacgtgtgacccaccggtaaaacgacaagcgtggcgcgtcgattgcgctttgaacgtcgtttgttggactccagatgaacctcaaaatcaaagcggtgattgacgaaaatcaaatgacagcccgcaaaatttcatcagccttcggatcggattctcagaatctgattgtccctgctggctacatttatgaaatttcgtacattttggcagaaatgtcccaataccatagcactgccgcctgagctcacccgagcaatgcatactgggtacctcgcccatctcgccctctttccaagcccagtgctgttgtaaatagccaaagggctcagtaacaatggccaaactgacatccgctgttcctgtgttgacagcaagagatgttgcaggtgcagtggagttttgtgagttctgagaagctgattgttgtttaacttctttgaaagctttatcgaagattctgcaagcgatgaacattgcttgtcaagaccgagagctgcatgcccacttgacatccagctttgaacggctcttcatgtttgatttgtttctgattgtagggacagatagactggggtttagcagggactttgtggaggacgattttgcaggagtggtgagggatgatgtgacactgtttatctcagcagtgcaggatcaagtgagtgcagcgtcagctgtggcagttgttggctttcgtctcagtcagtagtttgctgggattgattatggagggcacagttgcaattttgagttgcacgttgcgacaagcgtgttgacaaagcgtggtcaagccggccagtcttgccggtggcgggtggcttggtctaacttccgctctacagcaatcgttttgttcatggttacggggctggcgtgccagaaagtcctggtcagccaccctcgcttcaaagccgtagcccaacaactttgcgaatatgttcgatttgcaggtggtgcccgataatacactggcatgggtttgggtgagaggtacagctctgcgtgcaacaggttgcaagatgcagcgcaggtcttccctggtcaaacgatgtatgcagagttgagaggcacttgagctgggtgaatggcgtgggctcgtaggtagtgtgcagggcaggaagggcagccaattttggagttgtggtccggtgtcgttgcttcgagccttattaggactcttgctcatcaaagcgttagttgtgaataagttgatctgaaaggatgttatgtacagcaagcagcagcagttaagagtctggggagtagctgcacagggcgaggtgtcaagatgggaagggtcctgcctccttatgtgtttttccctgtaggggaggaagcctcttatgggcaatggttgggcatattttccagccagcccttctttctataggggccagggtgggcccagctcgtcttggcttccaccaccaggagagtgagggcattgaagggccataaatagtcctcccatctacgtgcaccagagggtgtcgtctaggctgtgcatgccacgaggggaaggagccaagaatgagtgtatgggttgttttcatgtttaggctgggataaaactgttttcaattgcgcctgccgggtgaaaaccacagcagcatcagcaagcttggagaaggccagcccgcccagcacaggctcacgttcccactcaggcggtcagtcgggcgggggtgtgagtcaggcaggcgagggtgtctgtgcctgacatcagcacctctgcttagccactgcagcccctggagcagggtagggcgtcatttgcagcaatcacctgctgcctcacacgtcgcagcttggaatttcaacgaccatcagcgctggggttgttgagggatcatagcagattttggtgcagcctggttgtcatgctctttgtggaatggcctctatgttcgagcaattcgttggatgttgaggtgcttggggacagagagtcgaatgatgggccagggtcaaacatgcgagcgtttggctgagtcagcggtttttgctggtcactttttcttttgtttcttatttaggtttgatggatgtgttttgtgctgctgccctgaagctgcagcagcgtgtctgccctgcgctactgcgggcaccaaggctatgtgctggtgcactcggctgcgctgcacctgtgcacctcgcactccgtccagcctccatgcagcacacgtactcacggtgtcctcctgacctgtcgtacgctattccaaacttgctcttttgctgccgctgctctcgtacacaattgctgttgattatcgatatctaatcgagcgcctgctgactgaactccgcaggtttggatgaactgtatgcagagtggtctgaagtggtgagcaccaactttaggtgggtgggctctgaaggaggaggagggagcgggtgattaaacagggcctgcatgaagaggagcaggggctgcatggacagcagggggaaggtgcagaagggagggtcaagcggggttcaggtggctgtgggtttctgcacgagcagtgaaagaagctgtatccttccacctgctttcactggcgaaaggttgaaaacaggatgtcgcagctggaaagatgttgcgctgtcaagtgcaagccatggttgagggtatgcctgtgtgcatgtgcttcttaaagttactcctgttctatggttctgggtgcttgttgtttgtggtgcagggatgcaagcggacctgcaatgacagagattggagaacaaccttggggaagggagtttgcattgagagatcctgcaggtgagggggcatgtaagcaatggcaggcaattcaagaacgaatcattgctgcaaatgctgggatggtatgcagctgaggtatctattgccttgtattttgtctcgcattgcatcggtggtgcgttctgtggcctgaggcacagttcttgctgtttgataagggttcgactgagttgtcgtgtgtgctgtgctgcaggcaattgcgtgcactttgttgcagaagaacaggactgagcatagcatcagcctgtggcagggttgtggtagggctgagtggcagggttaaaggggttgcctaccccacccctactctcatgacaccagcaacagcagcagctcatgcagtactcaaatcactgatgtcaatggtgtgacacatttggttaaggctgctttttaaagtgctgctttgggggcagtgactgtgcagagcttggagcgtatccccatgtaatcagaaccgacgagagttcggggcaacctttcatcttcacattttttgtgatcagctacagagtctgaaatcaaatagaggctgccatctaaacgcaggagtcacaacgaaggcgaaaactccaattgctgtactcaatgcactaagtgattgttcaatggataaatacactatgctcaattcatgccagcagagctgctccttccagccagctacaatggctttttccacgccttttgaagtatgaatgttcagcttgctgtgcttgatgcatcaccataaacacaattctacaacatttcatgccaacaacagtacgggctttccctgcaggcagttggtacggcatattatggtttaaacatctatcctccagatcaccagggccagtgaggccagtttgcatagttaagtatgctggctattgcagtaccttatatgcaaacaagtgctcaatctgtttcatcattgtctgtgggcaaattgcctgccaatattctccagttattgcctgttgtttcaaatgattgaaattggaagttgtattgctctacatttttgacttgtgattttttcatttgttgatatctgacaactgtgaactgcactgaacttgctgtgcttataaatgcatttttttgttttgggccacgttgattccttgtgatactttcctgctatcaaaccaaaaatatactctcatgactgacgtgcaacaaatgcatggaagctttcaacgttacgacagctgcttgccccccatcagctattctacatgtgtaacctaccttgcatggccaccacaacgctactgcatgcaagatctggcgcaactggatgtcccaatagtagaagtatccggattatctccgagagttttacatatgtaatcgacgccatttctgtcatcaactataaatccattgctcctgcatttctggcactgacattctaccacaagcaataccaatgttggagagcgacgagagcggcctgcccgccatggagatcgagtgccgcatcaccggcaccctgaacggcgtggagttcgagctggtgggcggcggagagggcacccccgagcagggccgcatgaccaacaagatgaagagcaccaaaggcgccctgaccttcagcccctacctgctgagccacgtgatgggctacggcttctaccacttcggcacctaccccagcggctacgagaaccccttcctgcacgccatcaacaacggcggctacaccaacacccgcatcgagaagtacgaggacggcggcgtgctgcacgtgagcttcagctaccgctacgaggccggccgcgtgatcggcgacttcaaggtgatgggcaccggcttccccgaggacagcgtgatcttcaccgacaagatcatccgcagcaacgccaccgtggagcacctgcaccccatgggcgataacgatctggatggcagcttcacccgcaccttcagcctgcgcgacggcggctactacagctccgtggtggacagccacatgcacttcaagagcgccatccaccccagcatcctgcagaacgggggccccatgttcgccttccgccgcgtggaggaggatcacagcaacaccgagctgggcatcgtggagtaccagcacgccttcaagaccccggatgcagatgccggtgaagaataagcagcagcttgttatgccttccccatgggcatcagcatgctgcaagctgtctagatatccagctttcagtggaggttgagcgagggtcagcagcggttccctggcgatggcggtcagcttttctggaagccttcactaggactgcgcccagcgcatgtgacgccaatcgaacttgtgtgcaaggccaaattttgtgaccctgtgctgcacttcatgtattcaagaattgagaagaaatttcattgctgcccttctttcactttaatttccatccctggatccacctcccaccattgtggttgatgggtaggggttttgggtaggtgcagttcgttgtgcacgttgacatgtgtaacggtgagcaaaggaattgctgggcaagtagctattgcagcttaagggcatggtgaaacacttgtgctgtatttacagaggaagccagacaggtaaggagtgtgtggcagcttggaacaggagggctggtcgcaacaagtatgcatatcccatgattgttgacataagagcagcaggtgcatattgccagcctttgtgaaagtggattgaaaatcaattagttggtgtgatagctgaggctaggcactgccaacctgcagtgaaatgaggctccaagaccgggtaataatacaggcaatcgaatccagttgaaattacggcgattaaatccaagcgagcgttgtaagaacatctgcacctgtctgaagtagtgagcggataatgagcattgcttgccttctatcactatacctgacagttacgtgtcacacactctcaagcacaacacacagcggcaaagttacttgctaaacctcacagtcaagctgaaaataaaggctaaattacgtgagaccggcgcgccataacttcgtataggatactttatacgaagttatcaccagatataggtgacccgataacttaattaatcttgcgaagattgaattgctaatagaaggttctcatctatacatgagttaccagtgaaccccatatctgctctataatatagtccccgctgaggcgcagtgctgaggttccagctcgaacgagccagtagggcttcgactcacggctcatttattttagagctaggttgacttcccagtctcatgcaatacatgagagcaggtgttggtcgcacgcctctctcacggtgcctcttgattttcggccccttgcacccgctctcatatgacatattcgcgctgcacccttgctcagagcaggcgcagcatgtggagtagcgggcgcaagccgtaatgaggagtctcagctcaacatgattgaggtcagcatcactgtaacaatacaaatcattgtggtgccttatatatttggtaaatgctcgctgcagtattcaaatcgaccttcactgcaagcaactcgattgaactacgcgcgttattgaaggcacatacaaccgggagttcagaggagtatgcccaagaagaagcggaaagtcgggagcaatctgttgaccgtgcatcaggtatcgagaagaactaaagagcgttcaaacgcatcaatattttgctaaagagctttacatctttttggggctattttctggctactcggtagtgacttgaccactttcttcccaagtgggggcaagccgataagccgctgtgaccgttgatttttttataaaagacgtagacatgttcaatcagccacaattgatatgcttgaatacagaacctgcccgcattgcctgttgacgcaacatctggtgagctgcggttgctatcctcccaatataacctgaagtcatgcatatattcgcactaatctacatcccatgttgtgttgagctattcggtattgatgccagctcagtgaactaattatcaaatgtatatcggtgctgccagaatcgatccatgtatcaatgccacaagtaactggagatacatttgctacatgtagatgaggtgcgcaagaacctgatggacatgtttagggaccgccaagccttcagcgagcatacatggaagatgctgctgagcgtgtgcagatcttgggcagcatggtgtaagctgaacaaccgcaagtggttcccagcagaacccgaaggtatgcctgggtaactgtcaaaatcatgtatattcccgcaatgcaagtggttcattgttgtgctttacgttaaagacgtgtcagctgcaggagaattattttgaggatgattgtccgttgttggcgatgtcttgcattgtgaagtatgttttgaagtcatacaggaagtgtgaaatcccaaagcagctggctgccgctgcatgcgaccagtcattcacctgcattgtgtgtgctgtagatgtgagggactatctgctgtacctgcaagcaaggggactggcagtgaagaccattcagcagcatctgggacagctgaacatgctgcataggaggtctggactgcctaggccaagcgatagcaatgcagtgtctctggtgatgcgccgcattagaaaggagaacgtggatgctggggagagggcaaaacaagcactggcatttgagcgcaccgactttgaccaagtgaggtgggcttcgcaactgctgcctgaacttcctgttcctgtgcatgtacatgagagtcggttggaacaggctcatactgcgcctgattgataggctgtcccacattgttttatttgctgtatcgatgtattcattttgcattgggtcctttctgctcatgaagcaccaagaaggctggctgtcaatggcatgccagctcatgccatctggatgacattatgcaagaccagtgttgactcgaacatgaatcttactggaaactttaatgaatgctttcgagctttttgtgcaggtctctgatggagaactcagaccgctgccaagacatccgcaatctggcatttctggggatcgcctacaacacactgctgaggattgccgagatcgcacgcattagggtgaaggacattagccgcacagatggagggaggatgctgatccatatcgggaggacaaagaccctggtgagcacagctggagtggagaaagcactgtctctgggagtgaccaaggtaagcttaccatgtgtttatatgaagctgatatttggaagaaaggaggaagcaacgacaacaagggcggtgcacaatctattgccgcttttgaatcttgcccgcaaaggcagtcgatgattgctcactgtatcaggttgatttagttgatgaggtgtagctggggaagctccaatccccagtccagatagccttggttatgaattgcataatgtaggcaccacttgcactggtcctaaaccccagttcattcctgtccttctcgtgcattttgtcaaatgaacatgcaaccgagtgtgttttcctactcgacatgtgtgcgattgcccacgtgtgctgcagctggtggaacggtggattagcgtgtctggagtggcagatgaccccaacaactacctgttttgccgcgtgcgcaagaatggagttgctgcacctagcgcaaccagtcaactgtctacaagggcactggaggggatctttgaggcaacacatcgcctgatctacggggcaaaggatgattctgggcagaggtatctggcctggtctggacattctgcaagggttggagcagcaagggacatggcaagagctggagtgagcattcccgagatcatgtgagaggccccagcaaaaacaacagcactagctgttgctgctcagtttgtgctcgtgatgtttgaaaggaatggacaaggttcatccatgatgttcattatctgggctggtcttgtacatggggttattctatactaaacaggagcgatacaaataacaaacaatcaatgtctatatacacatatacttggctaaatttttctcccggccttacatacataacaaaggctaaactaattgacccaaaataattgtatgaataatcaaattgatgcatacaaataatcctaaaaatgaaaaaaatttcattgaaataagtatagaaataacaaatgtttgacccacagccctcactctccaacccaatcctgcctctcacaagacttgccatgtaccaacttacaatgacagcgagctacaacaagttccatcaaggtgtgggttgctattagttggtggaacgtttgtacatttcacagttggacatgcacttgcgaaaaaggcgttggcttcagtgaggcagtgcttgctcgtatcccctccaagcatgccttgtgcacccattttgcaacgcaggcaagctggagggtggacaaacgtgaacatcgtgatgaactacatccgcaacctggacagcgagactggagcaatggtgagactgctggaggatggggattaatcaggatgttttgagcggttgtaggttctgtagttgtatggtaggttgcatggaggaaataggccaacaacaattccaaatcaaaggagattgtagcgttgctcttggtccccctgaaaatttttgttgttatgtgtctataaatctagttctgcaccttgcaaactgtgggatgccctgtccagagcagaaggtaatcccaaaacagtcgagaaagtctcgttgggtggttgtgtaaagtacaaatgtatgttttccaccttgtctttgtattgtgcacgagctacagcattggtggaagggcttatagctgctgggtcatcatgctgtcctgttcttgatggtttaggtgtcatccctttcactgactcagcgaaatcggatgcgtaccattcatgaacggtgttgcacttgctgtttgtgaaaggtactgcatgtgcattgtacaatagactactataatgtctcatgcacgtggtcaatgatgtagatttctggaatatgcatcgtgtaattgattcgatgaacccctcgtttggaactctatttgaaaagcaatcgagtgtcattatccataatggatgatgatcatgagcattgcaaatagcaccattagaacaaactgaatattgtacaccttgacctggatatgcatccgtccttcatcccactttattaaggcaggttataattggcaaggagtcggcagaatagtcgtttggttataccccagttttagtggggcctttggcagctatattatggtcgcgactgtaaccgggtccgtttaaagttcgattacatctcagaaatataattgggctgcatgttagaaacttttcgccgggtataaccggggtataatcggcatactgcccaatgacggccagccgctggtcagtgaccgtcaaacggtcggacggtctgcatcgcatgtgcgctgacatgtcaagtgcatgcttctcttacattcaggcaaaagactacaagtcattgaagaattgtcaactcagtaagctgacaattacgttcatgaaggtcagtcgtatgaaactcgtatttctccctaagtcgttactatggaaagtacatcgtgccacgtcatcgtcatcgtggcaatgacagatgatggatagggtggggttggcattaattgctatcattttctttgcagaaaacaaatacctggcacataatttgttgataatcatatgtatgtatgtccacatgtcaacgttatatgtataaaaatcaagacttgtttgcttaactctaaatttaatgtaagaatttcggtaataatctgatctacattatcacttgtgattaatgttgaaatttgttatccttaattatcgtgcttggcacaactttcagattttgtctgctgtcacattcatgcagtttcatttgcagtaaattctcaatcatttatgtagttgataagaatatttgatctgcttttcattaagcaaattttgttagctttctccccttgattgttcattcaatgagattacattgaatgatgtctacacatataataagaacgcatgtctacacaaatctaaaaatcagctgcacgctcccaattactatcgcacactctgacaccagaccgtgctgtgacaatataagctgcactgacaaatttggaaaacacaagattcagaagaaaacaaatactggaacccctcacacaccacctttctacagcacaaacacgaagcagtagccaaggtaagaaaatccgatcaaaatacattaaatcatgtctaatatacagcataagtatagctaatgaaatcgttggtcgggccttaataacacacagtctaccaacacctagttggtaaataccgttgctgatattgctctgtaccagtaaaagagggctgcgatgagcgtttttagtgcacttcttcaacacggaatatttttcacaaattggtatgagaaccaattttgcaaaatgttcgccctgtaaagtatcgctctgggacgatcagcttgacgtaattgtaggcgaaaagggcgttcaaagtgcagctttatgtatgaacgtcataaaatataaagcatagcacaatcactgatagaaaatatttgtgcgcattaaaactctcacttctgttgcggatacaacgacggaaatgagaagcttgtgtaagaagcaattcaagttttcattttgtcatctaaggtgtgatcctccgatattcattaccgaatgctgatctgagttggaaagatggcaatatttagctgtgcacactttgacctccaggccttggcgggaatttagtattctagctttcctattggaacgataggccagccaagtctccagcttgtatacgctacaccagcagacatgctctcaatttagctgacagtgtcttcatatttgtattatctgttgtgtctatgccgaagaagaagcgcaaggtgggcgactacaaggacgacgacgacaagctggagccaggtatgcataacctttcaatagatgctgccgcgccttgggttcgctgcctgtgtcctgaagtacttttcaccaggtctacatgcatgcagcaactaatcgttagttgttcctttgtaaacagcgttttctgtctttaccatgattcaggcgagaagccgtacaagtgtccagagtgcggcaagagcttcagccagtcaggagcactgacccgccaccagagaacacatacacgcgacaagaagtacagcatcggcctggacatcggcaccaactctgttggttgggcggtgatcaccgacgagtacaaggtgccgaggtatgttatctttgattgcactacttgcagtcctggtgggcactattgttgtgcataggcgctcttttgcattcatgtattgaatgtagagaagttgtacactcctcctaggagactagctgatggagtcctgtattaaatttgttcacatcatatgccttacagcatgatccattagaagtaactaaatttctaagcacccagtctgagaaaccagatcgatggcaagttgctcttggcttgctgtgcttgcagcaagaagttcaaggtgctgggcaacaccgaccgccacagcatcaagaagaacctgatcggcgcgctgctgttcgattctggcgagacagcagaggcgacacgcctgaagagaacagcacgcagacgctacacacgccgcaagaaccgcatctgctacctccaggagatcttcagcaacgagatggcgaaggtggacgacagcttcttccacaggctggaggagtcgttcctggtggaggaggacaagaagcacgagcgccacccggtaagtcgcgtgccaagcactagtttaccatcccacaaatgacaggtctgggtgggacatctgcacctgaaaatggcttacgacagctgcttctcaattcgagtgtgcatattgcaagcattagattttttcctgcagatcttcggcaacatcgtggatgaggtggcgtaccacgagaagtacccgaccatctaccacctgcgcaagaagctggtggacagcaccgacaaggcggacctgagactgatctacctggcactggcgcacatgatcaagttccgcggccacttcctgatcgagggtgagtgtggaatgcatcacagtggaaactgctttgtagtacaatttgtttgtgaagtttgtgtctagatgtccatttgatctgtggaatgaatgtgctagctctcatgcacagcagtatttggaatgctgaattacagtgtttcctttgttggtgtcaggcgatctgaacccggacaacagcgacgtggacaagctgttcatccagctggtgcagacctacaaccagctgttcgaggagaacccgatcaacgcaagcggcgtggacgcaaaggtgtcttgatgtaaagtcgaacattgcatttgaacgaaggagctcccttgttggctaagcatgggtattgactctaccccagcagggaatcatcttgctgcaacagctcacgtcgtatttgtatgtggtgcaggcgattctgagcgcaaggctgagcaagagccgcagactggagaacctgatcgcgcaactgccaggcgagaagaagaacggcctgttcggcaacctgatcgcgctgtcactgggcctgacgccgaacttcaagagcaacttcgacctggcggaggacgcgaagctgcaactgagcaaggtgaacgtccccctcggccctgtgctggtgtgcctgctgtccaatggcacgtttgtgcttcacaattctacaggttgatgcaatgtaggttggttgtgctgatgccagagatgcactcaaccaacaccgtgttgctttgttggttcccaaccagcctgcaatgcaacctgtgaatcgtgcaccatacgatctgcatgcaggacacctacgacgacgacctggacaacctgctggcgcaaatcggcgaccagtacgcagacctgttcctggcagcgaagaacctgagcgacgcgattctgctgagcgacattctgtaagtctcagagcacatcacctgcatcacacaggatttcttttgtcagcatatcctgccttttcgggtcatgtttggatgccgtgcggctgtgtgccactggtccaggcgtactgggctttctgacaagctggatgttatgcttatattgcaggcgcgtgaacaccgagatcaccaaggtgagccgcacacttgctattgctcgctttcacaaaatacccgtcgtgaaaacgtcatgtgaaggttgctatcatcgggtcagagagtatattacatcatgaacaggctgcaagggtttgattcctgcaggcaccactgagcgcgagcatgatcaagcggtacgacgagcaccaccaggacctgacactgctgaaggcactggtgaggcagcagcttccggagaaatacaaggagatcttcttcgaccagagcaagaacggctacgcgggctacatcgatggcggtgcatctcaagaggagttctacaaattcatcaaggtatgtttggcacaccattgacagaaggggcatgtcttgcccagtgtgcactgctgtcaggtcgatgagagaagtggcaatgaaaaattttggtttgacaacaaatatgagggggtactcgggactgattggcaatgcgttagaaactccgtaagatcaaatttctgaagtggtagcagtggaagttcctagctgagggtgtcactcactcttatttctgcagccgatcctggagaagatggacggcaccgaggagctgctggtgaagctgaaccgcgaggatctgctgcgcaagcagcgcacattcgacaatggcagcatcccgcaccagatccatctgggtgagctgcacgcgattctgagaaggcaggaggacttctacccgttcctgaaggacaaccgcgagaagatcgagaagatcctggtacgtggcccgggttcacctgttgcgtgcatgttgacttcaggacaaagttagcattattacacagcggcagcacagtgagggtcatcatgtggctggctttccaattgctccgagggaataatcggttgaatgtgtgtttctcttgccagtgtgtccttggaggtgcgtgcgtgcttcgcaaaaaaggagtacccaataacccttgaaacaaccagttttgggctgcaacaacacaagaccgcggtttactgcctgactatgcagacgttccgcatcccgtactacgtcggtccactggcacgcggcaacagcagatttgcgtggatgacccgcaagagcgaggagacaatcaccccgtggaacttcgaggaggtggtggataagggtgcgtggccagtaccagctgcaccccacaggcggttgttttgacatttaaaccgctttcaggaagcgtttgtacactcatgcgcttcatggtctaccagcaggaggtctggaacacattcagatctaacatgaaatcaagcttgcatttcaaaagcggggcatccaagtgcagcggggatgaactgctgtctcatttctatgcaggcgcgtctgcacagagcttcatcgagcgcatgaccaacttcgacaagaacctgccgaacgagaaggtgctgccgaagcatagcctgctgtacgagtatttcaccgtgtacaacgagctgaccaaggtgaagtacgtgaccgagggcatgcgcaagccggcatttctgagcggtgagcaaaagaaggtgggtggtgcacaatgttgatgcagatttgacgctgtatcactgctgtctcgctgtacagcatctgatacactgctgttcccgctccccgcaggccatcgtggacctgctgttcaagaccaaccgcaaggtgaccgtgaagcagctgaaggaggactacttcaagaagatcgagtgcttcgacagcgtggagatcagcggcgtggaggatcgctttaacgcgagtctgggcacctaccacgacctgctgaagatcatcaaggacaaggacttcctggacaacgaggaggtgattgtgggtggagtgcaccgcgaatgaatggggcactgcagcacaatggagcacacatccaatccgcaatgagctctcctgagactttttttggctcctgaagcaaaccagacaatgtgcgcctatttcacggacctggcgcatggaagtagtctggcaactatggctggagcacaacaatttctggttattttgattggaatgattgggggaaaaaacaatgtgttgcccgcagcacaggccctggtgcagttgagttagctgtagcagtagcagaaggcatgtcatcgaaaaagtaccgaattgtgccatcatccccaccctgctgcagaacgaggacatcctggaggacatcgtgctgaccctgaccctgttcgaggatcgcgagatgatcgaggagcgcctgaagacatacgcgcacctgtgagtggttgccctggacactggagatttcttgcatgttgggtgtggctgattgtgcctgcatcactggatgattgtggcacattttcggtttaatattcagggtactgctgcaaacgagcttggttcaactgacgtacctgaaccagtcgttttgctgcttgcaggttcgacgacaaggtaagctgtgacaggacaagctggcagattcttcacttgcacctgtccagctgaatctacaaccatgggtgaaggatgctgccgttgctggcagccacacctgtttgaaactaaaatgggagcaacctgtgcagcaaggtcctacgatatcatacctgcttcttcaaccatctgatgccccttatcaacaagcgcaccctgcaggaattacccttgcaccaaaacctgggcacgttgcctgccgcttgccagaactagctgtctgtgccactcccaacatgtgcctagcatctgtgatatctgctacaggtgatgaagcagctgaagcgccgccgctatacaggttggggtagactgagccgcaagctgatcaacggcatccgcgacaagcagagcggcaagacaatcctggacttcctgaagagcgacggcttcgcaaaccgcaacttcatgcagctgatccacgacgacaggtgagccaggggaggtgcattcctagcctgtgcttgcttgtgtggaccctatttgggaggaggaagattgacctggtatgaaatgtgaggctagacaacacatgcgactatttctctccagcagcactggcaggacgatgggactgcatgtgagggcatgtcttgacatgaaatgtcttgccaccagtttgatgtgttgacatcgaacatcagccccccttccccagctattatctagttctggtcctatcagaccatgcgcaatctgctggcggtctcatctttaaaagcattcttgtcatcaggctgtgcagtggagccagcaataaaaccaacctattgttttgcagcctgaccttcaaggaggacatccagaaggcgcaggtgtctggtcagggcgatagccttcacgagcacatcgcgaacctggcaggctcaccagcgatcaagaagggcatcctgcagaccgtgaaggtggtggatgagctggtgaaggtgatgggccgccacaaaccggagaacatcgtgatcgagatggcgcgcgagaaccagacaacccaaaagggccagaagaacagccgcgagcggtacgcagaactctggcgtagccacgcaaatcatgtttgcagatgaaagttttgtcatatgcgcaagaccagggaccttctatgtatcaaaaggcttaacagtgtgttgttggttatgttgtgcagcatgaagcgcatcgaagagggcatcaaggagctgggtgagtcatgtggaaaggtatcatacattagatggtgttcccctgttgtacaagatctggcagcatttggatgctgccattggagatttcatgagatattcagttaaactaaaagcgtgagttttcgcagcagaggatagagccaaactcacaaatcattttggcttggtgcaggcagccagatcctgaaggagcatccagtggagaacacccagctgcagaacgagaagctgtacctgtactacctgcagaacggccgcgacatgtacgtggatcaggagctggacatcaaccgcctgagcgactacgacgtggaccacattgtgccgcagtcgttcctgaaggacgacagcatcgacaacaaggtgctgacccgcagcgacaagaatcgcggcaagagcgacaacgtgccgtctgaagaggtgaggcatcgcacaggatatacagtgggttccatgagtgctgttgtgttgtgcattgcttcgacccgctttccaacctgtgcgtggtgtatgggtttgcaccatggcgtgcacgggcacaggcatgtcatgctgcaagcaacagggccgccaagcttccttcacctgctcggtgatctttgtcccttcctccaccctccctttttccccgccccaggtggtgaagaagatgaagaactactggcgccagctgctgaacgcgaagctgatcacacagcgcaagttcgacaacctgaccaaggcagagaggggtggcctgtctgagctggataaggcgggcttcatcaagcgccagctggtggagacacgccagatcacaaagcacgtggcgcagatcctggacagccgcatgaacaccaagtacgacgagaacgacaagctgatccgcgaggtgtgacccgggtgtattagagagatgcgcaacgcgtgctggttgttgttgccgttgcacctagggagtaggtcgaatgccgcgttggtgcccgctggggtggctgtatcatgctggatggggttgcaatcagacccgggtaagaatgaagtgtggagctcactgttccgtcgagcgcttcagcctgcttgatggtgatgccggtttggcgcaggtgaaggtgatcaccctgaagagcaagctgtgagtggcgtgctgcacaattgtttgtcaagtgcacttgttcttgatacaaagttgggctcgccattgatagcaagaaaaagaacttgccacctggatagctgcgtctggaacatgttgcatggagggaattttatggtgacacccatggtgacactcttcatggaacctgctggccacctgctggtatgcctcttgaggctggatgatcaacaaatgatgtgccgcagtctacagtcaatttcagttcacccagtagctgtttttcattcgtgctgcagggtgagcgacttccgcaaggacttccagttctacaaggcaagtgccttctagggttcagatctaagccagagcagtgaacaactggtgctattatatcgtacatatggtgctaattcgcctgcttgcagctcagcaggcaccattggtgcacaggaaaatcggcgcatgatccaagtgcagctgcgcctcgcagcttgtacccctgctgagttttctttcggctgttgcccatgcaggtgcgcgagatcaacaactaccaccacgcgcacgacgcctacctgaatgcagtggttggcaccgcgctgatcaagaagtacccgaagctggagagcgagttcgtgtacggcgactacaaggtgtacgacgtgcgcaagatgatcgcgaagagcgaggtgagcactcacaggcagttctgttaccaacatctgcgattttcttgggcagagagtgtatcttagacctcattcacctcagattcctgagcgagctgcaatgcccgttgtcagcctgtgcaatgaaggaaaaacctgtcgtaatgcttgcagcaggagatcggcaaggcaaccgcgaagtatttcttctactcgaacatcatgaacttcttcaagaccgagatcaccctggcgaacggcgagattgtgagtgtcacagtagtgtgcatcttcgtttgatccagtttgatccacgtgcagctgcccatcaagtccaggttgtggaccttcatctttggactggcagtgtatgaaaagtccactgggaacctgctctttttcataccgcatcatgcatatcgtgtcccatcgtgcgtacttcatgagttgtccctatttttattactgtcgtcatcacttccaacgtccacagagccaacacgacttgtgctgaataaaggaatgaaatcgcctatttaatataaactggtattgtgggacaaagtccaattcgcaagtctgatgcgcacctgtgcagaggaagaggccgctgatcgagaccaacggcgagacaggcgagatcgtgtgggataagggccgcgactttgcgacagtgcgcaaggttctgagcatgccacaggtgaacatcgtgaagaagaccgaggtgcagaccggcggcttcagcaaagagagcatcctgccaaagcgcaacagcgacaagctgatcgcgcgcaagaaggactgggacccgaagaagtatggcggcttcgacagcccaaccgtggcatatagcgtgctggtggtggcgaaggtggagaagggcaagagcaagaagctgaagagcgtgaaggagctgctgggtgagcggccagcacatgcacctaggttgcctatcacatggcaccaaattgcatagccatttcagggtgattcacttcccggtaacaggcattgtctggcagcctcatcgtatgcatgaatggagatgggtcaattcaagcttgcatttcaaaagcagggcatccaagtgcagctgggatcaactgctgtctcatttctatgcaggcatcaccatcatggagaggagcagcttcgagaagaaccccatcgacttcctggaggcgaagggctacaaggaggtgaagaaggacctgatcatcaagctgccgaagtacagcctgttcgagctggagaatggccgcaagcgcatgctggcatctgcaggtgggtggtgcacaatgttgatgatagtgccctgatgtagtgcgcagatttgacgctgtatcactgctgtctcgctgtacagcatctgatacactgctgttcccgctccccgcaggtgagctgcaaaagggcaacgagctggcactgccgagcaagtacgtgaacttcctgtacctggcgagccactacgagaagctgaagggctcaccggaggacaacgagcagaagcagctgttcgtggagcagcacaagcactacctggacgagatcatcgagcagatcagcgagttcagcaagcgcgtgatcctggcagacgcgaacctggataaggtaggaattttcccctccctgcaggtggccagggaaatgaaccggtcaccatgtaccgggtagcacgggtggacacacggcagtggccagggaatcgtactgctgagggtccccctgcatgcagactgtgggggttccctcaggctccgtctttgttgcacatgcaatggtttgatcggtctcagttggcatctctattgaaactgctatattcctatgccagtgacgcagaggtgaggatggttgacaaggttttgacgtagtgggtgttgagggtgctgtgcaggtgctgagcgcgtacaacaagcaccgcgacaagccaatccgcgagcaagcagagaacatcatccacctgttcacgctgaccaacctgggcgcaccagcagcgttcaaatatttcgacaccaccatcgaccgcaagcggtacacaagcaccaaggtactacctgcctgcccaaatgctgttgggctttgcagcacaaaggaaaattctccagccagggtttttcctgctgcaacactgttgtatgatcgctcacaataagggggaaataggtttccaagtcatggttgtgacagtggaaaccaagtcttttttgcctccaccaagtttttgtcctcaaatttaattcaatggtggtttgtaggaggtgctggacgcgaccctgatccatcagagcatcacaggtacagtgcagcagcacaatccctcgtcaagcttacttgtgttgcattgccaaattgcccaatttcctatgaagtttgctgtacatttgatcatgcgctaaattgcttttacgttctatcgctttgtatgcatgcaggcctgtacgagacccgcatcgacctgtctcaactgggtggcgactgaggtgcgaatagtgcttcagtaaaaaagtagcaacttggtgcaatatcgtcagggtcgtgtggtctgctcgccagcaagttttttggcacaggagagcgctttttccgagtaccgccaaagttcaagcatgtgctgtgattcgctgttgcctcttatgataattgctcaaagtttccaagcattctatgtccaccctgcaccactaagttgtatggtgcttattctgcaggggatgattcatggtgcctaaaaattttgtgctgctgtcgcgtctgttttctgtcgcagtttagtgaatgtaactccaaataccaaacttttcatcacaatcatattgatgcctttgtaagtgaattacagcgttttttgccataaaaagaagtaccgtgacattggggtcgtcataacaagaagctttatgaacaagcagcttgatctacgagacttatacataaatggtttcgggtaactcctaatacggggctacgttagttcagcagctgagaacgaccacgaacgggaagaattccagccatgttgaagaggtgcagctatcaaggtgaggtctttactggtgtctgttattgctgtaacatcatttcgctgttgcacaatttaaacatttgtaatttactgttgttattgcagtggccacttgtagcagtggcagcgaggcactgacacttctacgtgaacgcaacgaggacggatcctccgaccagttcgacctcgtactgtcagatgtttacatgccgggtatgtcgtattcctttgtaaactttacaatatgcgtctagtttgacgcgtacactttgtacactttgcaaaaacgcaccctgcgaggtctgccatttggtcactacaacttggccaccttggttgcaagtttgcaagttcgctctacgtcaacgctgcaaaatgaaccaattgttttgcactgaccctgccaaccttcatttgtggctgcagacatggacggtttcaagctgcttgaacacatcggtctagagttggagcttcccgttatcagtaagttgatcgagccgagtccagagcgaagcctgcttctatactattagcagctgtcttttgatatttgacagcttgacttgatatggtcacagagcatacttgcaaccaggttacctgttgaactagcaactgtgcccaagcatctcttcaagcacctccgtcagtccatagggtactgttgatttgtactctgcaatactgcactgtaatgcgctgtgaatcactgcccttcacctctagatggtgcttccctggagccctcccccacctccgcctcaagcccctcacatgcctctcccccccctgcagtgatgtcatccaacggggacacgaatgtcgtgctgcggggggtcacccacggggctgtggactttctgatcaagcccgttcgaattgaggagctgcggaacgtgtggcagcacgtggtgcgtcgtcgttccatggcgctggccaggacgccagacgaggggggacactcggacgaggactctcaggtgcccttggcagcttctgggcggcttgctgtgtcggatgccacttggactggggatgcacgaggggtggggggacaatgggagatgggccatagtaggccagagttgatggcagtggtggtgggggggagtaggcgggagagaagcagccatcctggtgttggttttgatgattgagtgcatggggatgatgcacaggtgagctgactggatgccttgtcttgctgtgctgcgctgcagcggcacagtgtgaaacgcaaggagtcggagcagagcccgctgcagctcagcacagagcagggcgggaacaagaagccaagagtggtgtggtcggtggagatgcaccaacaggtgtgcttgcgggcgggtgtatacgggggaggggggccagctgctggctgacctggcgtgcgcggtgcattgcacttggcgatgaggggcgtgcttcagtatgtagctgggacgcaattggttgtgctgtgtgaccagtgcacaaaatacatccctgaattccagtgggttgaacagagttgtcctggaggtgggaagcaaacgcgcacgtggtagaggggagcagggtgcagaacagccgcagcaggggtgttgcgcagtgtgcaggtatcctgcctccatgccccgggccatgggcatactacgctggtaccgtcaggatgggcgttgagcctggcttggggggcagggggcgagcgaatgcggaatgggagcggcaggtgctgggagggtggctgactggcttgcaggagcgcaagtcctgtcgggggcgtcgtcctgttccctcctgcccgcttcacccacgttcactctcatgcctccacactcctgctgctgacacacctgtcgccacctccgctgcagtttgtgaacgcggtcaactccctgggcattgacaaggcggtgcccaagcggattctggacctgatgaacgtggaggggctgacgcgcgagaacgtggccagccatctgcaggtgcctgccatgacccgcgat

SEQ ID NO: 87 - DNA, 30 bp, Artificial Sequence
  Description of Artificial Sequence: Synthetic primer
aggctactctcagacatgacggtggctctg

SEQ ID NO: 88 - DNA, 30 bp, Artificial Sequence
  Description of Artificial Sequence: Synthetic primer
gccacaaatgaaggttggcagggtcagtgc

SEQ ID NO: 89 - DNA, 23 bp, Artificial Sequence
  Description of Artificial Sequence: Synthetic oligonucleotide
acaccaccttaaggcacatgagg

SEQ ID NO: 90 - DNA, 23 bp, Artificial Sequence
  Description of Artificial Sequence: Synthetic oligonucleotide
ggcgtgggacatggtgcgcaagg

SEQ ID NO: 91 - DNA, 55 bp, Artificial Sequence
  Description of Artificial Sequence: Synthetic oligonucleotide
tgaagcaccccccggcctctccccccgcagggccgcccctcccgcctcgtcgtgc

SEQ ID NO: 92 - DNA, 56 bp, Artificial Sequence
  Description of Artificial Sequence: Synthetic oligonucleotide
cgcaacgctctccctccccaccccccagcctcacatccgcctcaagcagcgccctg

SEQ ID NO: 93 - DNA, 25 bp, Artificial Sequence
  Description of Artificial Sequence: Synthetic primer
caagctatgcgaggaagggagggtc

SEQ ID NO: 94 - DNA, 23 bp, Artificial Sequence
  Description of Artificial Sequence: Synthetic primer
ctgccgcaagtgagtgtgctgtc

SEQ ID NO: 95 - DNA, 25 bp, Artificial Sequence
  Description of Artificial Sequence: Synthetic primer
caccagatataggtgacccgataac

SEQ ID NO: 96 - DNA, 24 bp, Artificial Sequence
  Description of Artificial Sequence: Synthetic primer
aaaactccactgcacctgcaacat

SEQ ID NO: 97 - DNA, 20 bp, Artificial Sequence
  Description of Artificial Sequence: Synthetic oligonucleotide
tgcggtgaagcttggagctg

SEQ ID NO: 98 - DNA, 59 bp, Artificial Sequence
  Description of Artificial Sequence: Synthetic oligonucleotide
ttgccgtcgacgagacttcggggcgcgcatttatcgactctcttgaagatacaccggtt

SEQ ID NO: 99 - DNA, 65 bp, Artificial Sequence
  Description of Artificial Sequence: Synthetic oligonucleotide
tccaattgtagatatcatattgtttccggacctaccttacgcactgagtgctgccagatgttctt

SEQ ID NO: 100 - DNA, 28 bp, Artificial Sequence
  Description of Artificial Sequence: Synthetic primer
gaggtgggtggtagtgcttcgcgaggtg

SEQ ID NO: 101 - DNA, 29 bp, Artificial Sequence
  Description of Artificial Sequence: Synthetic primer
atcacagctcacagggcagacactgcgtc

SEQ ID NO: 102 - protein, 7 aa, Unknown
  Description of Unknown: 'SHAQKYF' class family protein sequence
SHAQKYF

SEQ ID NO: 103 - DNA, 23 bp, Artificial Sequence
  Description of Artificial Sequence: Synthetic oligonucleotide
gggacatggtgcgcaaggacggg

SEQ ID NO: 104 - DNA, 23 bp, Artificial Sequence
  Description of Artificial Sequence: Synthetic oligonucleotide
tgcggtgaagcttggagctgtgg

SEQ ID NO: 105 - DNA, 23 bp, Artificial Sequence
  Description of Artificial Sequence: Synthetic oligonucleotide
acaccaccttaaggcacatgagg